European Patent Application EP 4 744 482 A1, published May 20, 2026. Title: Transgenic insect of Lepidoptera. Applicant: National Agriculture and Food Research Organization. Application JP. The sequence listing filed with the application follows.

SEQUENCE LISTING (38 sequences)

SEQ ID NO: 1 - protein, 5263 aa, Bombyx mori
MRVKTFVILCCALQYVAYTNANINDFDEDYFGSDVTVQSSNTTDEIIRDASGAVIEEQITTKKMQRKNKNHGILGKNEKMIKTFVITTDSDGNESIVEEDVLMKTLSDGTVAQSYVAADAGAYSQSGPYVSNSGYSTHQGYTSDFSTSAAVGAGAGAGAAAGSGAGAGAGYGAASGAGAGAGAGAGAGYGTGAGAGAGAGYGAGAGAGAGAGYGAGAGAGAGAGYGAGAGAGAGAGYGAGAGAGAGAGYGAGAGAGAGAGYGAASGAGAGAGYGQGVGSGAASGAGAGAGAGSAAGSGAGAGAGTGAGAGYGAGAGAGAGAGYGAASGTGAGYGAGAGAGYGGASGAGAGAGAGAGAGAGAGYGTGAGYGAGAGAGAGAGAGAGYGAGAGAGYGAGYGVGAGAGYGAGYGAGAGSGAASGAGSGAGAGSGAGAGSGAGAGSGAGAGSGAGAGSGAGAGSGAGAGSGAGAGSGTGAGSGAGAGYGAGAGAGYGAGAGSGAASGAGAGSGAGAGSGAGAGSGAGAGSGAGAGSGAGAGYGAGAGAGYGAGAGAGYGAGAGVGYGAGAGSGAASGAGAGSGAGAGSGAGAGSGAGAGSGAGAGSGAGAGSGAGAGSGAGAGSGAGAGSGAGVGYGAGVGAGYGAGYGAGAGAGYGAGAGSGAASGAGAGAGAGAGTGSSGFGPYVANGGYSRSDGYEYAWSSDFGTGSGAGAGSGAGAGSGAGAGSGAGAGSGAGAGSGAGAGYGAGVGVGYGAGYGAGAGAGYGAGAGSGAASGAGAGSGAGAGSGAGAGSGAGAGSGAGAGSGAGAGSGAGAGSGAGAGSGAGAGSGAGAGSGAGVGSGAGAGSGAGAGVGYGAGAGVGYGAGAGSGAASGAGAGSGAGAGSGAGAGSGAGAGSGAGAGSGAGAGSGAGAGSGAGAGSGAGAGSGAGVGYGAGVGAGYGAGYGAGAGAGYGAGAGSGAASGAGAGSGAGAGSGAGAGSGAGAGSGAGAGSGAGAGSGAGAGSGAGAGSGAGAGSGAGAGSGAGAGSGAGAGYGAGAGAGYGAGYGAGAGAGYGAGAGSGAASGAGSGAGAGSGAGAGAGSGAGAGSGAGAGSGAGAGSGAGAGSGAGAGSGAGAGYGAGVGAGYGAGYGAGAGAGYGAGAGSGAASGAGAGSGAGAGSGAGAGSGAGAGSGAGAGSGAGAGSGAGAGSGAGVGYGAGYGAGAGAGYGAGAGSGAASGAGAGAGAGAGTGSSGFGPYVAHGGYSGYEYAWSSESDFGTGSGAGAGSGAGAGSGAGAGSGAGAGSGAGYGAGVGAGYGAGYGAGAGAGYGAGAGSGAGSGAGAGSGAGAGSGAGAGSGAGAGSGAGAGSGAGAGSGAGAGSGAGAGSGAGAGYGAGYGAGAGAGYGAGAGSGAGSGAGAGSGAGAGSGAGAGSGAGAGSGAGAGSGAGAGSGAGAGSGAGAGYGAGVGAGYGAGYGAGAGAGYGAGAGSGAGSGAGAGSGAGAGSGAGAGSGAGVGSGAGAGSGAGAGSGAGAGSGAGAGYGAGYGAGAGAGYGAGAGSGAGSGAGAGSGAGAGSGAGAGSGAGAGSGAGAGSGAGAGSGAGAGSGAGVGYGAGVGAGYGAGYGAGAGAGYGAGAGSGAASGAGAGAGAGAGTGSSGFGPYVANGGYSGYEYAWSSESDFGTGSGAGAGSGAGAGSGAGAGSGAGAGSGAGAGYGAGYGAGAGAGYGAGAGSGAGSGAGAGSGAGAGSGAGAGSGAGAGSGAGAGSGAGAGSGAGAGSGAGSGSGAGAGSGAGAGSGAGAGYGAGVGAGYGVGYGAGAGAGYGAGAGSGAASGAGAGAGAGAGTGSSGFGPYVAHGGYSGYEYAWSSESDFGTGSGAGAGSGAGAGSGAGAGSGAGAGSGAGAGSGAGAGSGAGAGYGAGVGAGYGAAYGAGAGAGYGAGAGSGAASGAGAGSGAGAGSGAGAGSGAGAGSGAGAGSGAGAGSGAGAGSGAGAGSGAGAGSGAGAGSGAGAGYGAGAGAGYGAGAGSGAGSGAGAGSGAGAGSGAGAGSGAGAGSGAGAGSGAGSGSGAGAGSGAGAGSGAGAGYGAGVGAGYGAGYGAGAGAGYGAGAGSGAGSGAGAGSGAGAGYGAGAGAGYGAGYGAGAGAGYGAGAGTGAGSGAGAGSGAGAGSGAGAGSGAGAGSGAGAGSGAGAGSGAGSGSGAGAGSGAGAGSGAGAGSGAGAGSGAGAGSGAGAGYGAGAGAGYGAGYGAGAGAGYGAGAGSGAGSGAGAGSGAGAGSGAGAGSGAGAGYGAGYGAGAGSGAASGAGAGAGAGAGTGSSGFGPYVAHGGYSGYEYAWSSESDFGTGSGAGAGSGAGAGAGAGAGSGAGAGYGAGVGAGYGAGYGAGAGAGYGAGAGSGTGSGAGAGSGAGAGYGAGVGAGYGAGAGSGAAFGAGAGAGAGSGAGAGSGAGAGSGAGAGSGAGAGSGAGAGYGAGYGAGVGAGYGAGAGSGAASGAGAGSGAGAGSGAGAGSGAGAGSGAGAGSGAGAGYGAGVGAGYGAGYGAGAGAGYGAGAGSGAASGAGAGSGAGAGAGSGAGAGSGAGAGSGAGAGSGAGSGAGAGSGAGAGSGAGAGYGAGAGSGAASGAGAGAGAGAGTGSSGFGPYVANGGYSGYEYAWSSESDFGTGSGAGAGSGAGAGSGAGAGSGAGAGSGAGAGYGAGVGAGYGAGYGAGAGAGYGAGAGSGAGSGAGAGSGAGAGSGAGAGSGAGAGSGAGAGSGAGAGSGAGAGYGAGAGSGAASGAGAGSGAGAGSGAGAGSGAGAGSGAGAGSGAGAGSGAGAGYGAGVGAGYGVGYGAGAGAGYGAGAGSGAGSGAGAGSGAGAGSGAGAGSGAGAGSGAGSGAGAGSGAGAGSGAGAGSGAGSGAGAGSGAGAGYGVGYGAGAGAGYGAGAGSGAGSGAGAGSGAGAGSGAGAGSGAGSGAGAGSGAGAGSGAGAGSGAGAGYGAGVGAGYGVGYGAGAGAGYGAGAGSGAGSGAGAGSGAGAGSGAGAGSGAGAGSGAGAGSGAGAGSGAGAGSGAGSGAGAGSGAGAGSGAGAGSGAGAGSGAGSGAGAGSGAGAGSGAGAGSGAGAGYGAGVGAGYGVGYGAGVGAGYGAGAGSGAASGAGAGSGAGAGAGSGAGAGSGAGAGSGAGAGSGAGAGSGAGAGSGAGAGYGAGYGAGVGAGYGAGAGVGYGAGAGAGYGAGAGSGAASGAGAGAGSGAGAGTGAGAGSGAGAGYGAGAGSGAASGAGAGAGAGAGTGSSGFGPYVANGGYSGYEYAWSSESDFGTGSGAGAGSGAGAGSGAGAGSGAGAGSGAGAGYGAGVGAGYGAGAGSGAGSGAGAGSGAGAGSGAGAGSGAGAGSGAGAGYGAGAGSGTGSGAGAGSGAGAGSGAGAGSGAGAGSGAGAGSGAGAGSGVGAGYGVGYGAGAGAGYGVGYGAGAGAGYGAGAGSGTGSGAGAGSGAGAGSGAGAGSGAGAGSGAGAGSGAGAGSGAGAGYGAGVGAGYGVGYGAGAGAGYGAGAGSGAGSGAGAGSGAGAGSGAGAGSGAGAGSGAGSGAGAGSGAGAGSGAGAGSGAGSGAGAGSGAGAGYGVGYGAGAGAGYGAGAGSGAGSGAGAGSGAGAGSGAGAGSGAGSGAGAGSGAGAGSGAGAGSGAGAGYGAGVGAGYGVGYGAGAGAGYGAGAGSGAGSGAGAGSGAGAGSGAGAGSGAGAGSGAGAGSGAGAGSGAGAGSGAGSGAGAGSGAGAGSGAGAGSGAGAGYGAGVGAGYGVGYGAGAGAGYGAGAGSGAASGAGAGAGAGAGTGSSGFGPYVANGGYSGYEYAWSSESDFGTGSGAGAGSGAGAGSGAGAGYGAGYGAGVGAGYGAGAGVGYGAGAGAGYGAGAGSGAASGAGAGAGAGAGSGAGAGSGAGAGAGSGAGAGYGAGYGIGVGAGYGAGAGVGYGAGAGAGYGAGAGSGAASGAGAGSGAGAGSGAGAGSGAGAGSGAGAGSGAGAGSGAGAGYGAGYGAGVGAGYGAGAGVGYGAGAGAGYGAGAGSGAASGAGAGAGAGAGAGSGAGAGSGAGAGSGAGAGSGAGAGSGAGAGSGAGAGSGAGAGSGAGAGSGAGAGYGAGVGAGYGAGYGGAGAGYGAGAGSGAASGAGAGSGAGAGSGAGAGSGAGAGSGAGAGSGAGAGYGAGAGSGAASGAGAGAGAGAGTGSSGFGPYVNGGYSGYEYAWSSESDFGTGSGAGAGSGAGAGSGAGAGYGAGVGAGYGAGYGAGAGAGYGAGAGSGAASGAGAGSGAGAGSGAGAGSGAGAGSGAGSGAGAGSGAGAGSGAGAGSGAGAGSGAGAGSGAGAGYGAGVGAGYGAGYGAGAGAGYGAGAGSGAASGAGAGSGAGAGAGSGAGAGSGAGAGSGAGAGSGAGAGSGAGAGSGAGSGAGAGSGAGAGYGAGYGAGVGAGYGAGAGVGYGAGAGAGYGAGAGSGAASGAGAGSGSGAGSGAGAGSGAGAGSGAGAGAGSGAGAGSGAGAGSGAGAGYGAGYGAGAGSGAASGAGAGAGAGAGTGSSGFGPYVANGGYSGYEYAWSSESDFGTGSGAGAGSGAGAGSGAGAGYGAGVGAGYGAGYGAGAGAGYGAGAGSGAGSGAGAGSGAGAGSGAGAGSGAGAGSGAGAGSGAGAGSGAGAGSGAGAGYGAGYGAGAGAGYGAGAGVGYGAGAGAGYGAGAGSGAGSGAGAGSGSGAGAGSGSGAGSGAGAGSGAGAGSGAGAGSGAGAGSGAGAGSGAGAGSGAGAGYGAGYGIGVGAGYGAGAGVGYGAGAGAGYGAGAGSGAASGAGAGSGAGAGSGAGAGSGAGAGSGAGAGSGAGAGSGAGAGSGAGAGSGAGAGSGAGAGYGAGAGVGYGAGAGSGAASGAGAGSGAGAGSGAGAGSGAGAGSGAGAGSGAGAGSGAGAGSGAGSGAGAGSGAGAGYGAGYGAGVGAGYGAGAGYGAGYGVGAGAGYGAGAGSGAGSGAGAGSGAGAGSGAGAGSGAGAGSGAGAGSGAGSGAGAGYGAGAGAGYGAGAGAGYGAGAGSGAASGAGAGAGAGSGAGAGSGAGAGSGAGSGAGAGSGAGAGYGAGAGSGAASGAGAGSGAGAGAGAGAGAGSGAGAGSGAGAGYGAGAGSGAASGAGAGAGAGTGSSGFGPYVANGGYSRREGYEYAWSSKSDFETGSGAASGAGAGAGSGAGAGSGAGAGSGAGAGSGAGAGGSVSYGAGRGYGQGAGSAASSVSSASSRSYDYSRRNVRKNCGIPRRQLVVKFRALPCVNC

SEQ ID NO: 2 - protein, 5242 aa, Bombyx mori
NINDFDEDYFGSDVTVQSSNTTDEIIRDASGAVIEEQITTKKMQRKNKNHGILGKNEKMIKTFVITTDSDGNESIVEEDVLMKTLSDGTVAQSYVAADAGAYSQSGPYVSNSGYSTHQGYTSDFSTSAAVGAGAGAGAAAGSGAGAGAGYGAASGAGAGAGAGAGAGYGTGAGAGAGAGYGAGAGAGAGAGYGAGAGAGAGAGYGAGAGAGAGAGYGAGAGAGAGAGYGAGAGAGAGAGYGAASGAGAGAGYGQGVGSGAASGAGAGAGAGSAAGSGAGAGAGTGAGAGYGAGAGAGAGAGYGAASGTGAGYGAGAGAGYGGASGAGAGAGAGAGAGAGAGYGTGAGYGAGAGAGAGAGAGAGYGAGAGAGYGAGYGVGAGAGYGAGYGAGAGSGAASGAGSGAGAGSGAGAGSGAGAGSGAGAGSGAGAGSGAGAGSGAGAGSGAGAGSGTGAGSGAGAGYGAGAGAGYGAGAGSGAASGAGAGSGAGAGSGAGAGSGAGAGSGAGAGSGAGAGYGAGAGAGYGAGAGAGYGAGAGVGYGAGAGSGAASGAGAGSGAGAGSGAGAGSGAGAGSGAGAGSGAGAGSGAGAGSGAGAGSGAGAGSGAGVGYGAGVGAGYGAGYGAGAGAGYGAGAGSGAASGAGAGAGAGAGTGSSGFGPYVANGGYSRSDGYEYAWSSDFGTGSGAGAGSGAGAGSGAGAGSGAGAGSGAGAGSGAGAGYGAGVGVGYGAGYGAGAGAGYGAGAGSGAASGAGAGSGAGAGSGAGAGSGAGAGSGAGAGSGAGAGSGAGAGSGAGAGSGAGAGSGAGAGSGAGVGSGAGAGSGAGAGVGYGAGAGVGYGAGAGSGAASGAGAGSGAGAGSGAGAGSGAGAGSGAGAGSGAGAGSGAGAGSGAGAGSGAGAGSGAGVGYGAGVGAGYGAGYGAGAGAGYGAGAGSGAASGAGAGSGAGAGSGAGAGSGAGAGSGAGAGSGAGAGSGAGAGSGAGAGSGAGAGSGAGAGSGAGAGSGAGAGYGAGAGAGYGAGYGAGAGAGYGAGAGSGAASGAGSGAGAGSGAGAGAGSGAGAGSGAGAGSGAGAGSGAGAGSGAGAGSGAGAGYGAGVGAGYGAGYGAGAGAGYGAGAGSGAASGAGAGSGAGAGSGAGAGSGAGAGSGAGAGSGAGAGSGAGAGSGAGVGYGAGYGAGAGAGYGAGAGSGAASGAGAGAGAGAGTGSSGFGPYVAHGGYSGYEYAWSSESDFGTGSGAGAGSGAGAGSGAGAGSGAGAGSGAGYGAGVGAGYGAGYGAGAGAGYGAGAGSGAGSGAGAGSGAGAGSGAGAGSGAGAGSGAGAGSGAGAGSGAGAGSGAGAGSGAGAGYGAGYGAGAGAGYGAGAGSGAGSGAGAGSGAGAGSGAGAGSGAGAGSGAGAGSGAGAGSGAGAGSGAGAGYGAGVGAGYGAGYGAGAGAGYGAGAGSGAGSGAGAGSGAGAGSGAGAGSGAGVGSGAGAGSGAGAGSGAGAGSGAGAGYGAGYGAGAGAGYGAGAGSGAGSGAGAGSGAGAGSGAGAGSGAGAGSGAGAGSGAGAGSGAGAGSGAGVGYGAGVGAGYGAGYGAGAGAGYGAGAGSGAASGAGAGAGAGAGTGSSGFGPYVANGGYSGYEYAWSSESDFGTGSGAGAGSGAGAGSGAGAGSGAGAGSGAGAGYGAGYGAGAGAGYGAGAGSGAGSGAGAGSGAGAGSGAGAGSGAGAGSGAGAGSGAGAGSGAGAGSGAGSGSGAGAGSGAGAGSGAGAGYGAGVGAGYGVGYGAGAGAGYGAGAGSGAASGAGAGAGAGAGTGSSGFGPYVAHGGYSGYEYAWSSESDFGTGSGAGAGSGAGAGSGAGAGSGAGAGSGAGAGSGAGAGSGAGAGYGAGVGAGYGAAYGAGAGAGYGAGAGSGAASGAGAGSGAGAGSGAGAGSGAGAGSGAGAGSGAGAGSGAGAGSGAGAGSGAGAGSGAGAGSGAGAGYGAGAGAGYGAGAGSGAGSGAGAGSGAGAGSGAGAGSGAGAGSGAGAGSGAGSGSGAGAGSGAGAGSGAGAGYGAGVGAGYGAGYGAGAGAGYGAGAGSGAGSGAGAGSGAGAGYGAGAGAGYGAGYGAGAGAGYGAGAGTGAGSGAGAGSGAGAGSGAGAGSGAGAGSGAGAGSGAGAGSGAGSGSGAGAGSGAGAGSGAGAGSGAGAGSGAGAGSGAGAGYGAGAGAGYGAGYGAGAGAGYGAGAGSGAGSGAGAGSGAGAGSGAGAGSGAGAGYGAGYGAGAGSGAASGAGAGAGAGAGTGSSGFGPYVAHGGYSGYEYAWSSESDFGTGSGAGAGSGAGAGAGAGAGSGAGAGYGAGVGAGYGAGYGAGAGAGYGAGAGSGTGSGAGAGSGAGAGYGAGVGAGYGAGAGSGAAFGAGAGAGAGSGAGAGSGAGAGSGAGAGSGAGAGSGAGAGYGAGYGAGVGAGYGAGAGSGAASGAGAGSGAGAGSGAGAGSGAGAGSGAGAGSGAGAGYGAGVGAGYGAGYGAGAGAGYGAGAGSGAASGAGAGSGAGAGAGSGAGAGSGAGAGSGAGAGSGAGSGAGAGSGAGAGSGAGAGYGAGAGSGAASGAGAGAGAGAGTGSSGFGPYVANGGYSGYEYAWSSESDFGTGSGAGAGSGAGAGSGAGAGSGAGAGSGAGAGYGAGVGAGYGAGYGAGAGAGYGAGAGSGAGSGAGAGSGAGAGSGAGAGSGAGAGSGAGAGSGAGAGSGAGAGYGAGAGSGAASGAGAGSGAGAGSGAGAGSGAGAGSGAGAGSGAGAGSGAGAGYGAGVGAGYGVGYGAGAGAGYGAGAGSGAGSGAGAGSGAGAGSGAGAGSGAGAGSGAGSGAGAGSGAGAGSGAGAGSGAGSGAGAGSGAGAGYGVGYGAGAGAGYGAGAGSGAGSGAGAGSGAGAGSGAGAGSGAGSGAGAGSGAGAGSGAGAGSGAGAGYGAGVGAGYGVGYGAGAGAGYGAGAGSGAGSGAGAGSGAGAGSGAGAGSGAGAGSGAGAGSGAGAGSGAGAGSGAGSGAGAGSGAGAGSGAGAGSGAGAGSGAGSGAGAGSGAGAGSGAGAGSGAGAGYGAGVGAGYGVGYGAGVGAGYGAGAGSGAASGAGAGSGAGAGAGSGAGAGSGAGAGSGAGAGSGAGAGSGAGAGSGAGAGYGAGYGAGVGAGYGAGAGVGYGAGAGAGYGAGAGSGAASGAGAGAGSGAGAGTGAGAGSGAGAGYGAGAGSGAASGAGAGAGAGAGTGSSGFGPYVANGGYSGYEYAWSSESDFGTGSGAGAGSGAGAGSGAGAGSGAGAGSGAGAGYGAGVGAGYGAGAGSGAGSGAGAGSGAGAGSGAGAGSGAGAGSGAGAGYGAGAGSGTGSGAGAGSGAGAGSGAGAGSGAGAGSGAGAGSGAGAGSGVGAGYGVGYGAGAGAGYGVGYGAGAGAGYGAGAGSGTGSGAGAGSGAGAGSGAGAGSGAGAGSGAGAGSGAGAGSGAGAGYGAGVGAGYGVGYGAGAGAGYGAGAGSGAGSGAGAGSGAGAGSGAGAGSGAGAGSGAGSGAGAGSGAGAGSGAGAGSGAGSGAGAGSGAGAGYGVGYGAGAGAGYGAGAGSGAGSGAGAGSGAGAGSGAGAGSGAGSGAGAGSGAGAGSGAGAGSGAGAGYGAGVGAGYGVGYGAGAGAGYGAGAGSGAGSGAGAGSGAGAGSGAGAGSGAGAGSGAGAGSGAGAGSGAGAGSGAGSGAGAGSGAGAGSGAGAGSGAGAGYGAGVGAGYGVGYGAGAGAGYGAGAGSGAASGAGAGAGAGAGTGSSGFGPYVANGGYSGYEYAWSSESDFGTGSGAGAGSGAGAGSGAGAGYGAGYGAGVGAGYGAGAGVGYGAGAGAGYGAGAGSGAASGAGAGAGAGAGSGAGAGSGAGAGAGSGAGAGYGAGYGIGVGAGYGAGAGVGYGAGAGAGYGAGAGSGAASGAGAGSGAGAGSGAGAGSGAGAGSGAGAGSGAGAGSGAGAGYGAGYGAGVGAGYGAGAGVGYGAGAGAGYGAGAGSGAASGAGAGAGAGAGAGSGAGAGSGAGAGSGAGAGSGAGAGSGAGAGSGAGAGSGAGAGSGAGAGSGAGAGYGAGVGAGYGAGYGGAGAGYGAGAGSGAASGAGAGSGAGAGSGAGAGSGAGAGSGAGAGSGAGAGYGAGAGSGAASGAGAGAGAGAGTGSSGFGPYVNGGYSGYEYAWSSESDFGTGSGAGAGSGAGAGSGAGAGYGAGVGAGYGAGYGAGAGAGYGAGAGSGAASGAGAGSGAGAGSGAGAGSGAGAGSGAGSGAGAGSGAGAGSGAGAGSGAGAGSGAGAGSGAGAGYGAGVGAGYGAGYGAGAGAGYGAGAGSGAASGAGAGSGAGAGAGSGAGAGSGAGAGSGAGAGSGAGAGSGAGAGSGAGSGAGAGSGAGAGYGAGYGAGVGAGYGAGAGVGYGAGAGAGYGAGAGSGAASGAGAGSGSGAGSGAGAGSGAGAGSGAGAGAGSGAGAGSGAGAGSGAGAGYGAGYGAGAGSGAASGAGAGAGAGAGTGSSGFGPYVANGGYSGYEYAWSSESDFGTGSGAGAGSGAGAGSGAGAGYGAGVGAGYGAGYGAGAGAGYGAGAGSGAGSGAGAGSGAGAGSGAGAGSGAGAGSGAGAGSGAGAGSGAGAGSGAGAGYGAGYGAGAGAGYGAGAGVGYGAGAGAGYGAGAGSGAGSGAGAGSGSGAGAGSGSGAGSGAGAGSGAGAGSGAGAGSGAGAGSGAGAGSGAGAGSGAGAGYGAGYGIGVGAGYGAGAGVGYGAGAGAGYGAGAGSGAASGAGAGSGAGAGSGAGAGSGAGAGSGAGAGSGAGAGSGAGAGSGAGAGSGAGAGSGAGAGYGAGAGVGYGAGAGSGAASGAGAGSGAGAGSGAGAGSGAGAGSGAGAGSGAGAGSGAGAGSGAGSGAGAGSGAGAGYGAGYGAGVGAGYGAGAGYGAGYGVGAGAGYGAGAGSGAGSGAGAGSGAGAGSGAGAGSGAGAGSGAGAGSGAGSGAGAGYGAGAGAGYGAGAGAGYGAGAGSGAASGAGAGAGAGSGAGAGSGAGAGSGAGSGAGAGSGAGAGYGAGAGSGAASGAGAGSGAGAGAGAGAGAGSGAGAGSGAGAGYGAGAGSGAASGAGAGAGAGTGSSGFGPYVANGGYSRREGYEYAWSSKSDFETGSGAASGAGAGAGSGAGAGSGAGAGSGAGAGSGAGAGGSVSYGAGRGYGQGAGSAASSVSSASSRSYDYSRRNVRKNCGIPRRQLVVKFRALPCVNC

SEQ ID NO: 3 - DNA, 18763 bp, Bombyx mori
  source 1..18763: mol_type = genomic DNA
aatcagcttctttagaactaaaatatcatttttttcgtaatttttttaatgaaaaatgctctagtgttatacctttccaaaatcaccattaattaggtagtgtttaagcttgttgtacaaaactgccacacgcatttttttctccactgtaggttgtagttacgcgaaaacaaaatcgttctgtgaaaattcaaacaaaaatattttttcgtaaaaacacttatcaatgagtaaagtaacaattcatgaataatttcatgtaaaaaaaaaatactagaaaaggaatttttcattacgagatgcttaaaaatctgtttcaaggtagagatttttcgatatttcggaaaattttgtaaaactgtaaatccgtaaaattttgctaaacatatattgtgttgttttggtaagtattgacccaagctatcacctcctgcagtatgtcgtgctaattactggacacattgtataacagttccactgtattgacaataataaaacctcttcattgacttgagaatgtctggacagatttggctttgtatttttgatttacaaatgtttttttggtgatttacccatccaaggcattctccaggatggttgtggcatcacgccgattggcaaacaaaaactaaaatgaaactaaaaagaaacagtttccgctgtcccgttcctctagtgggagaaagcatgaagtaagttctttaaatattacaaaaaaattgaacgatattataaaattctttaaaatattaaaagtaagaacaataagatcaattaaatcataattaatcacattgttcatgatcacaatttaatttacttcatacgttgtattgttatgttaaataaaaagattaatttctatgtaattgtatctgtacaatacaatgtgtagatgtttattctatcgaaagtaaatacgtcaaaactcgaaaattttcagtataaaaaggttcaactttttcaaatcagcatcagttcggttccaactctcaagatgagagtcaaaacctttgtgatcttgtgctgcgctctgcaggtgagttaattattttactattatttcagaaggtggccagacgatatcacgggccacctgataataagtggtcgccaaaacgcacagatatcgtaaattgtgccatttgatttgtcacgcccgggggggctacggaataaactacatttatttatttaaaaaatgaaccttagattatgtaacttgtgatttatttgcgtcaaaagtaggcaagatgaatctatgtaaatacctgggcagacttgcaatatcctatttcaccggtaaatcagcattgcaatatgcaatgcatattcaacaatatgtaaaacaattcgtaaagcatcattagaaaatagacgaaagaaattgcataaaattataaccgcattattaatttattatgatatctattaacaattgctattgcctttttttcgcaaattataatcattttcataacctcgaggtagcattctgttacattttaatacattggtatgtgattataacacgagctgcccactgagtttctcgccagatcttctcagtgggtcgcgttaccgatcacgtgatagattctatgaagcactgctcttgttagggctagtgttagcaaattctttcaggttgagtctgagagctcacctacccatcggagcgtagctggaataggctaccagctaataggtagggaaaacaaagctcgaaacaagctcaagtaataacaacataatgtgaccataaaatctcgtggtgtatgagatacaattatgtactttcccacaaatgtttacataattagaatgttgttcaacttgcctaacgccccagctagaacattcaattattactattaccactactaaggcagtatgtcctaactcgttccagatcagcgctaacttcgattgaatgtgcgaaatttatagctcaatattttagcacttatcgtattgatttaagaaaaaattgttaacattttgtttcagtatgtcgcttatacaaatgcaaacatcaatgattttgatgaggactattttgggagtgatgtcactgtccaaagtagtaatacaacagatgaaataattagagatgcatctggggcagttatcgaagaacaaattacaactaaaaaaatgcaacggaaaaataaaaaccatggaatacttggaaaaaatgaaaaaatgatcaagacgttcgttataaccacggattccgacggtaacgagtccattgtagaggaagatgtgctcatgaagacactttccgatggtactgttgctcaaagttatgttgctgctgatgcgggagcatattctcagagcgggccatacgtatcaaacagtggatacagcactcatcaaggatatacgagcgatttcagcactagtgctgcagtcggtgcaggagctggtgcaggtgctgccgctggttctggtgcgggtgccggagctggttatggagctgcttctggtgctggtgccggtgctggggctggtgccggagctggttatggaactggtgcaggtgcaggtgccggagctggttatggagctggtgcaggtgcaggtgccggagctggttatggggctggtgcaggtgcaggtgccggagctggttatggagctggtgcaggtgcaggtgccggagctggttatggggctggtgcaggtgcaggtgccggagctggttatggagctggtgcgggtgccggtgccggggctggttatggagctgcctctggtgctggtgctggcgctgggtacggacaaggagtaggaagcggagctgcttctggagctggtgcaggtgcaggagcaggttctgccgctggttctggggcaggtgccggtgctggtaccggtgctggtgcaggttacggagctggtgcaggtgccggtgccggagctggttatggagctgcctctggtactggagcaggttatggagctggtgccggagctggttacggaggtgcctctggtgctggtgctggtgccggtgctggggctggagccggtgctggtgcaggttatggaactggcgctggatacggagcaggagccggagcaggagccggagcaggagctggtgctggatacggagcaggagctggtgctggatacggagcaggatatggagtaggagctggtgctggatacggagcaggatacggagcaggagctggaagcggagctgcctctggtgctggttcaggtgccggtgctggttcaggtgccggtgctggttcaggtgccggtgctggttcaggtgccggtgccggttcaggtgctggtgctggttcaggtgctggtgctggttcaggtgctggtgcaggttcaggtgctggtgctggttcaggtactggtgctggttcaggagctggtgctggatacggagcaggagctggtgctggatacggagcaggagcaggaagtggagctgcctctggtgccggtgctggttcaggtgcaggtgctggttcaggtgctggtgctggttcaggtgctggtgctggttcaggtgctggtgctggttcaggagctggtgctggatacggagcaggagctggtgctggatacggagcaggagctggtgctggatacggagcaggagctggcgttggatacggagcaggagctggaagcggagctgcctctggtgctggtgctggttcaggagccggtgctggttcaggtgctggtgctggttcaggtgctggtgctggttcaggtgctggtgctggttcaggtgccggtgctggttcaggtgctggtgctggttcaggagctggtgctggttcaggtgctggtgctggttcaggagctggagttggatacggagcaggagttggtgctggatacggagcaggatatggagcaggagctggtgctggatacggagcaggagcaggaagcggagctgcctctggtgctggtgccggtgctggagctggtgcaggaacaggctcttctggatttggaccatatgtagcaaatggcggatatagcagaagtgatggctacgaatacgcttggtcgtctgactttggaactggaagcggagctggtgctggttcaggtgctggtgctggttcaggtgctggcgctggctcaggtgctggtgctggttcaggtgctggtgctggttcaggagctggagctggatacggagcaggagttggtgttggatacggagcaggatatggagcaggagctggtgctggatacggagcaggagcaggaagcggagctgcctctggtgccggtgctggttcaggtgctggtgctggttcaggtgccggtgctggttcaggtgctggtgctggttcaggtgccggtgctggttcaggtgctggtgctggctcaggtgccggtgctggttcaggtgctggtgctggttcaggtgccggtgctggttcaggtgctggtgctggttcaggtgctggtgttggctcaggtgctggtgctggttcaggtgctggtgctggcgttggatacggagcaggagctggcgttggatacggagcaggagctggaagcggagctgcctctggtgctggtgctggttcaggagccggtgctggttcaggtgctggtgctggttcaggtgctggtgctggttcaggtgctggtgctggttcaggtgccggtgctggttcaggtgctggtgctggttcaggagctggtgctggttcaggtgctggtgctggttcaggagctggagttggatacggagcaggagttggtgctggatacggagcaggatatggagcaggagctggtgctggatacggagcaggagcaggaagcggagctgcctcaggtgccggtgctggttcaggtgctggtgctggttcaggtgccggtgctggttcaggtgctggtgctggttcaggtgctggtgctggttcaggtgctggtgctggttcaggtgctggtgctggttcaggtgctggtgctggttcaggtgctggtgctggctcaggtgctggagctggttcaggtgctggtgctggttcaggagctggagctggatacggagcaggagctggtgctggatacggagcaggatatggagcaggagctggtgctggatacggagcaggagctggaagcggagctgcctctggtgctggttcaggtgccggtgctggttcaggtgccggtgctggtgctggttcaggtgctggtgctggttcaggtgctggtgctggttcaggtgctggtgctggctcaggtgctggagctggttcaggtgctggtgctggttcaggagctggagctggatacggagcaggagttggtgctggatacggagcaggatatggagcaggagctggtgctggatacggagcaggagcaggaagcggagctgcctctggtgccggtgctggttcaggtgctggagctggttcaggtgccggtgctggttcaggtgctggtgctggttcaggagctggtgctggttcaggagctggtgctggttcaggtgctggtgctggttcaggagctggagttggatacggagcaggatatggagcaggagctggtgctggatacggagcaggagcaggaagcggagctgcctctggtgctggtgccggtgctggagctggtgcaggaacaggctcttctggatttggaccatatgtagcacatggcggatatagcggctacgaatacgcttggtcgtcagaatctgactttggaactggaagcggagctggtgctggttcaggtgctggtgctggttcaggtgctggtgctggctcaggtgctggtgctggttcaggagctggatacggagcaggagttggtgctggatacggagcaggatatggagcaggagctggtgctggatacggagcaggagcaggaagcggagctggctcaggtgctggtgctggttcaggagctggagctggttcaggtgccggtgctggttcaggtgctggtgctggttcaggagctggtgctggttcaggtgctggtgctggttcaggagctggtgctggttcaggtgccggtgctggttcaggtgctggtgctggatacggagcaggatatggagcaggagctggtgctggatacggagcaggagcaggaagcggagctggctcaggtgctggtgctggttcaggtgctggtgctggttcaggagctggagctggttcaggtgccggtgctggttcaggtgctggtgctggttcaggtgctggtgctggctcaggtgctggtgctggttcaggagctggagctggatacggagcaggagttggtgctggatacggagcaggatatggagcaggagctggtgctggatacggagcaggagcaggaagcggagctggctcaggtgctggtgctggttcaggagctggagctggttcaggtgctggtgctggttcaggtgccggtgttggttcaggtgctggtgctggttcaggagctggtgctggttcaggtgccggtgctggttcaggtgctggtgctggatacggagcaggatatggagcaggagctggtgctggatacggagcaggagcaggaagcggagctggctcaggtgctggtgctggttcaggtgctggtgctggttcaggagctggagctggttcaggtgccggtgctggttcaggtgctggtgctggttcaggagctggtgctggttcaggtgctggtgctggttcaggagctggagttggatacggagcaggagttggtgctggatacggagcaggatatggagcaggagctggtgctggatacggagcaggagcaggaagcggagctgcctctggtgctggtgccggtgctggagctggtgcaggaacaggctcttctggatttggaccatatgtagcaaatggcggatatagcggctacgaatacgcttggtcgtcagaatctgactttggaactggaagcggagctggtgctggttcaggtgctggtgctggttcaggtgctggtgctggctcaggtgctggtgctggttcaggagctggagctggatacggagcaggatatggagcaggagctggtgctggatacggagcaggagcaggaagcggagctggctcaggtgctggtgctggttcaggagctggagctggttcaggtgccggtgctggttcaggtgctggtgctggttcaggtgccggtgctggttcaggtgctggtgctggttcaggagctggtgctggttcaggtgccggttctggttcaggagctggtgctggttcaggtgctggtgctggttcaggagctggagctggatacggagcaggagttggtgctggatacggagtaggatatggagcaggagctggtgctggatacggagcaggagcaggaagcggagctgcctctggtgctggtgccggtgctggagctggtgcaggaacaggctcttctggatttggaccatatgtagcacatggcggatatagcggctacgaatacgcttggtcgtcagaatctgactttggaactggaagcggagctggtgctggttcaggtgctggtgctggttcaggtgctggtgctggctcaggtgctggtgctggttcaggagctggtgctggttcaggtgctggtgctggttcaggagctggagctggatacggagcaggagttggtgctggatacggagcagcatatggagcaggagctggtgctggatacggagctggagcaggaagcggagctgcctctggtgccggtgctggttcaggtgctggtgctggttcaggtgccggtgctggttcaggtgctggtgctggttcaggtgctggtgctggttcaggtgctggtgctggttcaggtgctggtgctggttcaggagctggtgctggttcaggagctggtgctggttcaggtgccggtgctggttcaggagctggagcaggatatggagcaggagctggtgctggatacggagcaggagcaggaagcggagctggctcaggtgctggtgctggttcaggtgctggtgctggttcaggagctggagctggttcaggtgccggtgctggttcaggtgctggtgctggttcaggtgccggttctggttcaggagctggtgctggttcaggtgctggtgctggttcaggagctggagctggatacggagcaggagttggtgctggatacggagcaggatatggagcaggagctggtgctggatacggagcaggagcaggaagcggagctggctcaggtgccggtgctggttcaggagctggagcaggatatggagcaggagctggtgctggatacggagcaggatatggagcaggagctggtgctggatacggagcaggagcaggaaccggagctggctcaggtgctggtgctggttcaggtgctggtgctggttcaggtgctggtgctggttcaggagctggagctggttcaggtgccggtgctggttcaggtgctggtgctggttcaggtgccggttctggttcaggtgctggtgctggttcaggagctggagctggttcaggtgccggtgctggttcaggtgctggtgctggttcaggtgctggtgctggttcaggagctggagctggatacggagcaggagctggtgctggatacggagcaggatatggagcaggagctggtgctggatacggagcaggagcaggaagcggtgctggttcaggtgctggtgctggttcaggtgctggtgctggttcaggtgctggtgctggttcaggagctggtgctggatatggagctggatacggagcaggagctggaagcggagctgcctctggtgctggtgccggtgctggagctggtgcaggaacaggctcttctggatttggaccatatgtagcacatggcggatatagcggctacgaatacgcttggtcgtcagaatctgactttggaactggaagcggagctggtgctggttcaggtgctggtgctggcgcaggtgctggtgctggttcaggagctggagctggatacggagcaggagttggtgctggatacggagcaggatatggagcaggagctggtgctggatacggagcaggagcaggaagcggaactggctcaggtgctggtgctggttcaggagctggagctggatacggagcaggagttggtgctggatacggagcaggagcaggaagcggagctgcctttggtgccggtgctggtgctggtgctggttcaggtgccggtgctggttcaggtgctggtgctggttcaggtgctggtgctggttcaggtgctggtgctggttcaggagctggtgctggatacggagcagggtacggagcaggagttggtgctggatacggagcaggagctggaagcggagctgcctctggtgccggtgctggttcaggtgctggtgctggttcaggtgccggtgctggttcaggtgctggtgctggctcaggtgctggtgctggttcaggagctggagctggatacggagcaggagttggtgctggatacggagcaggatatggagcaggagctggtgctggatacggagctggagcaggaagcggagctgcctctggtgccggtgctggttcaggtgctggtgctggtgctggttcaggtgccggtgctggttcaggtgctggtgctggttcaggtgctggtgctggttcaggtgctggttcaggtgctggtgctggttcaggtgccggtgctggttcaggagctggtgctggatacggagcaggagcaggaagcggagctgcctctggtgctggtgccggtgctggagctggtgcaggaacaggctcttctggatttggaccatatgtagcaaatggcggatatagcggctacgaatacgcttggtcgtcagaatctgactttggaactggaagcggagctggtgctggttcaggtgctggtgctggttcaggtgctggtgctggctcaggtgctggtgctggttcaggagctggagctggatacggagcaggagttggtgctggatacggagcaggatatggagcaggagctggtgctggatacggagcaggagcaggaagcggagctggctcaggtgctggtgctggttcaggagctggagctggttcaggtgccggtgctggttcaggtgctggtgctggttcaggtgccggtgctggttcaggtgctggggctggttcaggagctggtgctggatacggagcaggagcaggaagcggagctgcctctggtgccggtgctggttcaggtgctggtgctggttcaggtgccggtgctggttcaggtgctggtgctggttcaggagctggtgctggttcaggtgctggtgctggttcaggagctggagctggatacggagcaggagttggtgctggatacggagtaggatatggagcaggagctggtgctggatacggagcaggagcaggaagcggagctggctcaggtgctggtgctggttcaggtgctggtgctggttcaggtgccggtgctggttcaggtgctggtgctggttcaggtgccggttcaggtgctggtgctggttcaggagctggtgctggttcaggtgctggtgctggttcaggtgctggttcaggtgctggtgctggctcaggtgctggtgctggatacggagtaggatatggagcaggagctggtgctggatacggagcaggagcaggaagcggagctggctcaggtgctggtgctgggtcaggtgccggtgctggttcaggtgctggtgctggttcaggtgccggttcaggtgctggtgctggttcaggagctggtgctggttcaggtgctggtgctggttcaggagctggagctggatacggagcaggagttggtgctggatacggagtaggatatggagcaggagctggtgctggatacggagcaggagcaggaagcggagctggctcaggtgctggtgctggttcaggtgctggtgctggttcaggtgccggtgctggttcaggtgctggtgctggttcaggagctggtgctggttcaggtgccggtgctggttcaggtgctggtgctggttcaggtgccggttcaggtgctggtgctggttcaggagctggtgctggttcaggtgccggtgctggttcaggtgctggtgctggttcaggtgccggttcaggtgctggtgctggttcaggagctggtgctggttcaggtgctggtgctggttcaggagctggagctggatacggagcaggagttggtgctggatacggagtaggatatggagcaggagttggtgctggatacggagcaggagcaggaagcggagctgcctctggtgccggtgctggttcaggtgctggtgctggtgctggttcaggtgccggtgctggttcaggtgctggtgctggttcaggtgctggtgctggttcaggtgctggtgctggttcaggtgctggtgctggttcaggagctggtgctggatacggagcagggtacggagcaggagttggtgctggatacggagcaggagctggcgttggatacggagcaggagctggcgctggatacggagcaggagctggaagcggagctgcctctggtgccggtgctggtgctggttcaggtgccggtgctggtacaggtgctggggctggttcaggagctggtgctggatacggagcaggagcaggaagcggagctgcctctggtgctggtgccggtgctggagctggtgcaggaacaggctcttctggatttggaccatatgtagcaaatggcggatatagcggctacgaatacgcttggtcgtcagaatctgactttggaactggaagcggagctggtgctggttcaggtgctggtgctggttcaggtgctggtgctggctcaggtgctggtgctggttcaggagctggagctggatacggagcaggagttggtgctggatacggagcaggagcaggaagcggagctggctcaggtgctggtgctggttcaggagctggagctggttcaggtgctggtgctggttcaggagctggtgctggttcaggagctggagctggatacggagcaggagcaggaagcggaactggctcaggtgctggtgctggttcaggtgctggtgctggttcaggtgccggtgctggttcaggtgctggtgctggttcaggagctggtgctggttcaggtgctggtgctggttcaggagttggtgctggatacggagtaggatatggagcaggagctggtgctggatacggagtaggatatggagcaggagctggtgctggatacggagcaggagcaggaagcggaactggctcaggtgctggtgctggttcaggtgctggtgctggttcaggtgccggtgctggttcaggtgctggtgctggttcaggagctggtgctggttcaggtgctggtgctggttcaggagctggagctggatacggagcaggagttggtgctggatacggagtaggatatggagcaggagctggtgctggatacggagcaggagcaggaagcggagctggctcaggtgctggtgctggttcaggtgctggtgctggttcaggtgccggtgctggttcaggtgctggtgctggttcaggtgccggttcaggtgctggtgctggttcaggagctggtgctggttcaggtgctggtgctggttcaggtgctggttcaggtgctggtgctggctcaggtgctggtgctggatacggagtaggatatggagcaggagctggtgctggatacggagcaggagcaggaagcggagctggctcaggtgctggtgctgggtcaggtgccggtgctggttcaggtgctggtgctggttcaggtgccggttcaggtgctggtgctggttcaggagctggtgctggttcaggtgctggtgctggttcaggagctggagctggatacggagcaggagttggtgctggatacggagtaggatatggagcaggagctggtgctggatacggagcaggagcaggaagcggagctggctcaggtgctggtgctggttcaggtgctggtgctggttcaggtgccggtgctggttcaggtgctggtgctggttcaggagctggtgctggttcaggtgccggtgctggttcaggtgctggtgctggttcaggtgccggttcaggtgctggtgctggttcaggagctggtgctggttcaggtgctggtgctggttcaggagctggagctggatacggagcaggagttggtgctggatacggagtaggatatggagcaggagctggtgctggatacggagcaggagcaggaagcggagctgcctctggtgctggtgccggtgctggagctggtgcaggaacaggctcttctggatttggaccatatgtagcaaatggcggatatagcggctacgaatacgcttggtcgtcagaatctgactttggaactggaagcggagctggtgctggttcaggtgctggtgctggttcaggagctggtgctggatacggagcagggtacggagcaggagttggtgctggatacggagcaggagctggcgttggatacggagcaggagctggcgctggatacggagcaggagctggaagcggagctgcctctggtgccggtgctggtgccggtgctggtgctggttcaggtgccggtgctggttcaggtgctggtgctggtgctggttcaggagctggtgctggatacggagcagggtacggaataggagttggtgctggatacggagcaggagctggcgttggatacggagcaggagctggcgctggatacggagcaggagctggaagcggagctgcctctggtgccggtgctggttcaggtgctggtgctggttcaggtgctggtgctggttcaggtgctggtgctggttcaggtgctggtgctggttcaggtgctggtgctggttcaggagctggtgctggatacggagcagggtacggagcaggagttggtgctggatacggagcaggagctggcgttggatacggagcaggagctggcgctggatacggagcaggagctggaagcggagctgcctctggtgccggtgctggtgccggtgctggtgctggtgctggttcaggtgccggtgctggttcaggtgctggtgctggttcaggtgctggtgctggttcaggagctggtgctggttcaggtgctggtgctggttcaggtgctggtgctggttcaggtgctggtgctggctcaggtgctggtgctggttcaggagctggagctggatacggagcaggagttggtgctggatacggagcaggatatggaggagctggtgctggatacggagcaggagcaggaagcggagctgcctctggtgccggtgctggttcaggtgctggtgctggttcaggagctggtgctggttcaggtgctggtgctggttcaggtgctggggctggttcaggtgctggtgctggatacggagcaggagcaggaagcggagctgcctctggtgctggtgccggtgctggagctggtgcaggaacaggctcttctggatttggaccatatgtaaatggcggatatagcggctacgaatacgcttggtcgtcagaatctgactttggaactggaagcggagctggtgctggctcaggtgctggtgctggttcaggagctggagctggatacggagcaggagttggtgctggatacggagcaggatatggagcaggagctggtgctggatacggagcaggagcaggaagcggagctgcctctggtgccggtgctggttcaggtgctggtgctggttcaggtgccggtgctggttcaggtgctggtgctggttcaggtgctggttcaggtgctggtgctggttcaggtgctggtgctggttcaggtgctggtgctggttcaggtgctggtgctggttcaggtgctggtgctggttcaggagctggagctggatacggagcaggagttggtgctggatacggagcaggatatggagcaggagctggtgctggatacggagcaggagcaggaagcggagctgcytctggcgccggtgctggttcaggtgctggtgctggtgctggttcaggtgccggtgctggttcaggtgctggtgctggttcaggtgctggtgctggttcaggtgctggtgctggttcaggtgctggtgctggttcaggtgctggttcaggtgctggtgctggttcaggagctggtgctggatacggagcagggtacggagcaggagttggtgctggatacggagcaggagctggcgttggatacggagcaggagctggcgctggatacggagcaggagctggaagcggagctgcctctggtgccggtgctggttcaggttctggtgctggttcaggtgccggtgctggttcaggtgctggtgctggttcaggtgctggtgctggtgctggttcaggtgctggggctggttcaggagctggtgctggttcaggagctggtgctggatacggagcagggtacggagcaggagcaggaagcggagctgcctctggtgctggtgccggtgctggagctggtgcaggaacaggctcttctggatttggaccatatgtagcaaatggcggatatagcggctacgaatacgcttggtcgtcagaatctgactttggaactggaagcggagctggtgctggctcaggtgctggtgctggttcaggagctggagctggatacggagcaggagttggtgctggttacggagcaggatatggagcaggagctggtgctggatacggagcaggagcaggaagcggagctggctcaggtgccggtgctggttcaggtgctggtgctggttcaggtgccggtgctggttcaggtgctggtgctggttcaggagctggtgctggttcaggtgctggtgctggttcaggtgctggtgctggttcaggtgctggtgctggatacggagcaggatacggagcaggagctggtgctggatacggagcaggagctggcgttggatacggagcaggagctggcgctggatacggagcaggagctggaagcggagctggctctggtgccggtgctggttcaggttctggtgctggtgctggttcaggttctggtgctggttcaggtgctggtgctggttcaggtgctggtgctggttcaggtgctggtgctggttcaggagctggtgctggttcaggtgctggtgctggttcaggtgctggtgctggttcaggtgctggtgctggatacggagcagggtacggaataggagttggtgctggatacggagcaggagctggcgttggatacggagcaggagctggcgctggatacggagcaggagctggaagcggagctgcctctggtgccggtgctggttcaggtgctggtgctggttcaggagctggtgctggttcaggtgctggtgctggttcaggtgctggtgctggttcaggtgctggtgctggttcaggagctggtgctggttcaggtgctggtgctggttcaggtgctggtgctggttcaggagctggtgctggatacggagcaggagctggcgttggatacggagcaggagctggaagcggagctgcctctggtgctggtgctggttcaggtgctggtgctggttcaggtgctggtgctggttcaggtgctggtgctggttcaggtgctggtgctggttcaggtgctggtgctggttcaggtgctggtgctggttcaggtgctggttcaggtgctggtgctggctcaggtgctggtgctggatacggagcagggtacggagcaggagttggtgctggatacggagcaggtgctggatacggagcaggatatggagtaggagctggtgctggatacggagcaggagcaggaagcggagctggctctggtgctggtgctggttcaggtgctggtgctggttcaggtgctggtgctggttcaggtgctggtgctggttcaggtgctggtgctggttcaggtgctggttcaggagctggtgctggatacggagcaggagctggcgctggatacggagcaggagctggcgctggatacggagcaggagctggaagcggagctgcctctggtgctggtgctggtgccggtgctggttcaggtgctggtgctggttcaggtgctggtgctggttcaggtgctggttcaggtgctggtgctggttcaggagctggtgctggatacggagcaggagctggaagcggagctgcctctggtgccggtgctggttcaggtgctggtgctggtgctggtgccggtgctggtgctggttcaggagctggtgctggttcaggagctggtgctggatacggagcaggagcaggaagtggagctgcctctggtgctggtgctggagctggtgcaggaacaggctcttctggatttggaccatatgtagcaaatggcggatatagcagacgtgaaggctacgaatacgcttggtcgtcaaaatctgactttgaaactggaagcggtgctgcctctggtgctggtgctggtgctggttcaggtgctggtgctggttcaggtgccggtgctggttcaggtgctggtgctggttcaggtgccggtgctggtggtagcgtcagttacggagctggcaggggatacggacaaggtgcaggaagtgcagcttcctctgtgtcatctgcttcatctcgcagttacgactattctcgtcgtaacgtccgcaaaaactgtggaattcctagaagacaactagttgttaaattcagagcactgccttgtgtgaattgctaatttttaatataaaataacccttgtttcttacttcgtcctggatacatctatgttttttttttcgttaataaatgagagcatttaagttattgtttttaattacttttttttagaaaacagatttcggattttttgtatgcattttatttgaatgtactaatataatcaattaatcaatgaattcatttatttaagggataacaataatccatgaattcacatgcacatttaaaacaaaactaaattacaataggttcatataaaaacaacaagtatgccttctcaactaagaatactatattgtttaaaccgtaaaaaaagtcatatttctgtatatcaaaacacatctaatattaaaaaaacagtcagcaagcacttacaagtgtgggctcggacagcaattacctggtctcaggagacacttgaagaacgagaagcacgtctctctgtcgattgcgaggctcatgcactatcgcttgagtctgagacctttactgatagggaaatccgtttgagctctcagagggttcggacagcaaaagcttgcccggtctcaggagacattagaagaacgggaagcataactcaataccgatcgcgtttccattgagcctatgcttcgtgataataataaataaagcccaaggtcagacgctaaaagttgtgggtgtagatataagtgttaactgcttttcacacagtcaactcggtcacgcggttatgtagctctgtcacatgctagcaatcctagcaacctgtatgctttgatccccgatggctatacgtctacgtcgtgtatagagaagctttactttaaattacatttttctaaatacctaaatgacggtgcttataaaccaaaagatatgtcctaaaactgctgcccaaagtcgctattccacgcggacggagtcgcgggcacagctagtaatacataaaataccttggaactcgaaacggtctttgagatatgggtcgttctttgaggtatgagggtaca

SEQ ID NO: 4 - protein, 232 aa, Bombyx mori
MKPIFLVLLVATSAYAAPSVTINQYSDNEIPRDIDDGKASSVISRAWDYVDDTDKSIAILNVQEILKDMASQGDYASQASAVAQTAGIIAHLSAGIPGDACAAANVINSYTDGVRSGNFAGFRQSLGPFFGHVGQNLNLINQLVINPGQLRYSVGPALGCAGGGRIYDFEAAWDAILASSDSSFLNEEYCIVKRLYNSRNSQSNNIAAYITAHLLPPVAQVFHQSAGSITDS

SEQ ID NO: 5 - protein, 216 aa, Bombyx mori
APSVTINQYSDNEIPRDIDDGKASSVISRAWDYVDDTDKSIAILNVQEILKDMASQGDYASQASAVAQTAGIIAHLSAGIPGDACAAANVINSYTDGVRSGNFAGFRQSLGPFFGHVGQNLNLINQLVINPGQLRYSVGPALGCAGGGRIYDFEAAWDAILASSDSSFLNEEYCIVKRLYNSRNSQSNNIAAYITAHLLPPVAQVFHQSAGSITDS

SEQ ID NO: 6 - DNA, 14809 bp, Bombyx mori
  source 1..14809: mol_type = genomic DNA
tgagttgaaaaattaatttcaggaaacaacaaaaataatgacgcaaaagtacaccggagtgaaaattaaaactaagaaagtaatcgctaaaaattattcatctcgtgaattgattgagcgcgataataacgcagtactattggagagattctatgtttaatatattaatgatatgatataaaaaagggtgcgtgtacttatctacgcgcgtaagaagttatactttattttcattaaatttatttctttttttttatttcaattttaatcaattttaaaaaaaatcgaataaacaacatcctcaaacacgcatattggacatcccttttcttgacatcgtataaattcggtaattctcggtacggttcggaaagtgcacctgcggctatattcagactcgccaagttacgtcagtcgtattgtaatgagcgatttagtgggcaacttcattctgttaattttgtgtcacggtgcgcgcgcatcgtaaaatttcactctcatagatttttcataacgtgcctaaagaagtataacttcaataatttaaattaaaaaaaaaaacatgcatagaataattatatgaattatttaaaatgtcatttaccgacattgacataacagacgacgttaacactacaaaacattttaattccacattgttacatattcaacagttaaatttgcgttaattctcgatgcgaacaaatataagaacaatcggatcaattagatcgctttgtttcgagcaacacttagtttaactagaggcgtacacctcaagaaatcatcttcattagaaactaaaccttaaaatcgcaataataaagcatagtcaattttaactgaaatgcaaaatcttttgaacgttagatgctgtcagcgttcgttggtacagttgtttgatatttattttaattgtctttttatatataaatagtggaacattaatcacggaatcctgtatagtatataccgattggtcacataacagaccactaaaatgaagcctatatttttggtattactcgtcgctacagtaagtaattttaacttttttcaaatttatttagaatatatgtatatatatatactcaccacgttttaaaacaatttttacaattctagaactttcgttctgttttttctttatttgttcaatttgtgtatttgtggattccctacaatatggaaaagatgatttcgtgtattttttttattgctttgatgtttggacgagctcacagcccacctgatgttatgtggttactggagcccatagacatctacaacgtaaatgcgccgccacccaccttgagatttgagatataagttctaagatctcactatagttacaacggctgccctacccttcaaaccgaaaggcattactgcttcgcggcagaaatagccagggcggtggtacatacccgcgcggactcataagaaatcctaccaccaggagtattttcatagatagaagaaaaaacaattgtctagagcgtagacaattaattcttattaattagtttttgactatgacctatatagttacatttactttcatgttagtattatttactatttttaaaatgcatcaatcatgcagtgtatttgttaaaaaaatatattttactgcattgtgaaattatcaataaaaagtgtacgagaatcgcactggaagcaatttcaaaaattaagacgtcaaaaatcctttcgcattacaatgtgagattaaaaataaaattatgcgcggaatggccggcattcacggtatcgcaatcactacatagtataaaacaaagtcgctttctctgtccctatatctgtccctatgtatgcttaaatctttaaaactacgcaacggattttgatgcggtttttttaaatagatagagtgattgaagaggaaagtttatatatataataacatccattaaataggggagaaatcaataataaattacagtttccgaagcgaagcgagggcgtttcgctagttgtaacaataacttccaaagtcgacagatatgtttcctactttttatttcattttgttcattgcccgagcccacaactatcacaatgtagggcaccaagtggatataccaatattgtaatgcttggttcaattagaccagatttagaatataacgaaattatataacagttagagcgggtttgatttttattacacgattttattctttcatcgtggaagatagaaaacttttgttaagtacatattttatcagaaaaattggtatctgcctgcgggattcgaacatcggtacagtcgcatcgctcgatacgaatgcactggacgtctcatcctttaggacacaacgacttctaggctctttttacccctacctattcgctagtaggctaaagagctattccagcttcacgtgaacgggtaggtgagatcacgggttcaacttgagagattttgctaatacaagccttagcaagagtactgcttcgcagaatctactgccggatcggaatcgggacccactgagaagatccggcaagaaactcagtgggccatgtccatggattaagttcgctcgtcaaactcttaatcgactagttcgacgagaacggtgaccgactcttgaagatcctaaaatcaccgagagtggatccgcaggattcgacaagacatgtttcgggaaaaggtggctttgcgttgcttcgtcgcctaggtcggataggtaattagcggtgatcactggttttactggtggtaggacctcttgtgagtccgcacgggtaggtaccaccaccctgcctatttctgccgtgaagcagtaatgcgtttcggtttgaagggtggggcagccgttgtaactataattgagaccttagaacttatatctcaaggtgggtggcgcatttacgttgtagatgtctatgggctccagtaaccacttaacagcaggtgggctgtgagctcgtccactcaactaagcaataaaaaaaaaaaaaaaaaaaaaaaaaaaaaacagatcataagatcatgggagcggacatcttataagtccgcacgggtaggtaccaccgccctgcctatttctgccgtgaagcagtaatgcagtagtttgttttaatataaacatttgaatatactgttttattcatttatttattacacttcatgtaatatctacatgggctgatttaatgcttaaggcattctctaccagtcaaccaaaactagggcagaatgaataatggtaggtgcattaaaatatacattttattatttttaataattttataaaatattatttatgaaattattttatataaatatttattaaatagttttaatattattttcaatattctcagttagttcggtcgttaaataaatttttttaaccatgataagtttcgcggaaaactgatagtatatctcaattcgcacgaaaaatttaaaaacacttatttctcagaactttattagccaattaggattaattatttaaatcgtgtattaaaaacaatgaaatattgactcaaattggacacaataataatatctaggacacggcccatggctggagcggtgtggccacccactttttttttttgcttagatgggtagacgagctcacagcccacctgatgataagtggttaccggagcccatagacatctacaacgtaaatgggccacccaccttgagatataagttctaaggtctcaagtatagatacatgtgaattcaaataattatagtagaataaataaaatgtgatgtaaataataatacattgacgtaagagttccatgtcgagttcgacactagttagtggaaacattagggaacagtaatcagtatcggtatcagtatcagtatcagtatcagtatcagtatcagtatcagtatcagtatcagtatcagtgtcagtgtcagtgtcagtatcagtatctgtatcagtgtcagtatctgtgtcagtatctgtgtcagtacctgtgtcagtatctgtgtcagtatcagagtcagtattagtattagtatcagtatcagtatcagtatcagtatcagtatcagtttcaaagggtttgcgtacatgcgatctagcccgtagaaaacccactgagcttttcaccggattttcgcactggatcccgatttcgatctgatggtagattctgcgaagcactgttcctgctagagccagtgctagcaaagtctctcaggcttagcccgtgagctcaccgtcccgtccgcacgtataaaaacaatagcaccttaggctcccagcgaataggtaggagataaaaagaattatattattggtttttataaatttttattataaattacgtactaaacgagaccctggaaataaatatgtcgtaaattgcaaaacgtaaacattaaaaccatccctaaacccgtcattaagtaatctgacagcatattttatatgaacaacgtgttgcgtgttttgaatatataaatattatccgaagcgtgcggtgaaactttccaaattggaaatactccgacgtaaatacctagaaacgttagtattatgccctacgacttgtttcgcttctcctctgtcttattatatcacatccaattgcttatctatacttctatactagtctatactaatattataaagaggaaagatttgtttgtttgtttgtattgaataggctccgaaactgctgaaccgatttgaaaaattccttcactgtttggaagctacactattcccgagtgacataggctataatattttttgaaaaaattaggtatccttactaaaactccaataatgtaaccaaaagtgtaaaaaaattacctcaaatattctttacatcgtgtgccctgcgaaaattattgatgatagaataaaataatgtattacgactttgtagaacacattgttatttacaaaaagtgtcgcgacagcatatgtttaactattatacatagttatgccgcaagaagtgttcttttatttttttaaataaaacaacgtcaaatatcgtagaaatttttgttaaagacccgagcggatccggagcgggccgctagttaaatataaactgcttttacagtttgatttgacatttcattattttttaatttattttttctgatctgaacttatagatgattatatatgctgcaagaaataaacttaatttgtcttcacaatctattagtgctgatgttagaagtaaaaaaaaaaatatctataagataagaatcctagtgtaatcgtatcgtctgatgcgactgtgcccctattcaaattctaaaggatgcttaaagatgcccaatcttttctcaataaataataggtaactaggacagtttaattttcacaatgaaataattacatacaacacgtaataaaaatcaaatcaccaaatcttttaagctttgcgtaaacagtgtgtgcacaaattgtaagccgctacaggtaggtatcatagttttgcctatttcaatcacaccacgattcgaagagtgaggtagttttgaaacgattgctacctggacaaggtactttcaaggtttttgcattcatgctgtctataagctacggtaacggcttagctgaggcgagccataagctcacttggccttcttttttttgtgtttgaaagattactttccagtttcaccaggacaggtgggcgagcaaaggctcagccagaagggccggaatttgctaacaactgcccgagcgcctccgaaggagacctaacaactcaagagcaattgcttcgcgaatgaatctactaccgaatcggaatcacgacccgctgagaagatccggcgagaaactcagcgggctgatgcatgggttaggttgcacgtcgacctctttgtcgagttcgacgagtacggttaccggggtccttaagcctgctcctagtattagagctgaaggtgtctaatgcacaggttattggatctgatggatccgtaaggacgtgacttggcttatttgcctatctgcctataaaaatgtattccgtgaaatcaaaattcaaatttaacgtcaaatttatatgtgaattacatatgtatgaggaatgcgtgatcgtgtgaagtgcggaccgtggaaaattgaaattggctttgaggatgacgggtctgattaggtgcctgaagcgcgttcattccgtagaattgaaatgttcggaacatcgttcgtgaccaagaaaactgtagagtgattgaaacttcggaattatcttgtaaataaaaccagcgagattaaaccttaaaattaaagattaaaattaagttattttaaatatgtctataattttttaatttttttttttattgcttatatcggtggacgagctcacagcccacctggtgttaagtggttactggagcacatagacatctacaacgtaaattcgccacccacctcgagatataagttaaatatagttacaacggctgccccactcttcaaaccgaaacgcattactgcttcacggcagaaatgggcggggtggtggtacctacccgtgcggactcacaagaggtcctaccaccagtaattatgcaaattataattttgcgggtttgatttttattaactacacgatgctattccttcaccgtggaagtcaatcgtgaagatttcttaagtacgtattacattagaaaatttggtacctgcctgcgggattgcaacaccgatgcatcgctagatacgaatgcaccggacgtcttatcttttaggccacgacgacttttaaaaccaaatagataatgaggtatcgggagagtacatggaaccccagagtcatttccacttcctctacatacaaatgcgtatatatcgtaatgatgaaacacaaatcgtttaaaatgaaattcgcagaagacactaaatacaaaatcatgatcggattgtgtcttactgcgaacgagctgacacacaagtcctaaagcaaaacaaccgtgcattttattcggtacacaatggaaatatttatttcgccttgtcattcctcaagatggcttcatacgtcaaacgcaggatatgccggtacatcgcggcgaagcgtttcgtaccggattcgcgtgtcaggatactcagatttgcagagcgaacacaaaaatactgacggcttttcttggcggggaaattagcttggaatcatgagtgaattatttgatgtttcttcagtaatgaacggcaattaaataacatacacataagagataacgaatctatataattaatacgtgaagcaaaaactttgtatccctttttacgaaaattgcgtggacggagtagtatgaaattttccacacttatagagaatatagagaagaagtacacaatgctaatatttttttaaaataatgcataaaagatacattaaatcaataaagaaaacattacacacactacataccatatatttgacgcacacacgcatgcatagtgcatactatttattgtcaaacttttgttctggacgtctgttgtcaaattgagaatagattaaatattgtttgtctttgataatattttttatagtgtagtcttggccaaatttcttggcgaagtataaaatacaatcgtaatagtgtacaaacttacaattccaattaattatagtcgaatttcgactactgcgggacctctagttcagataattctgcgatataatctcaatgtgctacattaagatatgattaatattaaaaatactgttactgttttatttcacgttttgaactgtcattatattatttcctgtttttcgaatactgaacggtcgaatgactacttgaacggtcgaaggtcacttgaacatcttatataagaagggtcaattcgttctttttcgtctctttgtatgtctgtcttttcagaagtcaaaaaatgtactgccgtgccgctggtcacgtacgccctcgtttcatttattttcgaattattttcaaatctctgtcttcgtttgtctatgtctagtcattgtaggtcttatgtggtgtcaaaaaggttacacgccactacaaatactttagcgttttcgtgaacacggacgatttaattattatcaaattctctagaaaaacattgctaaagattctcaaggttcgtttagaatgtctgttcgttcgtttggtaaaaacaaaaggagcacacaaaacataaagattttatgtttgtcatttctcgcaatcccctttttttacggaaatacctaccatgcgtttacgaactagctttactgatggacctcttgtcagtccacacgggtaggtaccaccaccctgcctatttttgacgtgaagcagtaatgcgtttcggcttgaagggtgggacagcagttttaactataccttagaacttatatttcaagatgggtggcgcatttacattatagatgtctatgggctccagtaaccacttaacaccaggtgggctgtcatcccgtaaaatcacctaggcaataaaaatataaaaaataaaaataacttcctcacaaaaagaatatcatcgcgtatgtagttatagtgaaataatttattgcaagctcgcacgaatatcctccctatgcctattactgcggcgaaatcatacactttccaagatgaaacaatataataatactcagactacaacctcatgtctcaaggtctcatgtgaatttgtttgccaccgagcgctatttaacgtgagatcgaacgcgaactccatctagaacgataatataataatcattagaatgtagtaggccgtctgaaattcgattctccgctataacccgttaatctaacctgaccattaagtaaataaaaattagctctagatgagctcccggcgtacctggtcgcattaacacatcgatcggtggagcgacaaagctcttcgctctaagcctcaaaagaacaatcccgagaaaacaatttgttgtgtataatttaaaccaaaacccgaatttaatttttcgcagagcgcctacgctgcaccatcggtgaccatcaatcaatacagtgataatgaaattccacgcgacattgatgatggaaaagctaggtaattatgtaagctttaactaatattaatataggtctaatataatccggcagaggcaaatgcactgagcgtcttccgcaatagaccacgacgacttcgactaaaatttttttaatactttctaaaaaaatatgaaaatacggctcattgaatggtcaataactaccgtcacagatcacatcagcagtgccaaagacacatacactaactgacactagactcttttccaaccccatttaaagaaggaaatgttatagcgctcgatctgcgccatagagggtgaatcatttcaggattacatggcaaaaatgtaaaccgagaatgcactgtaaatgatcgtagtcaagtggctttaagaagtggaaatgatctcttctccgttgctgagttgtgtgattcacctcaattgacaaattcctcagaacactgcccatggtaaaaagtaaaaaatacaaaggaaatcaaaatcccatcttaactccagaagctctgactgatccttctgtatggagtcaaacagaattatctcaatttaagatagaaattccgtacgccaaatagaaattaaaagtctttatattggagagaaaagactctcacccaaaatcccttgaccctcccaggcctcgatgagtgagtgatcgatatctgaacttccatgaccaagacagttactgataaactgagacctatcaagttaggccaagttctctaggaacagcatattgataaaccactctatcatctcggaaagcagagtactcatagttatcgtataggccttaactcatagtcagttacgtcattttatttgggaagagaatggacgtgagtattctgtcacaaagacgaaatcctattgccatgtgtctttgaatctaatttgggtatcggaaaatctgggagttgtacggtctacacatcgtttgaagcagactatataatacgaatcgcaagtatgaagctaatcgtcacagtgcatctagtgataatagacatcacgacgtcaatggcaccgactatcttgaggctagaatttaaactgcctgttgcattgaaatctattacatcgaaatcgttttgctgcttcaaaactgtaacaggcaaagctcacagtatcctttctttaaactatgtttttattgcacaaaacttttcaatcatggttcaagtgttaatataataattattataattttagttccgtaatctcacgtgcatgggactacgtcgatgacactgacaaaagcatcgccatcctcaacgttcaagagatcttgaaggacatggccagccagggcgattatgcaagtcaagcatcagcggtggcccaaaccgccggaattatcgcccatctatctgccggtatccccggtgatgcctgtgcagccgctaacgtaagtagatgccgctgttagaaacaataaaacagtacgtctaaatatttattacccgaaactgataagactgataagaagaagcagtgtcacttttgcgattggaggaaatcgggaccctttctaaatccgacacaaattttcaatggttagggtaattaccaataaaatagaggttaaaacggttccggagggttaaattttaatatacggtgcgttattatacatatttcattacaaaatctacacaaaaactgaaaaaactagcttgacccgattcaccttggctttgtggttaaaccggtttcgtatggggacaatagagtttttcgataaggctggtactatttagtagttaggtaggcacgtaactttagataattaactttttaatatccctaatgatttacaaacctctgatgactgaattagactatttaaaactaacacttaataaaagtcattttcagttcaacaaagttaaatttaacaactcaacaaaagtattatgacatcacagatatatccctatactaactcttagtctttattcccccaatctactgtatccaaaattattccttaaacatccaatattacctgttgtttcagtaaaaggaaatggaaaatctaattaaaatcttctttgcaggtcattaactcttacacagacggcgtcaggtccggaaacttcgccggcttcagacaatctctcggtcccttcttcggacacgtgggacaaaacttgaatcttatcaatcaactcgtcatcaaccctggtcaactccgatactctgtaagtactcagcaattgttaccgaagagttacatacttgaatcatggtcggggcttaaatattcgatttatcgattagagaaatctgcactgaggtcaatatagcggtatgaagctactaccctatcgctttttgttctgaagaaaatagaatataaaataatacaaaaaaggtcaatcatgaaacttcttgtctcatgccgaatggcagaatatattctgtgacgtccatgggctccgataacgactgagtgggaggtacttgattcttatcctgggtaacatgatcgtttcatcacgggatactatcaccatccaagctaaatagtttagtagaaactactaatatatgcacgacggtttttggtaggaaggccgtgatccaatgcaatcgataattcgacttcatgcctcaagttaggttgtggaattcaattctatgggttcctaaccgtcctaggatgaacttaagagaaaacgagcgctaattgtgtacgataatttaaaaatcacctgtgttttaaattttgtattcacacttccagtattaatattaaactatggttttttgagaaagatgataaaccacactagtccaaatcgagtatgttcaccagcgggtaagaataacaagtgttgttttttttaggtcggaccagccctgggttgtgccggaggtggaagaatctatgacttcgaagccgcttgggatgcaatcttagccagcagtgactctaggtaagcatattgagctttccaaataagaatgtaaactggcacacaaggaatcaattactaagaatttatctctagtattttattagagacattcattcttttgcaataacagatccttcttatcttaatctttagaagcagcaaatagaagacgtttgcacccttaccatccttgtgtcgtctccccgtccttaactcctcacctccaaacgcagatcgcaggagcttttagctaattacacacgctaataagattttaatcatgtgcacccatttaaatgagtgtgatcttatctgttctaatatagcacgaattacacgtgctttacgctagtttatgttttactgtaactgttcttgaccaaaattcttcttctttctctcatctagcatctctcctttatcaatgtgtggctctatagcatttataacaagggtgtgttatgatctcgcacggttggcacagattggcaggatagtgatgcctatttttgcggacttccgatacgccctagctccagaatatatatttcaactagcagtcccggccacacgttgctcttgctaaggttttcgtttctaaataacacgtggccgactatgctaataccaaaaattaacaaagtaagatcaattggattttactgtattgcgtttactacgaaataattttcacttatagtttagcctcaacaacacgtggtggttatgcttttaaattgtagcttatatgacacatttataggtttaacatagcagcgccatttattgattacttactgaatccagtcaacagatatcgccatctgttaaaatcgtttgaagttaacagataattgtgagtgtcaaataatagacaaatgattagcaataaaataatattgcggctataaattaagatgtaagctatcctatctttcaagatggatcaaactgcacacggtgtgcaaatttaatttaaaatcggttaagtagtttaggagtccatcgcggacaaacaacgtgacacgtgatttatatatattaagaaatgtaccgacgattgaattgtattttactttccttcaattcgattacagtttcttaaatgaagagtactgcatcgtcaagagattgtacaactctcgcaacagccaaagcaacaacatcgctgcctacatcaccgctcacttacttcccccggttgctcaagtgttccaccaatcagctggatcaatcacagacgtaagttactttaaattacccagggtctttatgtaattttgttattagtaatgattggacaaatgagcttatcgccgattcgtcacgatcactcgtcactgatgtcacaaaggtcacaaagtgaacgtgttttggagttgatagatatagaaactccttatcaacaaaaaaaaaaatacatagacagcagtgacaataggtgtctaaaaaaaaagtgaaataatgtctgtcggttcgagaagtaaaacaaaataacaaaactgtgattttgattaaaaaaaatctaaagcatccacgtatttaattctaatttataaaagtgtgttagtatgttatttcgtaactgcctgcactctgtgatttaaagattggactctgctaccaaaaactttatatcaacgcgaccatcactatgagacttaagctgaaattatttctttcaaaacacgcttcatagatttaaagctgcccttcaatccagacatataagagctacgaatcaaacttaggccagcaaggtgtccatcttgtttttaccacctaaattgggactactatatattaattcacgtttttaattatccacagctcctgagaggcgttggcaacggtaatgacgcgaccggtttagttgctaatgctcaaagatatattgcacaagcagccagccaggttcacgtctaaataagaactgtaaataatgtatatatataattatataaaagatatatataaaccatatacaaacatatatatatcattataagacaatctacctatataaaaacagactaaaattaataattatgtatactttaattgtgtttaggacattttatgcaaattgtgtttgcgttaggattttttttggaagttttttagattatttatgaatatataaataaatatacgttaatataatatatattatataaatcaacgacacggcttttcattttggtgatgatcaatcttattgttcttctaattgatttttttgtacaataaagatgtatccagttttccagataaagaatttagtttgttatttctggccccattaaaataagtacggtattcgataataccatataccatacggcatatacaatggatttcggtgctgttgtcaattgctttccaactggagagactgtatgcgatttttttcatgtattcggagattaagctgcgaaacatacaaaaatgtaccttattttttcatcgcattaggcacaattcactttaataaagcccctataacgagaatgtagtccgaagcagtcacacttaaatctctaattctatatttaacgtacctcaagaaatttcaagtggcatttttgaagatatttcattgtttttcaaaagcacatcaatatttcaatctttacgttttggcgagtttcaaatagtcaatgatgttattttatccgggataaagaaatgcttgtcaaccttcgatccataaagtaccaatcgatgacgtaaagacgcaagcgaccgttgtctgaattactgtcgtatttataataacagatatatatacccggagttgcccggatgatgttttttttttaaatttattgcctaaa

SEQ ID NO: 7 - protein, 3295 aa, Bombyx mori
MRFVLCCTLIALAALSVKAFGHHPGNRDTVEVKNRKYNAASSESSYLNKDNDSISAGAHRAKSVEQSQDKSKYTSGPEGVSYSGRSQNYKDSKQAYADYHSDPNGGSASAGQSRDSSLRERNVHYVSDGEAVAASSDARDENRSAQQNAQANWNADGSYGVSADRSGSASSRRRQANYYSDKDITAASKDDSRADSSRRSNAYYNRDSDGSESAGLSDRSASSSKNDNVFVYRTKDSIGGQAKSSRSSHSQESDAYYNSSPDGSYNAGTRDSSISNKKKASSTIYADKDQIRAANDRSSSKQLKQSSAQISSGPKGTSVSSKDRQYSNDKRSKSDAYVGRDGTVAYSNKDSEKTSRQSNTNYADQNSVRSDSAASDQTSNSYDKGYSDKNTVAHSSGSRGSQNQKSSSYRADKDGFSSSTNTEKSRFSSSNSVVETSDGTSASRESSAEDTKSSNSNVQSDETGEEEELFDVVSYQKIEDGKPVIIMKVIPVEKSASQSSSSRSSQESASYSSSSSSSTEESSSSSSRAASSTDASSNTDSNSNSAGSSTSGGSSTYGYSSNSRDGSVSTTGSSSNTDSNSNSVGSRKSGGSSSHEDSSKSRDENVSTTGSSSNTDSNSNSAGSSTSGGSSTYGYSSNSRDGSVSSTGSSSNTDSNSNSAGSSTSGGSSTYGYSSNSRDGSVSSTGSSSNTDSNSNSVGSRKSGGSSSHEDSSKSRDETVSTTDSSSNTDSNSNSVETRKSGGSSSHEDSSKSRDENVSTTGSSSNTDSNSNSAGSSTSGGSSTYGYSSNSRDGSVSSTGSSSNTDSNSNSAGSSTSGGSSTYGYSSNSHDGSVSSTGSSSNTDSNSNSVGSRKSGGSSSHEDSSKSRDENVSTTGSSSNTDSNSNSAGSSTSGGSSTYGYSSNSRDGSVSSTGSSSYTDSNSNSAGSSTSGGSSTYGYSSNSHDGSVSSTGSSSNTDSNSNSVGSRKSGGSSSHEDSSKSRDENVSTTGSSSNTDSNSNSAGSSTSGGSSTYGYSSNSRDGSVSSTGSSSNTDSNSNSAGSSTSGGSSTYGYSSNSHDGSVSSTGSSSNTDSNSNSVESKKSGGSSSHEDSSKSRDGSVSSTGSSSNTDSNSNSAGSSTSGGSSTYGYSSNSRDGSVSSTGSSSNTDSNSNSAGSSTSGGSSTYGYSSNSHDGSVSSTGSSSNTDSISNSVGSRKSGGSSSHEDSSKSRDENVSTTGSSSNTDSNSNSAGSSTSGGSSTYGYSSNSRDGSVSSTGSSSYTDSNSNSAGSSTSGGSSTYGYSSNSHDGSVSSTGSSSNTDSNSNSVGSRKSGGSSSHEDSSKSRDENVSTTGSSSNTDSNSNSAGSSTSGGSSTYGYSSNSRDGSVSSTGSSSYTDSNSNSAGSSTSGGSSTYGYSSNSRDGSVSSTGSSSNTDSNSNSVGSRKSGGSSSHEDSSKSRDENVSTTGSSSNTDSNSNSAGSSTSGGSSTYGYSSNSRDGSVSSTGSSSNTDSNSNSAGSSTSGGSSTYGYSSNSRDGSVSSTGSSSYTDSNSNSAGSSTSGGSSTYGYSSNSRDESVSSTGSSSNTDSNSNSVGSRKSGGSSSHEDSSKSRDENVSTTGSSSNTDSNSNSAGSSTSGGSSTYGYSSNSRDGSVSSTGSSSNTDSNSNSAGSSTSGGSSTYGYSSNSHDGSVSSTGSSSNTDSNSNSVGSRKSGGSSSHEDSSKSRDGSVSSTGSSSNTDSNSNSAGSSTSGGSSTYGYSSNSRDGSVSSTGSSSYTDSNSNSAGSSTSGGSSTYGYSSNSHDGSVSSTGSSSNTDSNSNSVGSRKSDGSSSHEDSSKSRDENVSTTDSSSNTDSNSNSAGSSTSGGSSTYGYSSNSRDGSVSSTGSSSNTDSNSNSAGSSTSGGSSTYGYSSNSRDGSVSSTGSSSNTDSNSNSAGSSTSGGSSNYGYSSNSRDGGVSSTGSSSYTDSNSNSAGSSTSGGSSTYGYSSNSHDGSVSSTGSSSNTDSNSNSVGSRKSGGSSSHEDSSKSRDENVSTTGSSSNTDSNSNSAGSSTSGGSSTYGYSSNSRDGSVSSTGSSSNTDSNSNSAGSSTSGGSSTYGYSSNSRDGSVSSTGSSSYTDSNSNSAGSSTSGGSSTYGYSSNSRDESVSSTGSSSNTDSNSNSVGSRKSGGSSSHEDSSKSRDENVSTTGSSSNTDSNSNSAGSRTSGGSSTYGYSYNSRDGSVSSTGSSSNTDSNSNSAGSSTSGGSSTYGYSSNSRDESVSSTGSSSNTDSNSNSVGSRKSDGSSSHEDSSKSRDESVSTTGSSSNTDSNSSSAGSSTSGGSSTYGYSSNSGDGSVSSTGSSSNTESNSNSEGSRTSGGSSTYGYSSNSRDGSVSSTGSSSNTDSNSNSAGSSTSGGSSTYGYSSNSRDESVSSTGSSSNTDSNSNSVGSRKSDGSSSHEDSSKSRDENVSTTGSSSNTDSNSSSAGSSTSGGSSTYGYSSNSGDGSVSSTGSSSNTDSNSNSAGSSTSGGSSTYGYSSNSRDGSVSSTGSSSNTDSNSNSAGSSTSGGSSTYGYSSNSRDGSVSSTGSSSNTDSNSNSAGSSTSGSSNTHGASHGLASSGGSIASATSTPDILTIALSEDSSEVDIDLGNLGWWWNSDNKAQRAAGGATKSEASSSTQATTVSGADDSADSYTWWWNPRRSSSSSSSASSSSSGSNVGGSSQSSGSSTSGSNARGHLGTVSSTGSTSNTDSSSKSAGSRTSGGSSTYGYSSSHRGGSVSSTGSSSNTDSSTKNAGSSTSGGSSTYGYSSSHRGGSVSSTGSSSNTDSSTKNAGSSTSGGSSTYGYSSSHRGGSVSSTGSSSNTDSSTKSAGSSTSGGSSTYGYSSRHRGGRVSSTGSSSTTDASSNSVGSSTSGGSSTYGYSSNSRDGSVSSTGSSSNTDSNSNSAGSSTSGGSSTYGYSSNSRDGSVSSTGSSSNTDSNSNSAGSSTSGGSSTYGYSSNSRDGSVSSTGSSSNTDASTDLAGSSTSGGSSTYGYSSDCGDGSVSSTGSSSNTDASTDLAGSSTSGGSSTYGYSSDSRDGSVSSTGSSSNTDASTDLAGSSTSGGSSTYGYSSNSRDGSVSSTGSSSNTDASTDLTGSSTSGGSSTYGYSSSNRDGSVLATGSSSNTDASTTEESTTSAGSSTEGYSSSSHDGSVTSTDGSSTSGGASSSSASTAKSDAASSEDGFWWWNRRKSGSGHKSATVQSSTTDKTSTDSASSTDSTSSTSGASTTTSGSSSTSGGSSTSDASSTSSSVSRSHRSGVNRLLHKPGQGKICLCFENIFDIPYHLRKNIGV

SEQ ID NO: 8 - protein, 3276 aa, Bombyx mori
FGHHPGNRDTVEVKNRKYNAASSESSYLNKDNDSISAGAHRAKSVEQSQDKSKYTSGPEGVSYSGRSQNYKDSKQAYADYHSDPNGGSASAGQSRDSSLRERNVHYVSDGEAVAASSDARDENRSAQQNAQANWNADGSYGVSADRSGSASSRRRQANYYSDKDITAASKDDSRADSSRRSNAYYNRDSDGSESAGLSDRSASSSKNDNVFVYRTKDSIGGQAKSSRSSHSQESDAYYNSSPDGSYNAGTRDSSISNKKKASSTIYADKDQIRAANDRSSSKQLKQSSAQISSGPKGTSVSSKDRQYSNDKRSKSDAYVGRDGTVAYSNKDSEKTSRQSNTNYADQNSVRSDSAASDQTSNSYDKGYSDKNTVAHSSGSRGSQNQKSSSYRADKDGFSSSTNTEKSRFSSSNSVVETSDGTSASRESSAEDTKSSNSNVQSDETGEEEELFDVVSYQKIEDGKPVIIMKVIPVEKSASQSSSSRSSQESASYSSSSSSSTEESSSSSSRAASSTDASSNTDSNSNSAGSSTSGGSSTYGYSSNSRDGSVSTTGSSSNTDSNSNSVGSRKSGGSSSHEDSSKSRDENVSTTGSSSNTDSNSNSAGSSTSGGSSTYGYSSNSRDGSVSSTGSSSNTDSNSNSAGSSTSGGSSTYGYSSNSRDGSVSSTGSSSNTDSNSNSVGSRKSGGSSSHEDSSKSRDETVSTTDSSSNTDSNSNSVETRKSGGSSSHEDSSKSRDENVSTTGSSSNTDSNSNSAGSSTSGGSSTYGYSSNSRDGSVSSTGSSSNTDSNSNSAGSSTSGGSSTYGYSSNSHDGSVSSTGSSSNTDSNSNSVGSRKSGGSSSHEDSSKSRDENVSTTGSSSNTDSNSNSAGSSTSGGSSTYGYSSNSRDGSVSSTGSSSYTDSNSNSAGSSTSGGSSTYGYSSNSHDGSVSSTGSSSNTDSNSNSVGSRKSGGSSSHEDSSKSRDENVSTTGSSSNTDSNSNSAGSSTSGGSSTYGYSSNSRDGSVSSTGSSSNTDSNSNSAGSSTSGGSSTYGYSSNSHDGSVSSTGSSSNTDSNSNSVESKKSGGSSSHEDSSKSRDGSVSSTGSSSNTDSNSNSAGSSTSGGSSTYGYSSNSRDGSVSSTGSSSNTDSNSNSAGSSTSGGSSTYGYSSNSHDGSVSSTGSSSNTDSISNSVGSRKSGGSSSHEDSSKSRDENVSTTGSSSNTDSNSNSAGSSTSGGSSTYGYSSNSRDGSVSSTGSSSYTDSNSNSAGSSTSGGSSTYGYSSNSHDGSVSSTGSSSNTDSNSNSVGSRKSGGSSSHEDSSKSRDENVSTTGSSSNTDSNSNSAGSSTSGGSSTYGYSSNSRDGSVSSTGSSSYTDSNSNSAGSSTSGGSSTYGYSSNSRDGSVSSTGSSSNTDSNSNSVGSRKSGGSSSHEDSSKSRDENVSTTGSSSNTDSNSNSAGSSTSGGSSTYGYSSNSRDGSVSSTGSSSNTDSNSNSAGSSTSGGSSTYGYSSNSRDGSVSSTGSSSYTDSNSNSAGSSTSGGSSTYGYSSNSRDESVSSTGSSSNTDSNSNSVGSRKSGGSSSHEDSSKSRDENVSTTGSSSNTDSNSNSAGSSTSGGSSTYGYSSNSRDGSVSSTGSSSNTDSNSNSAGSSTSGGSSTYGYSSNSHDGSVSSTGSSSNTDSNSNSVGSRKSGGSSSHEDSSKSRDGSVSSTGSSSNTDSNSNSAGSSTSGGSSTYGYSSNSRDGSVSSTGSSSYTDSNSNSAGSSTSGGSSTYGYSSNSHDGSVSSTGSSSNTDSNSNSVGSRKSDGSSSHEDSSKSRDENVSTTDSSSNTDSNSNSAGSSTSGGSSTYGYSSNSRDGSVSSTGSSSNTDSNSNSAGSSTSGGSSTYGYSSNSRDGSVSSTGSSSNTDSNSNSAGSSTSGGSSNYGYSSNSRDGGVSSTGSSSYTDSNSNSAGSSTSGGSSTYGYSSNSHDGSVSSTGSSSNTDSNSNSVGSRKSGGSSSHEDSSKSRDENVSTTGSSSNTDSNSNSAGSSTSGGSSTYGYSSNSRDGSVSSTGSSSNTDSNSNSAGSSTSGGSSTYGYSSNSRDGSVSSTGSSSYTDSNSNSAGSSTSGGSSTYGYSSNSRDESVSSTGSSSNTDSNSNSVGSRKSGGSSSHEDSSKSRDENVSTTGSSSNTDSNSNSAGSRTSGGSSTYGYSYNSRDGSVSSTGSSSNTDSNSNSAGSSTSGGSSTYGYSSNSRDESVSSTGSSSNTDSNSNSVGSRKSDGSSSHEDSSKSRDESVSTTGSSSNTDSNSSSAGSSTSGGSSTYGYSSNSGDGSVSSTGSSSNTESNSNSEGSRTSGGSSTYGYSSNSRDGSVSSTGSSSNTDSNSNSAGSSTSGGSSTYGYSSNSRDESVSSTGSSSNTDSNSNSVGSRKSDGSSSHEDSSKSRDENVSTTGSSSNTDSNSSSAGSSTSGGSSTYGYSSNSGDGSVSSTGSSSNTDSNSNSAGSSTSGGSSTYGYSSNSRDGSVSSTGSSSNTDSNSNSAGSSTSGGSSTYGYSSNSRDGSVSSTGSSSNTDSNSNSAGSSTSGSSNTHGASHGLASSGGSIASATSTPDILTIALSEDSSEVDIDLGNLGWWWNSDNKAQRAAGGATKSEASSSTQATTVSGADDSADSYTWWWNPRRSSSSSSSASSSSSGSNVGGSSQSSGSSTSGSNARGHLGTVSSTGSTSNTDSSSKSAGSRTSGGSSTYGYSSSHRGGSVSSTGSSSNTDSSTKNAGSSTSGGSSTYGYSSSHRGGSVSSTGSSSNTDSSTKNAGSSTSGGSSTYGYSSSHRGGSVSSTGSSSNTDSSTKSAGSSTSGGSSTYGYSSRHRGGRVSSTGSSSTTDASSNSVGSSTSGGSSTYGYSSNSRDGSVSSTGSSSNTDSNSNSAGSSTSGGSSTYGYSSNSRDGSVSSTGSSSNTDSNSNSAGSSTSGGSSTYGYSSNSRDGSVSSTGSSSNTDASTDLAGSSTSGGSSTYGYSSDCGDGSVSSTGSSSNTDASTDLAGSSTSGGSSTYGYSSDSRDGSVSSTGSSSNTDASTDLAGSSTSGGSSTYGYSSNSRDGSVSSTGSSSNTDASTDLTGSSTSGGSSTYGYSSSNRDGSVLATGSSSNTDASTTEESTTSAGSSTEGYSSSSHDGSVTSTDGSSTSGGASSSSASTAKSDAASSEDGFWWWNRRKSGSGHKSATVQSSTTDKTSTDSASSTDSTSSTSGASTTTSGSSSTSGGSSTSDASSTSSSVSRSHRSGVNRLLHKPGQGKICLCFENIFDIPYHLRKNIGV

SEQ ID NO: 9 - DNA, 27298 bp, Bombyx mori
  source 1..27298: mol_type = genomic DNA
attggttggcctttagttggcaaaatggtacgtctttaacctcaacgtggtcttctgcattaactaagtgctcaccactgtcagcagcaataaaaccatttttgaaataataacatcggtacactaacatagtgagctagtcgcaaaatttatgtacagagaaaacaaaccttctttggggtgttgagaggaaatcgctggattagaactatcgtgaagaccatccgctgatcttgtgtacttaaattcgcggatccagcattaagcgccggatctcagttcgatcgggatcccagttaaaggggtgaaattagctatcacttcgatatctgttctcaaagcaatgttccacttgtaaaagcataagcggtcagaaaccttgttaaccaatagagccaaatatagttaacataatcgaaatttattcaaatattattcgtgtattgtttatagcctttgtcaagtyttttacaaggcaagataataagtaatattccgtgattggacgtaacatttcgcggaagatccttagccgataagtcgaagagccgcgtgtggctagagagacgcgggttcccgaccgctagcttaggcgcttattccgccataatcaatgtacgtgttcacaattagcacccgaaattcgtaatacgagaagtatcgaacatcaaaaatgttaataattctctttaaaaaaaaaacagagcatcaaatactgcacaaatgtcaagcgggtctcaacgagccatgaataaattagaaatcaattaataacataaaaaagcaaacaaaataaaaccatttacagagagaacgtttgttgaacaaaaacaataacttgtatacattgtttgcacaaatgtttgaagcgaaaatttattactccctacgtaagcttgatcaaacttcgttttcgtataaaacgcgttggcccaacaactttggcatagtcgttttatcatcgggtctctaaggatcaagcgatccaaagaccgccaacatgcgtttcgttctgtgctgcactttgattgcgttggctgtgagtatcattgcttcgttatcaacaatgacgtatttactaagaacactcttagatatgccttcaaattaaagctttcaaagctctgaagttcaccaaatacgactgttttagcgtaagctatttctatcccccaacagccatttagcgactacccgaaaatcactcgatttaacttgggagtttctgcaaactaaaagttcacaggccgtccccgattaaacttttaaacgcttcgcgaaaatatcagagttattcaaaagttgccacaaaaacctttgtccactaatatctatagaaggactggcggttagcagcaaatcatctagattttgggtggttggttcagaattttccattttactcttgggagtcgtttcggtctgcattccctacgcattattagaatccatcgaatgtaatttgtataattacgagttaaatactgtgtacaaaccaatatgtgaatttttattcaactagtttattgtttttaacttataggtaccagttttgaaacgaacttcagagttatctagaaaacacataattatgagtcgcttcactaatctatattaaattatgctttaatacttttaatagcttacttggggaaattgtgatttttcatgtaataacagtccacttggtcataagcagcttttatgggcttgcgctggacatgaatgccgcagaaccaacgatcgttggagcagacggggtcttgagtggagaccgcgtgccggctaacgtagtgtgggacgcctcccgaccaagtggagggctggcttgcgatttgggagaggcctatgtctagcagggaacgattaggagctgatgattatggtcataattgacagtcacttcgtttatggcaatcaaatatcctgggcattttgagggtattttgctaaacgaagacatttattcgaacgtaatttaatttaatttaatttattgcttagatgggtgggcgagctcacagcccacctggtgttaagtggttactggagcccatagacatctacgacgtaaatgcgccacccaccttgagatataagttctaaggtctcagtgtagttacaacggctgccccgcccttcaaaccgaaacgcattaactgcttcacggcagaaataggcagggtggtggtacctacccgtgcggacccacaataggtcctaccaccagtccaatggtatcccaaaaatttatcataacaatcctgatttttaagaatgaggcagtcgttcttagactcttcgtttccaggaagacgacattaatattcggtttaattggctatagtgactatgttatcctagttggtaattaattcactagcataactatatgattatcgttaatccgattcgtctttttctttctctgtttgattgcttaccaatcgctctgggagcaatttggtttgactctgttggtttagtctttttttttaatcatcatcaccttgatgtcaaaataatgttcttgtgaacaatttcgactaacttaacgaggggtgaaaggcaatttggtataagcttaatagtatttatctttaattaaaggtccattttatttggtactagcgacccgccctcgcttcgctacggaaactgtaatttattattgatttctccactattcaatggatgttattatacatataaaccttcctcttcaatcgctctatctattaaaaaaaaaccgcatcaaaatccgttgcgtagttttaaagatttaagcatacgtagggacagacagatatagggacagagaaagcgactttgttttatactatgtagtgattagtatcaacagttcgatgtttttaatttaacttgaattaagtttaccccattcaaatagctgaagtttttttttttttcatattaaaaactttaaatggcttccatgtaaagttgcaaaaatgtcacttaaaatagacacccctcgatatattgtaaagcacaacatatatattaatgaattttttatttatttttcaggcgctcagcgtaaaagctttcggtcaccaccgtgagtattccttatgacacattattcccgcaaaactcttacagaaacttcttagaatgcatcctttttacataactctaacctaaacagtgctaatacacaaaagataaacagtattttttttcacgcaggacttggcaattatatcgcaatgatttgaatatatatggttctatatatgggatattactatatttatgtattacgatttgattttggatattttacgtgctgcctgaatttaattgactatgcgaagaatatttcttggataggaaagttaaattctcgcgaattagtagaacgtccaaatttaaaaataatgtatggttatttatatatctagagattaatgatccttatcgtccttaataatagaggtgaatatatcagataaaggaggagactgcgttatctcatcgaaagaccaacaaatttttgtcataaaacatttcttgaaaataaaatttgaaaagttattaagatgtcgaatttcgaaatccgttttcattaatcataatgcatttttttattgaacataacagcaaaatggatttaataagctttcgaactaaacaaaaggttagttctacaaaaaacaaaagtcttcatgtggaaatctaaatcgacataccgccgcttcggaatacagtatcgcaactaagaaaactcatatcgaggggtttttttttggtggaagagctcacagcccacctggtgttaagtggttactggagcccatagacatccacaacgtaaatgcgccacccaccttgagatataagttctaaggtctcagatatagttacaacggctgccccacccttctaaccgaaacgcattactgcttcacggcagaaataggcagggcggtggtacccacccgcgcggactcacaagacgtcctaccaccagtaaaatggggtggaatgctatctggtttaagcgtcatttatctttgtaattaaaggtctgttttattagcatcaacagttcgatatttttaattgaacttccattacgtttaccacactcaaatagctaaagaagttttttttgtaattatattctttccaaatgtttaaactttaaatggctctcttgtatctttgcaaaaatgtcgcttaaacatttcaatcctcgatatgataaggctatttgtacacacacattgtcttcataacattataatttaactatataaaaacattttgtataaaacaacaataccttacaaaatataacgttcgtggatacacttcatgtaggtgcgacaaacacaggcaattttaatttttttttattgcttaagtgtgtggacgagctaacagcccacctggttttcagtggttactggagcccatagacatgtacaacgcgccacccaccttgagaaatattttttttaaggtctcagtatagttacaacagttatattgcggatttgatttttattacacgttacgttattacttcaccgtggaagtcaatcgaaaacatttgttaagtacgtatttcattagaaaaattggtacccgcctgcgggattcgaacaccgttgcatcgctcgatacgaatgaaccggacggacgtcttatcctttaggccacgacgaataaaattagagaataaaaaaaattaaaatttaataaaaggattggtgaaatgtcttcggaaagagtttagttacgcgttaagaagtaatacaaagaaattcaatcatacgaaattcgttccagtttttatggcattagaacacctttttcaatgtcgtctgaatgttaatctatatatataaaaatgaattgctgttcgttagtctcgctaaaactcgagaacggctggaccgatttgcctaattttggtcttgaattatttgtggaagtccagagaaggttaaaaaggtagataaatatgaaaatgcgcggaattaaataaaaataacaattttgttttttctttaatgtgtcccccaaaagtttaggtcttttatttattgattgaggcactacggagtctgccgggtcagctagttgataatagaaacagtcctaagtaacgcggcattttatttatttattaggcacacaatacacattccaagctaaaaagatacataaaaaacacaagtaagaagaaacaaaatctgacttgcaacataagccatgtgcgcactaatccaactaattacgaattaagagggcttatcttttttttttgtatctaattcgaaataaaaatcggatttaagcatgtccgttaacttaatagacttcaacttaataataatctggatttggtcttgtcatggcaaagtttagtattttttttaatgcaaatggaaggttctggaacagaatgcgataatcggagaccacagggtcgttttgggcgcagtcgctgtttaagcaactagggatatatactaaaaaattatagccaaagggcatccggcttctgaaaacatccaaccaatttcggtactattttccatacaccatcaggccgtttgaggccaataagggctaatacatttatatacgcgcctgatctatttaagctttaccgcataaatacgtgaagtgttaacgcattgggagataacgacagaaggaagatcttccgccaggcggttgaaaatattctgtagacagaccatccgaatattattgttcggaacttgtatatacacaagcttatcttgaaaatgacgtgaagttcaggcatctatcagatatctgtcttttacgatagcttccgacacggtgtatcacacgagctcaccagaacccagaaacacttggaccgactaaactgtatacacattcagaaaaaacattcttcttttgtgaaaagaatattgaacttaacgaaaatgggcacaattatgaatttcctcacgcttacacaccacaaatgacgtacaaatcaaccatacactctcatgacaagaagcggcagcaatagagacggaaggcaattgaaaaagtaactaatgtcattctgtttgttgaacatttttagtaagtggcgacgtagctgaaaatagcaacgtcttcttccataaaccagttacgtaatagcagagacgaggatgtcccaatggcacatgatgttcacaattacatttcacattttttaataataatatttttaataaaattttaaattcataaattgactaagcgttttcacgtacccacacaagaggagtacactactggatccacgcacaagatacgccaagaacgccaaaacacaaagcaaaaccacaaactcgcctggaacatacaaacaaacagcagaccacactaacatggtaacacgcaaatgtgaaattaatccctctgtcttcactaatcttatattgattcgcagccggcaatcgagatacagtcgaagtcaaaaaccgaaagtacaatgcagctagcagtgaaagctcttacctcaacaaagataatgattcgataagtgccggagcgcaccgggccaagtccgtagagcagagtcaggataaaagcaaatatacatctggtccagaaggcgtgtcgtacagcggaaggtctcagaactataaagattccaagcaagcttatgccgattatcacagcgatccgaacggcggatctgcttctgccggacaatctcgcgacagcagcctgagagagagaaacgtacattacgtctctgacggtgaagcagtggccgcttccagtgacgctcgcgatgaaaaccgatccgcccaacagaatgctcaggccaattggaacgctgacggttcttacggagttagcgctgatcgaagtggttccgctagttctagacgccgccaagccaattactactccgataaagacatcactgctgcttctaaagacgattcacgtgcagattcttctaggagaagcaatgcctattacaacagagatagtgacggctcagaatccgctggattaagtgaccgtagtgcttcttcctcgaaaaatgataatgtatttgtttaccgcaccaaggattctattggaggacaagcgaaatcttcaagatcatctcattcacaagagagcgacgcttattataactccagtccggatggtagctacaacgctggtacgcgagacagttcaatttctaacaaaaagaaggcaagctctaccatctacgctgataaagatcaaatacgcgccgcgaatgatcgttcttcttcgaaacagttaaaacagagcagcgctcaaatctcctccgggccaaagggcacctctgtaagcagtaaggataggcagtactcgaacgacaaacgcagcaaatctgatgcgtacgtcggacgggacggcaccgttgcttactcaaacaaggacagcgaaaagacctcacgacaaagtaatacgaactatgccgaccaaaactccgttcgctctgactctgccgcttcggaccagaccagcaacagttacgacaagggctacagtgataaaaatacagttgcccatagctctggtagtaggggcagtcagaatcagaaatcgtcgagctaccgcgctgacaaggacggtttttcctccagtacgaatactgaaaaatccagatttagttcttcgaatagcgtcgtagaaacttcagatggaacttctgctagtcgcgaatcatcagcggaggataccaaatcatccaatagtaacgttcagagcgatggtgagtattaaatgcgacacaaaacacataatcaattataaattatcatggtctcatttatcatcgttttaatattattaagtaactcgtcgccatctgttcaaacagttataatgaacgcgatgtttttccgatcattggcttttaacaaaagacatcggtttgtttcattcgttattagaggttaatcgtgtttactcttttaatttattgataacacaagtcattattgtgtaagaagtcgataaatctacacatacatagattaatgggaataatgataaattacccgcatttaaattaaaattaaaacttgtatttcgaatcagcagtaactacctacttttgggattttaaacaaatcttgcttctcttctgggtgcttaagatacaccaagaatatgaagccttttcttcatggcatgcactttcttcattacgctatttaattgtctgctttttccgccacagtattagggtcatacacaaatagagaaaaaaaaagtgcagcaaaaaaaatatctctaaatcagtgtgaaacaaactatttattatttaactattgattatcaatcttttaatcactgtaaccgagatcaatgtgtcttatttttggcataatcgcaatttttatatttttgcggaccacagaagagacaatttagtctacaagagatgaaaagctgtgatgcagcgtaagctaaaatatattaagacaacataatcaaacacatgtagccactgatataaacgaataccaaaacgcaaataaaatgtcaaaataatcacattaattggaatataaaaaataaaataataatgtctacagaaaggaaaatcccttcggtggacttatgaaacaaaacaaaatttcgaatgataataattttacagccatggtatattattcgtattgaaccccctgaacgaaatcaataaaaataaaaataaatgttttcgtttcctctatttacattgattagatttataattttttctattgcgaatataaaatgtactaaaaagtttgaggctctaacttagaatatcaaatgttgccaaaatcaaacctctttctaaccaactttaaaaaaggagtaggccctcggttcaactatttttctacttactactttctctacttagacctaccaaggtatgtttcttacacattttctgttgacatagtcttttcggtggacatcgggaccacaggaaagatgtccacagaaaagatgtattataaaaactcttgcgtaaagaaattaactttaaggttagaaatcaagcaacatgcttttcatttacttgtactaaatgctcatataaaaacaataaatatacatttttatagataatatttacatgtctataattggaacaggaaagaacacttgatcttttacgtttatgtgtgttttggaataaaaaaaatattttcactcgcactgggatcgaaacaacaaaatatcaaacgccggaatggccactatttagtgatgccaacagttaaaaaaataataataatgcggtcgaataaattaaaatttgatgtcgttttatcgtgtccacagaaaagactcaatttgatgtaaccataggtttattggatttattgtatacagatagtaacgatatattttttttattctcaatattatcatctttattatattgtttgtattacaagtaaataattttaatatatagggtactttaactatttttaaacatggctcaaacattataccttcgtcttgtaacagtccacaggaagagattttttgatgtttaacgccatcaaaatgaacttatgaaatgtaatatttacaagatacgattaaaatgagtagtaatatagtacctttacgatttaaatactttcaaatattcgccaatttgctcttttagatgatacattgctataacactttttttaccctttttgtgtatgacccattagtcagctaacctttgcctgccgtgtaggtcaccggtgccctacgcggcgcactgaagcaattatttcgtattcagtttctaaggcgccggaatatgtagtagactctggaaaagacgaatccgaacgatactgagaatgaatcgtatttctaagagacctaaaagacaaaaacgtacattgaaaaacaagagaagataaagttaggctatccaggtgcttagtaacaggaatgggaataattactgtagtgcgtcacgtagggcaccggtgacctacatggcatcacacatatatgttaaaaatgttatttctccattattacatttgttctttaacaatcaatgaccgaaatcggcagtgctacatgcatatttcaactaatacaacattttgacattagaccaaactaataatattaatgtatgaacgattatgatcgggtctcgatatgtgtgaaaattattttgattactaatcggattttgattactacttgtttttgctgaaaattacattgaaacatctcatctgatcaaatgaagttcgctatgtatatattttatttggttcgttcacacaaaaatatacaacggttgaaagtaatataaaaacgcaataagtaagactctaacttaaataactggaacacgaaataaagacgagactgagacacggtcggtcagtgtgggtgggccttatcatagcgatcaaagtcacccaaagaactatggaggattatgctcagagtttccttgctagatcggatcaggaatgaggagaaacgtaggagaaccatgataactgacatggccaaaaggattgcgaggcttaagcggtgttttttttttttctacataatctgatagccttgagaggctatatcagcgtcgccttaaccagtagatgagctcacggggctcaaacctgatgacgttgctaacacgaaccctagcaagagccgtgcttcgcagaatctaccgccggatcggaaacgcgacccactgagaagatccggcgagaaactcagtgggctaagtggtagtggacagggcgcattgctagtagaaaagatggccgcaatggccaaaaagctctagagttgcgtccgcgtacccagtagcggatttgcagtctcggctgccctaggccccaagccaccaaccgcccctttctcagcatccaccatatagactacataatgaaattgctttattgccaacttttatttaaatagatttagaaatttaggaaaaaaaattagttttatttcgcaagaatatggtacatgagttcttacaactagttatttgctctaacatactctgccaacttggcatacttggttatgataacttttacacgagtgttatcaactttcaacacttaattgcgagttaaatatttgaatatctaattaaacacaattaatttgtacggagctacttgttatcgcaagtgtgggtgcgaagtgtgggtaaaagtatgttttttgacacgattggggccgtccctaaatctggccttagggtaaatcttagggtaaatccgccactgcgcgtaccggaagatgaatcgtggatacgcaaagcaaacctacgatctgttgaaggttgcgggatttcgctgggtacagacagcataggaccggtcattacgacgaggcttggagtagacctatgtccgtcagtgagactggtagatagataaagaccagcctttattcattcttgttcgtttaaggcctttaatggaccaaatcaatacaacggttttttcatgcttagcttgttaggttataatattattttttatttatattaggaatcgctccttagtacctatttatgggaatagcttatcttaccttcttgatgccttcctaagcaagaccattttatctaacaagataagctgttaccacagtagttcatttctattaatttgtttcataaggggttatcattataaatacgattgctatcggcatgtctccacggtctaacagctaaaacgcccacaggaagagcctttatcgtaattcgatccgcgtgtagatacaaatctcaaagcgattgtgtatccagcgtgtattcataaatgaaatgatgacgtcataattttttatttatttcgtgtgcactcatacttcgtgtgcacaataccaaaaacgccgtcacttttcatgtatttgtcgtgtttgtttgttcgaaaaccataagaagactaagctttttattgttacagattttaactttcagttacttttctatgtaatcgaatattatcagtgcttgggctccgaagacggtatctttctaacaagagcttattttaagacgccgctttgaggctacttaaattactaaataacgtaataagcacgagaatattcggatccggtagcagatgcattcgtgaagcagttgtccttttttttgagctgtaattttttttttattgcttagatgggtgggcgagctcacagcccaagtgttaagttactggagaccatagacatctacaacgtaaatgcgccacccaccttgagatctaagttctaaggtctcagtacagttactacggctgcctcacccttccagccaaaacgcattctgcttcacggcagaaataagcggggtggtggtacctacttgtgcggactcacaagaggtcctaccaccaagactctttcggaggcgatcgggaaactgttagctaatcccaactctcatggctgagcctttgctggcccacctatcctggtgaaactggaaaggcctccaggccaccagtaatctttcaatcataaaaaatcacaaacagtgtaaataaaataaaagcgtcctttgaagtaaccaaaatttggaatacaaacatttcttcatgacttacattttgaatgattaataagaaatgattagtttttaataattaacttcatgcttcctcacctctcaggttaaccataaagtattattatatgcgatttttaacttcacgttaacaggggaacgagtgcgcaaagaaacatttcgtatcaggtattgggttcagagcttcattctcattagtacagtcatcgctttgacattttggcttaacatccttatcagcgtgtcgatcttcattcgccattcgttccataccgacactcattaacaggacttcgtctgagtgtttcatgctctaattaatcgtatcgccaaaatcgtatctattcacatccattaacataccgaaaacgaaccataaaccataatggtgtcgcggaaaaaccgatgtaacgttttataaatatcggttttccagaaacaggcgaagaagaggaattgttcgatgttgtatcttaccagaaaattgaagatggcaagcctgtaatcataatgaaagttataccagtcggtaagataaacgttgatgaagatacaataatgtcgtttaattaaagacaaatgaaactgcattgcgcattcggtacagaaagtacgacaggcatgaagtaatcaatagttaaaggtattgaataggtacagtagatatgatgtctacttaacgaaatacaagatcgacaatgctattaagatattaagttaaaatgtcaaaaatctcaattattatctaagtcttgagggtaggaaaaatccgataaatgactatatgtcgggtattaggtattactatcgaaatttcggaagtaatttatttagcgtacgttttatagagaaatccgcgtcccaatcaagttcttcgcggtcatctcaggagtctgcaagctatagcagcagcagcagttcatcgagtaagttcattagcgttttatgaagcgaacacgaattaatcggccacaggcctgacatacgcctttaaatcctacgacaaatgaaaaagattctcttaaagaaggcaaagaatgacaattcttttctcaaagcacatcgttggtattgcgttgtgaactcttgggtgtccggcatctaattaacctaagaaggcgcatctacagcgcttcctcggttctacagcaggtgtaaattatgttttagttagacattcctcaagagtttttttgatttgttttttattaatatttgaatagcttccttctgtatcgtgataaacaggaatattggggaatagctttagtcatgatcaaatcggtattgcgctttaggtccacgtccactctccatatggaccggtccaggccgtgatatacccttcttcagaagaaaatactcaggcgctcgctctgttcctaagccaataccaataccaattcaatcaaaaggttcaacggaacgaccacagcctacagggcaccgttcaggtacttgtgatattacgtcaccacatgtcatcagcaatcatacgatcacaagtcatatcatttataatctgtccacattcatagaccagagaactgacgataaacttaaagctattcctttttgaaatttaaagcagaagaatcctcatcctcgagctctagggctgcttcatcaaccgacgcttctagcaacactgattcaaactcaaacagcgcgggatccagtacatccggcggtagcagcacttatggatacagttccaacagtcgtgatggaagtgtatcgaccaccggcagttccagtaacactgattcgaattcaaacagcgtaggatccaggaaatccggcggtagcagctctcatgaagacagttccaagagtcgtgatgaaaatgtatcgaccaccggcagttccagtaacaccgattcaaactcaaacagcgcaggatccagtacatctggcggtagcagcacttatggatacagttccaacagtcgtgatggaagtgtatcatccaccggcagttccagtaacaccgattcaaactcaaacagcgcaggatccagtacttctggcggtagcagcacttatggatacagctccaacagtcgtgatggaagtgtatcatccaccggcagttccagtaacactgattcaaactcaaacagcgtaggatccaggaaatccggcggtagcagctctcatgaagacagttccaagagtcgtgatgaaactgtatcgaccaccgacagttccagtaacactgattcaaattcaaacagcgtagaaaccaggaaatccggcggtagcagctctcatgaagacagttccaagagtcgtgatgaaaatgtatcgaccaccggcagttccagtaacactgattcaaactcaaacagcgcaggatccagtacatctggcggtagcagcacttatggatacagctccaacagtcgtgatggaagtgtatcatccaccggcagttctagtaacactgattcaaactcaaacagcgccggatccagtacatcgggcggtagcagcacttatggatacagttccaacagtcatgatggaagtgtatcatctaccggcagttccagtaacactgattcgaattcaaacagcgtaggatccaggaaatccggcggtagcagctctcatgaagacagttccaagagtcgtgatgaaaatgtatcgaccaccggcagttccagtaacactgattcaaactcaaacagcgcaggatccagtacatctggcggtagcagcacttatggatacagctccaacagtcgtgatggaagtgtatcatccaccggcagttccagttacactgattcaaactcaaacagcgccggatccagtacatcgggcggtagcagcacttatggatacagttccaacagtcatgatggaagtgtatcatctaccggcagttccagtaacactgattcgaattcaaacagcgtaggatccaggaaatccggcggtagcagctctcatgaagacagttccaagagtcgtgatgaaaatgtatcgaccaccggcagttccagtaacaccgattcaaactcaaacagcgcaggatccagtacatctggcggtagcagcacttatggatacagctccaacagtcgtgatggaagtgtatcatccaccggcagttccagtaacactgattcaaactcaaacagcgccggatccagtacatcgggcggtagcagcacttatggatacagttccaacagtcatgatggaagtgtatcatctaccggcagttccagtaacactgattcgaattcaaacagcgtagaatccaagaaatccggcggtagcagctctcatgaagacagttccaagagtcgtgatggaagtgtatcatccaccggcagttccagtaacactgattcaaactcaaacagtgcaggatccagtacatctggcggtagcagcacttatggatacagctccaacagtcgtgatggaagtgtatcatccaccggcagttccagtaacactgattcaaactcaaacagcgccggatccagtacatcgggcggtagcagcacttatggatacagttccaacagtcatgatggaagtgtatcatctaccggcagttccagtaacactgattcgatttcaaacagcgtaggatccaggaaatctggcggtagcagctctcatgaagacagttccaagagtcgtgatgaaaatgtatcgaccaccggcagttccagtaacaccgattcaaactcaaacagcgcaggatccagtacatctggcggtagcagcacttatggatacagctccaacagtcgtgatggaagtgtatcatccaccggcagttccagttacactgattcaaactcaaacagcgccggatccagtacatcgggcggtagcagcacttatggatacagttccaacagtcatgatggaagtgtatcatctaccggcagttctagtaacactgattcgaattcaaacagcgtaggatccaggaaatccggcggtagcagctctcatgaagacagttccaagagtcgtgatgaaaatgtatcgaccaccggcagttccagtaacaccgattcaaactcaaacagcgcaggatccagtacatctggcggtagcagcacttatggatacagctccaacagtcgtgatggaagtgtatcatccaccggcagttccagttacactgattcaaactcaaacagcgccggatccagtacatcgggcggtagcagcacttatggatacagttccaacagtcgtgatggaagtgtatcatccaccggcagttccagtaacactgattcgaattcaaacagcgtaggatccaggaaatccggcggtagcagctctcatgaagacagttccaagagtcgtgatgaaaatgtatcgaccaccggcagttccagtaacactgattcaaactcaaacagcgcaggatccagtacatctggcggtagcagcacttatggatacagttccaatagtcgtgatggaagtgtatcatccaccggcagttccagtaacactgattcaaactcaaacagcgcgggatccagtacatccggtggtagcagcacttatggatacagttccaacagtcgtgatggaagtgtatcatccaccggcagttccagttacactgattcaaactcaaacagcgcaggatccagtacatctggtggtagcagcacttatggatacagttccaacagtcgtgatgaaagtgtatcatccaccggcagttccagtaacactgattcgaattcaaacagcgtaggatccaggaaatccggcggtagcagctctcatgaagacagttccaagagtcgtgatgaaaatgtatcgaccaccggcagttccagtaacaccgattcaaactcaaacagcgcaggatccagtacatctggcggtagcagcacttatggatacagctccaacagtcgtgatggaagcgtatcatccaccggcagttccagtaacactgattcaaactcaaacagcgccggatccagtacatcgggcggtagcagcacttatggatacagttccaacagtcatgatggaagtgtatcatctaccggcagttccagtaacactgattcgaattcaaacagcgtaggttccaggaaatccggcggtagcagctctcatgaagacagttccaagagtcgtgatggaagtgtatcatccactggcagttccagtaacactgattcaaactcaaacagcgcaggatccagtacatctggcggtagcagcacttatggatacagctccaacagtcgtgatggaagtgtatcatccaccggcagttccagttacactgattcaaactcaaacagcgcaggatccagtacatcgggcggtagcagcacttatggatacagttccaacagtcatgatggaagtgtatcatctaccggcagttccagtaacactgattcgaattcaaacagcgtaggatctaggaaatccgacggtagcagctctcatgaagacagttccaagagtcgtgatgaaaatgtatcgaccaccgacagttccagtaacaccgattcaaactcaaacagtgcaggatccagtacatccggtggtagcagcacttatggatacagctccaacagccgtgatggaagtgtatcatccaccggcagttccagtaacactgattcaaactcaaacagcgccggatccagtacatcgggcggtagcagcacttatggatacagttccaacagtcgtgatggaagtgtatcatccaccggcagttccagtaacactgattcaaactcaaacagcgcgggatccagtacatccggtggtagcagcaattatggatacagttccaacagtcgtgatggaggtgtatcatccaccggcagttccagttacactgattcaaactcaaacagcgccggatccagtacatcgggcggtagcagcacttatggatacagttccaacagtcatgatggaagtgtatcatctaccggcagttccagtaacactgattcgaattcaaacagcgtaggttccaggaaatccggcggtagcagctctcatgaagacagttccaagagtcgtgatgaaaatgtatcgaccaccggcagttccagtaacactgattcaaactcaaacagcgcaggatccagtacatctggcggtagcagcacttatggatacagttccaatagtcgtgatggaagtgtatcatccaccggcagttccagtaacactgattcaaactcaaacagcgcgggatccagtacatccggtggtagcagcacttatggatacagttccaacagtcgtgatggaagtgtatcatccaccggcagttccagttacactgattcaaactcaaacagcgcaggatccagtacatctggtggtagcagcacttatggatacagttccaacagtcgtgatgaaagtgtatcatccaccggcagttccagtaacactgattcgaattcaaacagcgtaggatccaggaaatccggcggtagcagctctcatgaagacagttccaagagtcgtgatgaaaatgtatcgaccaccggcagttccagtaacactgattcaaactcaaacagcgcaggatccagaacatctggcggtagcagcacttatggatatagttacaacagtcgtgatggaagtgtatcatccaccggcagttccagtaacactgattcaaactcaaacagcgcaggatccagtacatctggtggtagcagcacttatggatacagttccaacagtcgtgatgaaagtgtatcatccaccggcagttccagtaacactgattcgaattcaaacagcgtaggatccaggaaatccgacggtagcagctctcatgaagacagttccaagagtcgtgatgaaagtgtatcgaccaccggcagttccagtaacactgattcaaactcaagcagcgcaggatccagtacatccggtggtagcagcacttatggatacagctccaacagtggtgatggaagtgtatcatccaccggcagttccagtaacactgagtcaaactcaaacagcgaaggatccagaacatctggcggtagcagcacttatggatacagttccaacagtcgtgatggaagtgtatcatccaccggcagttccagtaacactgattcaaactcaaacagcgcaggatccagtacatctggtggtagcagcacttatggatacagttccaacagtcgtgatgaaagtgtatcatccaccggcagttccagtaacactgattcgaattcaaacagcgtaggatccaggaaatccgacggtagcagctctcatgaagacagttccaagagtcgtgatgaaaatgtatcgaccaccggcagttccagtaacactgattcaaactcaagcagcgcaggatccagtacatccggtggtagcagcacttatggatacagctccaacagtggtgatggaagtgtatcatccaccggcagttccagtaacactgattcaaactcaaacagcgcaggatccagtacatctggcggtagcagcacttatggatacagctccaacagtcgtgatggaagtgtatcatccaccggcagttccagtaacactgattcaaactcaaacagcgcaggatccagtacatctggcggtagcagcacttatggatacagctccaacagtcgtgatggaagtgtatcatccaccggcagttccagtaacactgattcaaactcaaacagcgcaggatccagtacatctggcagtagcaacactcatggtgccagccatggtttggcatcatctggcggtagtatagcatcagcaactagtactcctgacatacttaccataggtacctgtattgtatttgaaaaaactttagctttttttttatcctacctgagttggtagctttagaggattatgttagcgtcaccgagcgaataggtgagctaacgggacttctaatctgtggaagtttagctaattatacaaatttgtaaacagtgacaaattaccaactgggatcgacgtaggaaataatgttatctatcatattttatgtaatttaaatactgtctaagctctgtattcattttaccatttttaaagttatacatgaatccatatgactcatttttgtatcggcaattagaaaatgcaaaatcatgcaacatttttaccgaagcggccggatattccttcgattaactgagaagttccgctaaagtcttgagagagaccctatctgattgaatgtctctcagctgatcagattaccgtacgataccgaactccttatcaaaattaaaacattgcagcttatattgtgcaagtaatttcgcggataccgaaaaccaatccgtaattttgagactgttttggacagctttattttcacttatgaagtcgacatggcctacgggataagacacggtgcattcgttactagcggtgtcgatgttcgaatcccgcaggcatgtgccaatttatcgaatgaaataagcaattaacatattttcacgaattactttcacggtgaaaataacatcgtggaatatagacaataacaatcccgtactagataattgtaatcgaaaaatcaatagctttaataaaccctgcctacttataccgtgtggcaataatacgtttcggcagccgttgtactgaaaaactgagacttaaaactcatgtgtcaagggtgggtggcggaatttacgtcgttgatatctatgagcgccggtgaccgctaaacaccaagtgggccgtgagttcgtcagttcatccattatagcaatcattaaaaattacgtttcatttctttccagcactaagtgaagactcttccgaggtggatattgatcttggcaatttaggctggtggtggaattcagacaataaggcacaaagagcggcaggcggcgcaacaaagtctgaagcttcatcatccactcaaggtagattttgtgattgtcgaataacaatcttaatgtgtaagggattatcaagaaaatacccaatattacttcaaactttggtatttttgggaaagacacgaccgcattttttgaaacttatgctgtgtaaggattgcatactttcaatccgacaattacgttacagtaaaaaggtgaagtttaattttattgagtctctgaaacaaccccataagggggttgcctccatcatcatcattagcccaccgacgtccactgctatacaagtatccccaaagtttcgccgcaaagaccggtcctacgcagcccggcatctagcgtattcccacaacctttagcagttgtcgttcaaactcattggaggtctacccaatctacgtttttcagagcacgatcgccaatcgagaactcgccctcgtactcccgcccaaattgaatacgacagaaaaagccttttttactatgaattggttccgatagacccgagtagatatgacaaataatcaccacccgaaatgatgaccagtgaccacgatcacccggccaagaatgcaagcgactgagaagaagtattgtacacaacccaccgagtttatcggcgattcttctcagggggtcgcgattccgatccggtggtagattctgcgaagtactgctcttgttagggctagttaaaaaaaatctcaggttgagcccgtgagacctgagggggtgaggccgcgcggcgcgctaccagcactctagcgcgctgccgtggaatgaatagagcgaccggtcgacggtgtatcgcgtcccgaccgggcaggctggttctggtccagcggggtattccgggacaccagcggcaccgtctgggcggcccgacgggctgccgtaccgagacggccgacgtttcagagccttcgattcgcctcgaaggctccgtcggctgggcgtccttggggtgagccgcgccgtctggttgtagtgttgaccgcggtagcccccctacctcatccgggttctgacctcggaggggatcggacgtcgggtgtaagagtgcaggggagtcgtttagtgggtgggtcctaaaatccttgggcccgcggtctgctcacaacaccatgcagatcgttgagtctcacataccccgcgcgccccttttgcgcggggacctcgtaggagattcggccctctacccgaaaaaaaaaaaaaaaaaaggttgagcccgtgagctcacctacccgtccgggcatagctggaatagcccttcagtttttaacatttctgacaaacgggcaggaactgcctcctagataccttggaacaaatagccccttagactaccagcgaataggtaggaggaaaaaaagtactgtatgtacaataatcaaaaactatcagttcaatatattcatagacctcttatgttcaaaagagtgcaaaactaaaattactttgtcgttttattaatttcgtttggtttattttaagtattcgacccttaacatttctcgagaataccatcgactaaggttgtttgttaaattcgtcgcgtcgatcgcgtaaagctaactcaaatttgctcaattatgcagctaactaaaaaaaattgtgtgaacttgaaacagcgcccctggcggcaaacgaagggaagctatttcaactccatacgaattggagttaacttttacgcgatcgagaacgttaaaaaaactcgccctaagcacacagtcctgtttaatttatttattgcccgtgtccacatattaatagtgctttgtgtacacagtcggtggagaatggtaacagtagcatggaatatttagtatagagtagtgttctatggtatgacgcataagtaacttagcataaacataacttctaactacaaataattgtaacacacccaatgtttcgactaattacacaaaaaaaaattacagctactacagtcagtggcgcagacgacagtgctgattcttacacctggtggtggaatcctagacgatcaagcagctcctcttcatcagcaagttctagcagctctggctccaatgttggtggttcctctcaatccagcggtagcagcacttctggaagtaatgcccgcggtcatctaggaaccgtttcgtccactggcagtaccagtaacaccgattcaagctcaaaaagtgcaggatcccgtacatccggcggtagcagcacttatggatatagctccagccatcgtggtggaagcgtatcatccaccggcagttccagcaacactgattcaagcacaaagaatgcaggatccagtacatccggcggtagcagcacttatggatatagctccagccatcgtggtggaagcgtatcatccaccggcagttccagcaacactgattcaagcacaaagaatgcaggatccagtacatctggcggtagcagcacttatggatatagctctagccatcgtggtggaagtgtatcatccaccggcagttccagcaacactgattcaagcacaaagagtgcaggatccagtacatccggcggtagcagcacttacggatatagctccaggcatcgtggtggacgcgtatcatccaccggcagttccagcacaactgatgcaagctcaaacagcgtaggatctagtacatccggcggtagcagcacttatggatacagttccaacagtcgtgatggaagtgtatcatccaccggcagttccagtaacactgattcaaactcaaacagcgcgggatccagtacatccggtggtagcagcacttatggatacagttccaacagtcgtgatggaagtgtatcatccaccggcagttccagtaacactgattcaaactcaaacagcgcgggatccagtacatccggtggtagcagcacttatggatacagttccaacagtcgtgatggaagtgtatcatccaccggcagttccagtaacactgatgcaagcacagacctggcaggatccagtacatctggcggtagcagcacttatggatacagttccgactgtggtgatggaagtgtatcatccaccggcagttccagtaacactgatgcaagcacagaccttgcaggatccagtacatccggcggtagcagcacttatggatacagttccgacagtcgtgatggaagtgtatcatccaccggcagttccagtaacactgatgcaagcacagaccttgcaggatccagtacatcgggcggtagcagcacttatggatacagttccaacagtcgtgatggaagtgtatcatccaccggcagttccagtaacactgatgcaagcacagaccttacaggatccagtacatccggcggtagcagcacttatggatatagctcaagcaatcgtgatggaagtgtattggccactggcagttccagtaacactgatgcaagcaccacagaagaatccaccacgtccgctggtagcagcactgaaggatatagttccagtagccatgatggaagcgtaacatccaccgacggttccagcacaagtggaggagcttcttccagctcaggtactctaaaaagtcacgttacttcctctttttaatcactgtcaactcaaactggatctatctatttttccatttcaataaactttaattttatttgatttaaatttgggcactaccgaacttcgcgcgatcactctctaggtaaatccgaagatatccttaaaattccaccgaaataggtccagccgtttcaaagtatatagggaaaataggtttacgcattggttgctcctcattagtgatctggaattgtgaccggaattgttgtcagtggaagtgttggcaggtctactgtcatagccaatctctgcttaatactgtaaatgtgacagtgtgtttatttatttgtccttttctttcacgtcgagacgaaacaacatgattttttgtaaagtaattaatagttttacgtcaggaaagtgacataggctaccttttatccagtaaaccatctcattacccgggaaaatactctgacattttacattgatcacgcggacgaagcagcgattaacagctagttcgtttattaccaaaacacttttgttctgttaactagtagcaggcctaaaactcaattggtgggtacagaaagaaattttctaacactagccccagcaagttaatttataaggatataacctgttttcaaaatatggtactgttatatcatatactccaagaggaagctattatttttaatgtagagaactgagccattaatgagatactgggccattgtttacatgtcccttgaatgaattcatattccaataagcagcaattgaaatcacgctgaattagaatagtcaaaatgaatacgtctttgaaaacgtataatgtgttggttttatatattacagcgtcaaccgccaaaagcgacgccgcgtcatctgaagacggtttctggtggtggaatagaaggaaatcaggatccggtcacaaaagcgctaccgtacagtcatccacaaccgataagacgagcaccgacagtgccagcagcaccgattccacctcaagcacgtccggggcaagcacaaccacttcaggcagttcttctacctcgggcggttcaagtacatcggacgcttcctccacttcgtctagtgtttccagaagtcatcgttcaggcgtgaacagacttttacacaagcctggtcaaggaaaaatatgcctttgcttcgaaaacatattcgatattccttaccatctccgtaagaatatcggtgtttaatacaactaaacacgacttggagtattccttgtagtgtttaagattttaaatcttacttaatgacttcgaacgattttaacgataactttctctttgtttaactttaatcagcatacataaaaagccccggttttgtatcgggaagaaaaaaaatgtaattgtgttgcctagataataaacgtattatcaaagtgtgtggttttcctttaccaaagacccctttaagatgggcctaatgggcttaagtcgagtcctttccgatgtgttaaatacacatttattacactgatgcgtcgaatgtacacttttaataggatagctccactaaaaattattttatttatttaatttgttgcaccaaaactgatacattgacgaaatgatgcaatagttagcggctgacttatgcgtcgagggttgtgggttcgattcccacgtcgggcaaacattctgtaatgaacaggtttgctcttcgtctgggtgattattatctatatatatatataaatgtatataagacagtttttggtatacataaaaaagggaatcataaattggggatgaccgtccgggtgaccgtgcgttcttacttatttatttcccagatgacggacgagctcacagcccgttgaggtgtcatcgatcgagtggaatcgaaatacattcgttgcctttttattcgtttattgcttagatagatggacgagctcacggcccgcctgatgttaaggggttaccgtagctcatagacatctacaaagtaaatgccgccacccaccttgagagttctctcggttattacagtacaacggctgccccgcccttcaaactgaaatgcgttactgcttcacggcaaaaatagacctttgaggaggtgttacctactcgtggggactcacaagacgcccccaagacctggcatttacactgtgatgtctatcaactccaataatcacttaaacacgtcagctaataatgctccagtctaaacaggaaaaaa

SEQ ID NO: 10 - protein, 220 aa, Bombyx mori
MLARCLAVAAVAVLASAGPPSPIYRPCYLDDYKCISDHLAAISKCIPGRGQIPSQYEIPVFQFEIPYFNATYVDHNLITRNHDKCRVSEFYDNVRTLKTVLTVDCPWLNFESNRTLAQHMSFKEDVVLSFYINGSYPLIRLTTVFDKGNNFDLCSAFTFADLAGGLPIFHINPNDQRTAQWLSKDLTLLHIYEREHIFGKRNWLARSFISRTLCDFGCHH

SEQ ID NO: 11 - protein, 203 aa, Bombyx mori
GPPSPIYRPCYLDDYKCISDHLAAISKCIPGRGQIPSQYEIPVFQFEIPYFNATYVDHNLITRNHDKCRVSEFYDNVRTLKTVLTVDCPWLNFESNRTLAQHMSFKEDVVLSFYINGSYPLIRLTTVFDKGNNFDLCSAFTFADLAGGLPIFHINPNDQRTAQWLSKDLTLLHIYEREHIFGKRNWLARSFISRTLCDFGCHH

SEQ ID NO: 12 - DNA, 4970 bp, Bombyx mori
  source 1..4970: mol_type = genomic DNA
acaattttgtttttcctttgatgtgttccccgtcggacggattcttttaggtcttttatttatcgattgaggcactacgaagtctgccgggtcagctagtgtactcataaataagctcaactttaatagggtattacatttaattaggcgtatttggtatttacgttcacgctttaatcttttttggttgattttaatttctgtctgtgatcgctatggcggttattgagcaatgccttcgtccaacagttgacgtttgttgatgatggtgatatcttgaaaattaccttagcgcaatgtaggcttatacagtatttctgtttttctaagttaattaccgctgtagccaataccgtctttaccataagggcacacggggcccgtgcccagggcccccattctcagggggccccgaaagaccgacaatttctctcacacgtttattcccaaaacatttttgtcgggcaaattacagttttttcacaaatcagtaatcagaaggtatttacaaggcatatactatgcctataatagaagattttgctcaacagaaatcccgaaagaaaccgttatcgaaatcgtaaccaaaaaaccagcagcattctaatatcattaatgacatattatatcatactgtatttgattacctataataaatggtcatactcagtaaaaaaatgttaatataattcgctttttttactttccaaaagggcctcaaattcttgtgtgtccaagggccccatcctagtttaagacgtccctggctgtagcccagttaccgccaaacaaacgtgcattactccccgcctacaccgaggagaacattttgcgccttagaaaataaaatggcgtcgccgcggcgcaacaatgagaacttaattcgtgcaattgtttccacgacaatatttatttaacgttattcgttatgaggaacaatactttgtataattaatgttgatcggtgcctaacgacgcagttgtttattattcgcgcaacatgctggcgcggtgtctagctgtagccgctgtggcagttttggcttctgcaggtaagtccgatgtttcttgattaggtcaattataactacacgtaacgctttgtgattaatcgggaagactattgattaattatattccgtaacacggggtatattagtcctggtgttaaacagttgtcgaagtccattgactttccattgaatttcgccgacatcctcatcaggcaacactgttgcaaggaattcttcccaaatccggatggtgcgtggcaaaattaacatttggaaacgtattgaacgcagaagatagctctggtgctggacggtgtggtagtaaaaaggagatggttgaatcatttccactaatttcttacagaagtcgctctggtactaagcccagagcacctgtctaaaattacaagtgaaggacggctgttttctctgcagcagaaggtggtaggactgtggacccactgcatgcgcactaacaagaagccccaccactcattgctcatatataatcttgtacccacagggccgccgagtccgatctacaggccctgctacttggacgattacaaatgcatctccgaccacctggccgcgatctcgaaatgtatcccgggcagagggcagatcccctcgcagtacgagataccggtgttccagtttgaaataccatacttcaacgccacctacgtcgaccataatctcattacccgtaaccacgacaaatgccgtgtcagcgaattttagtaagttctatggggcttcatatctttttccctgtggcttcatacctttttccctgtccccgtcctcttgctacctgcagccttcttgtctaagaacggtgggactatgccggtgtttgaatcccacaagcgggtaccagcttctctaaagaaatacgtatacttcgacgcatacgtgtgagagttcacacgtgttcacgaacatcttccacgttcagaaatagcatcgtgtagttaaatcatacgttagactttgaaaatttgggtaatgatcggtggcctcaccatcttgcctatttcagccgcgaagtagtcacgcattcccgtcgagagcggggcaacctcgtgtgtcaaggtgagtgcgggcattcgtgacgtaataaacactatggacttctcataagtcggaagtccgtctgccaaacttaactatagtagaattattttgtccgtgcagtttgggtcataaaaaaatcggaacggtgaagcgagtatttcgctttctcttccactcacgagccttatggacgggcatagtgatgcgcattattgttgtcgataagcgttatcgatattgtatttagttttgtcattttgtgggttagtgataaaaatgaaagaaaaaatcactaatcgaacacttacaccacatatcgccgcagcaagttcacgagaacggcagaaattaacactttgttacttttcgggatctattgttatttcagtgaaattttttaacccattgttgataacaacacgtgcacatattattttgaataaattctgccgttttgatacaaaacaaaggagtacccattgtgtcactaaagaatcagagaacgaatgcataaaaacacatctctcttcgacataatgtactataatttgcaggtaggtacaacaaatgactcataactgcatcaccacccttcgtatgccaccccgccaccgtgtacctgccttcgatgactaatttgtttttatcgatattggcgttgcgcccgcgcaacattctcaccgccctagccgggctatgttttatgacccaaactgcacggacaaaataataataattttactatagcaaataaaacttggatgaggtacctactaactgaggctgttgggcttctgctaaggcagaagcccaacagcccaatatcatacgtctgagaaagtatgaaaggtcgtgatacattttgtgtgacgatttttaaattatcattatttatgttatattaaaataattgagggtaggtaaattaaaatatttatttaagcttacctttgcattccaaccaccttcagtagatgtttgcaaatacgtcttgtttgcagtgacaatgtgagaactttaaaaacagttttaaccgtggactgtccgtggctgaactttgaatccaatcggaccttggctcagcacatgtcgttcaaggaagacgtcgtcttaagcttctacatcaatggatcttatcgtaagtttccaggagtacacggcacatgctttattaaaactagtgggtaagctgacctaagggtgagctggcttatttttcgttaaaacagactaaactataattttactattactattttattacgttaataatcttcttatttctccaccttatcccactaggtgggtcggcacagctaatttttctcttccattctcttctatcagccgtcatctcaacactcactcctctctctctcatatcgtcattcacacactccgttcatgtcttcttcggtcgacctcttccccctctaccttgcactaccatttccatacatctcctagtcacacgcatcttctctctactcatcacgtgtccacaccacgttaatactattttattcaacagctttgatcaggctaacgacagtgtttgataagggcaacaatttcgacttgtgttcggctttcacgttcgcagacctggccgggggtctgcccatcttccacattaaccctaatggtgagcagataaagtctggattacactggatatgagctatgcgtttataagggcgggtgcacgtcaacgttgtaccatgtattgttttccagaccaacgcacagcgcagtggttgtctaaagatctgaccctgctgcacatttacgagagagagcacatcttcggaaagaggaactggctggcgaggtccttcatcagcagaacactctgcgacttcggttgtcaccactgagcgacatttctccaacataatattctatttcgcaaatacttttcgacatatggccttttcgcattaaaagtgtacaattttcaaaaatatataaatatatgcggaatcatttggtatcactagtatttttctcataaatactgtcaaaagagcgtagtttagttttagtttacttatgtttcgactactattcacaaaattaatacataattttataaaagacagaaaatgtaactggtaaaaaataaatgttgcaaagatgtttaatattaaaaaaattacatgttaaacctttaaaacactctcctataaaattttagattagaaaagattagaaatgatacagttttaatgcgagaagacgttgtaccaaacatccaatgaatattgttccgtctgtgatttacttctcatctgaaactttttgacatcactattctgaattccaaaattgaaatttcaaataaaacacagagcgaattgatccaaatttattgtctttttttttaattttcaacagccgtgactgtagaatcgtaatcatatgtcgattttacagttttcatctaagcactatatttaagtctataccaacgtaggttttgttaaacataacataataaaagaatacaactgcacgctatatattaaataaacaaatgaactataaactttttacgaataatatttaatactagcgacccgccgtcgcttcgcttcggaaacattaaattttattattgatagctgagtcccgcgatgttacccgcggttattgtcgtatcgcgggtgacgccgcgaggcgaagctagtttaaaaaaaagtagcctaagttactccttatatcatcagctacctatcagtgaaagtcccgtcaaaatcggtcgtgccgttccagagattagccggaacaaacagacagacagacaaaaattgtaaaaaatgatattttggtgtatgtaccgtatatatatattcatatgcatgtagtaaaaagcgg

SEQ ID NO: 13 - DNA, 1092 bp, synthetic construct
  source 1..1092: mol_type = other DNA
taacttcgattgaatgtgcgatcaatattttcgaaatttatagcacttatcgtattgatttaagaaaaaattgttaacattttgtttcagtatgtcgcttatacaaatgcagtgagcaagggcgaggagctgttcaccggggtggtgcccatcctggtcgagctggacggcgacgtaaacggccacaagttcagcgtgtccggcgagggcgagggcgatgccacctacggcaagctgaccctgaagttcatctgcaccaccggcaagctgcccgtgccctggcccaccctcgtgaccaccctgacctacggcgtgcagtgcttcagccgctaccccgaccacatgaagcagcacgacttcttcaagtccgccatgcccgaaggctacgtccaggagcgcaccatcttcttcaaggacgacggcaactacaagacccgcgccgaggtgaagttcgagggcgacaccctggtgaaccgcatcgagctgaagggcatcgacttcaaggaggacggcaacatcctggggcacaagctggagtacaactacaacagccacaacgtctatatcatggccgacaagcagaagaacggcatcaaggtgaacttcaagatccgccacaacatcgaggacggcagcgtgcagctcgccgaccactaccagcagaacacccccatcggcgacggccccgtgctgctgcccgacaaccactacctgagcacccagtccgccctgagcaaagaccccaacgagaagcgcgatcacatggtcctgctggagttcgtgaccgccgccgggatcactctcggcatggacgagctgtacaagtaacctagggctaggaggaaatacaacaaacacgactggagtattccttgtagtgtttaagattttaaatcttacttaatgacttcgaacgatttaacgataactttctctttgtttaactttaatcagcatacataaaaagccccggttttgtaccgggaagaaaaaaaatgtaattgtgttgcctagataataaacgtattatcaaagtgtgtggttttcctttaccaaagacccctttaagatgggcctaatgggcttaagtcg

SEQ ID NO: 14 - protein, 259 aa, synthetic construct
MRVKTFVILCCALQYVAYTNAVSKGEELFTGVVPILVELDGDVNGHKFSVSGEGEGDATYGKLTLKFICTTGKLPVPWPTLVTTLTYGVQCFSRYPDHMKQHDFFKSAMPEGYVQERTIFFKDDGNYKTRAEVKFEGDTLVNRIELKGIDFKEDGNILGHKLEYNYNSHNVYIMADKQKNGIKVNFKIRHNIEDGSVQLADHYQQNTPIGDGPVLLPDNHYLSTQSALSKDPNEKRDHMVLLEFVTAAGITLGMDELYK

SEQ ID NO: 15 - DNA, 6424 bp, synthetic construct
  source 1..6424: mol_type = other DNA
taacttcgattgaatgtgcgaaatttatagctcaatattttagcacttatcgtattgatttaggatccatgagagtcaaaacctttgtgatcttgtgctgcgctctgcaggtgagttaattattttactattatttcagaaggtggccagacgatatcacgggccacctgataataagtggtcgccaaaacgcacagatatcgtaaattgtgccatttgatttgtcacgcccgggggggctacggaataaactacatttatttatttaaaaaatgaaccttagattatgtaacttgtgatttatttgcgtcaaaagtaggcaagatgaatctatgtaaatacctgggcagacttgcaatatcctatttcaccggtaaatcagcattgcaatatgcaatgcatattcaacaatatgtaaaacaattcgtaaagcatcattagaaaatagacgaaagaaattgcataaaattataaccgcattattaatttattatgatatctattaacaattgctattgcctttttttcgcaaattataatcattttcataacctcgaggtagcattctgttacattttaatacattggtatgtgattataacacgagctgcccactgagtttctcgccagatcttctcagtgggtcgcgttaccgatcacgtgatagattctatgaagcactgctcttgttagggctagtgttagcaaattctttcaggttgagtctgagagctcacctacccatcggagcgtagctggaataggctaccagctaataggtagggaaaacaaagctcgaaacaagctcaagtaataacaacataatgtgaccataaaatctcgtggtgtatgagatacaattatgtactttcccacaaatgtttacataattagaatgttgttcaacttgcctaacgccccagctagaacattcaattattactattaccactactaaggcagtatgtcctaactcgttccagatcagcgctatctacgattgaaagagcgtaatttatagctcaatattttatgctcataacgtattgatttaagaaaaaattgttaacattttgtttcagtatgtcgcttatacaaatgcaatggtgagcaagggcgaggagctgttcaccggggtggtgcccatcctggtcgagctggacggcgacgtaaacggccacaagttcagcgtgtccggcgagggcgagggcgatgccacctacggcaagctgaccctgaagttcatctgcaccaccggcaagctgcccgtgccctggcccaccctcgtgaccaccctgacctacggcgtgcagtgcttcagccgctaccccgaccacatgaagcagcacgacttcttcaagtccgccatgcccgaaggctacgtccaggagcgcaccatcttcttcaaggacgacggcaactacaagacccgcgccgaggtgaagttcgagggcgacaccctggtgaaccgcatcgagctgaagggcatcgacttcaaggaggacggcaacatcctggggcacaagctggagtacaactacaacagccacaacgtctatatcatggccgacaagcagaagaacggcatcaaggtgaacttcaagatccgccacaacatcgaggacggcagcgtgcagctcgccgaccactaccagcagaacacccccatcggcgacggccccgtgctgctgcccgacaaccactacctgagcacccagtccgccctgagcaaagaccccaacgagaagcgcgatcacatggtcctgctggagttcgtgaccgccgccgggatcactctcggcatggacgagctgtacaagtaaaacagctaggaggaaatacaacaaacacgactggagtattccttgtagtgtttaagattttaaatcttacttaatgacttcgaacgatttaacgataactttctctttgtttaactttaatcagcatacataaaaagccccggttttgtaccgggaagaaaaaaaatgtaattgtgttgcctagataataaacgtattatcaaagtgtgtggttttcctttaccaaagacccctttaagatgggcctaatgggcttaagtcggctagtgcatggctcagttcgctttaaatatcgatagtctttaaaaaaaaattatgatgtgaaatctgaaaaggtttgcgcactatgcgctcatgcaatttcaactttaatcaatagccctaaagcagtgctgccaacaaataaaaaaatatttattgtaagtgagataactaaatttgtcagaattcatcgcttctttgctattttttattatggtttgtgtttaattatattttaaacgtgttgatgaaatagtaagataattagcattaaatttacaccactttcgtgaaggttttctggctaatcgtttcagtttgtgtggcataaaactatgggctataactattgctggtgagactttaacagcttcataaggacgggtggattaactcaaaaacacagcttggagggaaagagtttgctaatagccgccagagtgcctccaaaaggggtttaatagtactaggacagttactttacgagtgcatctactccgtgtcgagaagcttagagctcagtatcacatacaaatcgtcgacgagttagctgaaccatgcttttattgctcttggcgttaaaattagtagtgataatgagaacgtatcaggtggatcttgcattatttgaaagatgagactaaagatctgtaggttgtgcgagagaatgtcgcgaggcaaaaatagtttcctctacctgtagataacgagaacacaaattttatacagggtgtataggagaagacgaggaacaattattttaatgatttctgacatctaaatgaacaataagattttacttttgatgaacaaaacaagtaactcacatcttaaactgaacgttactacgttctggtttgctattgtaattttaatcaatgttttctccaatctgcattatgatacaataaaagctcattattcgcgtttccttcactcgcgttttcactattcgcagattaaaatgtgtcccaattcctattttcgcaattaaagatctctttattcgcggatctaatcgatacatagacattgataaaaagaaatccaatattaagtattcaactgaatatcctttataatcgcgctataatcacggtttatctataaagccttgttcggactaggcgagtattttagtcgagtaccgagtaatttagtagctaaatgtgtccgagcaccaaaagtttagtcgagtaggttagtaaataatttagtaaagccaatccattttgttctattttatcgggcgagtagcgcctcccaccacgcgtcctagctcactggctcactgactaaacaagtccgaacctgttgattagtcgagttcattagtggcgcttctcaaatggaactttcggacattcttaaactatcgaagtattctttgggatctcttccaatgctaattctttcagaagacatttatctcttcaatcgatccattttcgtacctataacttatttttcataatcacagaaatttgctcgtccaccttttctaaaatagccattacgattagcttaatcagtttattcactctattgcgttgcagtctgttcatcctgcaaaacaccactcacttgtgtactctactggaccgtaatgcgaacgatttctgtgcagtagcgagtagtttagccactaaattactcggtactcgactaaaatactcgcctagtccgaacaaggctttagcgacatatttacgtaacgtatacaccccgataaagagatttactgtccaaaaaaaacgtcaaaaaatggaacaaattatgtgctttttatttattggtattactaatttcgttaagaatttcatcggaagcagccagcgccgaatgcggtgaatagtaaaactataagaaggaagcggttggaatgatctgggtaaaatgttatttcttacgaattacgatgattctttgattaaatttggaaaagttttgtggtcaaattatttaacattcatcttgtatcatttattgactctaatttcaactaagttatttctgtaatgttaaaatttcgatgcttttctagaatattcaggaatgttccagatattcttgtgtgtagatcgtattgccaccttgtgccaaatagcggcactaaaataattcggcagagctatacaacatttggtaattttatttattttgctattttccccagttttttaaattactgtgtttttaactagcaattacatttaattggatgcaatttacactgccttaataatttttttttagttgtaatttggtttcttacgtttatgctgtatatttttagtgatctgcaaaatgcgaaacactgaacagcttaggaaaatttaaaatgtgagatgtttcttttacttaaataaatacttaaaatataacagagaaaaaacatttttaactagactggcatattttagtgaatctattgatgaaaatgaacgaaatatgtaattacctttataatttcttgaattattttaaggaaatatatttttcctaacactttaaacttcaaagcgggtgatgcaataataactaacacaaaaagaaacttgcagtgttaagtaaatgatttttctcttcgttttatggcctcccaaaatgaaataattgccaattaatttgaaatgattaattatttttatttaatattgtttcggtttgtattgatggtaaaatgttgatgctctctgacggaaatagcgtcagaatcgagaaacttctactgattcatagatgtcgcttgctagaggaaagtataaaaacgaatttacacaccgcgcccggcgttatttgaactaagagaagtacggagactaacgtttgatactttgcgctttgaaacacgtgtgttaaaaaccctctagtcattttgtgtgaattaacatggcctcctccgagaacgtcatcaccgagttcatgcgcttcaaggtgcgcatggagggcaccgtgaacggccacgagttcgagatcgagggcgagggcgagggccgcccctacgagggccacaacaccgtgaagctgaaggtgaccaagggcggccccctgcccttcgcctgggacatcctgtccccccagttccagtacggctccaaggtgtacgtgaagcaccccgccgacatccccgactacaagaagctgtccttccccgagggcttcaagtgggagcgcgtgatgaacttcgaggacggcggcgtggcgaccgtgacccaggactcctccctgcaggacggctgcttcatctacaaggtgaagttcatcggcgtgaacttcccctccgacggccccgtgatgcagaagaagaccatgggctgggaggcctccaccgagcgcctgtacccccgcgacggcgtgctgaagggcgagacccacaaggccctgaagctgaaggacggcggccactacctggtggagttcaagtccatctacatggccaagaagcccgtgcagctgcccggctactactacgtggacgccaagctggacatcacctcccacaacgaggactacaccatcgtggagcagtacgagcgcaccgagggccgccaccacctgttcctgtaacctaggtaaacgcgttttttaatataaaataacccttgtttcttacttcgtcctggatacatctatgttttttttttcgttaataaatgagagcatttaagttattgtttttaattacttttttttagaaaacagatttcggattttttgtatgcattttatttgaatgtactaatataatcaattaatcaatgaattcatttatttaagggataacaataatccatgaattcacatgcacatttaaaacaaaactaaattacaataggttcatataaaaacaacaagtatgccttctcaactaagaatactataggccgggctagcaacatcaatgattttgatgaggactattttgggagtgatgtcactgtccaaagtagtaatacaacagatgaaataattagagatgcatctggggcagttatcgaagaacaaattacaactaaaaaaatgcaacggaaaaataaaaaccatggaatacttggaaaaaatgaaaaaatgatcaagacgttcgttataaccacggattccgacggtaacgagtccattgtagaggaagatgtgctcatgaagacactttccgatggtactgttgctcaaagttatgttgctgctgatgcgggagcatattctcagagcgggccatacgtatcaaacagtggatacagcactcatcaaggatatacgagcgatttcagcactagttaacttcgattgaatgtgcgaaatttatagctcaatattttagcacttatcgtattgattta

SEQ ID NO: 16 - DNA, 7495 bp, synthetic construct
  source 1..7495: mol_type = other DNA
tcccgagaaaacaatttgttgtgtataatttaaaccaaaacccgaatttaatttttcgcaggatcctctctttgtatgtctgtcttttcagaagtcaaaaaatgtactgccgtgccgctggtcacgtacgccctcgttccatttattttcgaattattttcaaatctctgtcttagtttgtctatgtctagtcattgtaggtcttatgtcctgtcaaaaaggtcacacgccactacaaatactttagcgttttcgtgaacacggacgatttaattactatcaaattctctaggaaaacatttctaaagattcttaaggttcgcttagaacgtctgtttgttcgtttggtaaaaacaaaaggagcacacaaaacataaaaattttatctttgtcatttctcgcaatcccctttttttacggaaacacctaccatgcgtttacgaactaactttactgatggacctcttgtcagtccacatgggtaggtaccaccaccctgcctatttttgacgtgaagcagtaatgcgtttcggtttgaagggtggggcagcacttttaactatacttgggaccttagaacttatatctcaagatgggtggtgcatttacattatagatgtctatgggcttcagtaaccacttaacaccaggtgggctgtcatctcgtacaatcatctaagcactaaaaaataaaaataacttcctcaccaaaacaatatcatcgcgtgtgtagttatagtgaaataatttattgcgagctcgcacgaatatcctccctatgcctattactgcggcgaaataatacactttccaagatgaaacaatataataatatgtactcagactacaacctcatgtctcaaggtctcatgtgaatttgttcgcctccgagcgctacttaacgtgagatcgaacgcgaactccatctagaactataatataataatcattagaatggagtaggtcgtctgaaattcgattctccgctataacccgttaatctaacctgaccattaagtaaataaaaattagctctagatgagctcccggcgtacctggtcgcattaacacatcgatcggtggagcgacaaagctcttcgctctaagcctcaaaagaacaatcccgagaaaagaattcgttctgtataatttaaaccaaaattcgaatttaatttttcgcagagcgcctacgctgtgagcaagggcgaggagctgttcaccggggtggtgcccatcctggtcgagctggacggcgacgtaaacggccacaagttcagcgtgtccggcgagggcgagggcgatgccacctacggcaagctgaccctgaagttcatctgcaccaccggcaagctgcccgtgccctggcccaccctcgtgaccaccctgacctacggcgtgcagtgcttcagccgctaccccgaccacatgaagcagcacgacttcttcaagtccgccatgcccgaaggctacgtccaggagcgcaccatcttcttcaaggacgacggcaactacaagacccgcgccgaggtgaagttcgagggcgacaccctggtgaaccgcatcgagctgaagggcatcgacttcaaggaggacggcaacatcctggggcacaagctggagtacaactacaacagccacaacgtctatatcatggccgacaagcagaagaacggcatcaaggtgaacttcaagatccgccacaacatcgaggacggcagcgtgcagctcgccgaccactaccagcagaacacccccatcggcgacggccccgtgctgctgcccgacaaccactacctgagcacccagtccgccctgagcaaagaccccaacgagaagcgcgatcacatggtcctgctggagttcgtgaccgccgccgggatcactctcggcatggacgagctgtacaagtaacctagggctaggaggaaatacaacaaacacgactggagtattccttgtagtgtttaagattttaaatcttacttaatgacttcgaacgatttaacgataactttctctttgtttaactttaatcagcatacataaaaagccccggttttgtaccgggaagaaaaaaaatgtaattgtgttgcctagataataaacgtattatcaaagtgtgtggttttcctttaccaaagacccctttaagatgggcctaatgggcttaagtcggctagtgcatggctcagttcgctttaaatatcgatagtctttaaaaaaaaattatgatgtgaaatctgaaaaggtttgcgcactatgcgctcatgcaatttcaactttaatcaatagccctaaagcagtgctgccaacaaataaaaaaatatttattgtaagtgagataactaaatttgtcagaattcatcgcttctttgctattttttattatggtttgtgtttaattatattttaaacgtgttgatgaaatagtaagataattagcattaaatttacaccactttcgtgaaggttttctggctaatcgtttcagtttgtgtggcataaaactatgggctataactattgctggtgagactttaacagcttcataaggacgggtggattaactcaaaaacacagcttggagggaaagagtttgctaatagccgccagagtgcctccaaaaggggtttaatagtactaggacagttactttacgagtgcatctactccgtgtcgagaagcttagagctcagtatcacatacaaatcgtcgacgagttagctgaaccatgcttttattgctcttggcgttaaaattagtagtgataatgagaacgtatcaggtggatcttgcattatttgaaagatgagactaaagatctgtaggttgtgcgagagaatgtcgcgaggcaaaaatagtttcctctacctgtagataacgagaacacaaattttatacagggtgtataggagaagacgaggaacaattattttaatgatttctgacatctaaatgaacaataagattttacttttgatgaacaaaacaagtaactcacatcttaaactgaacgttactacgttctggtttgctattgtaattttaatcaatgttttctccaatctgcattatgatacaataaaagctcattattcgcgtttccttcactcgcgttttcactattcgcagattaaaatgtgtcccaattcctattttcgcaattaaagatctctttattcgcggatctaatcgatacatagacattgataaaaagaaatccaatattaagtattcaactgaatatcctttataatcgcgctataatcacggtttatctataaagccttgttcggactaggcgagtattttagtcgagtaccgagtaatttagtagctaaatgtgtccgagcaccaaaagtttagtcgagtaggttagtaaataatttagtaaagccaatccattttgttctattttatcgggcgagtagcgcctcccaccacgcgtcctagctcactggctcactgactaaacaagtccgaacctgttgattagtcgagttcattagtggcgcttctcaaatggaactttcggacattcttaaactatcgaagtattctttgggatctcttccaatgctaattctttcagaagacatttatctcttcaatcgatccattttcgtacctataacttatttttcataatcacagaaatttgctcgtccaccttttctaaaatagccattacgattagcttaatcagtttattcactctattgcgttgcagtctgttcatcctgcaaaacaccactcacttgtgtactctactggaccgtaatgcgaacgatttctgtgcagtagcgagtagtttagccactaaattactcggtactcgactaaaatactcgcctagtccgaacaaggctttagcgacatatttacgtaacgtatacaccccgataaagagatttactgtccaaaaaaaacgtcaaaaaatggaacaaattatgtgctttttatttattggtattactaatttcgttaagaatttcatcggaagcagccagcgccgaatgcggtgaatagtaaaactataagaaggaagcggttggaatgatctgggtaaaatgttatttcttacgaattacgatgattctttgattaaatttggaaaagttttgtggtcaaattatttaacattcatcttgtatcatttattgactctaatttcaactaagttatttctgtaatgttaaaatttcgatgcttttctagaatattcaggaatgttccagatattcttgtgtgtagatcgtattgccaccttgtgccaaatagcggcactaaaataattcggcagagctatacaacatttggtaattttatttattttgctattttccccagttttttaaattactgtgtttttaactagcaattacatttaattggatgcaatttacactgccttaataatttttttttagttgtaatttggtttcttacgtttatgctgtatatttttagtgatctgcaaaatgcgaaacactgaacagcttaggaaaatttaaaatgtgagatgtttcttttacttaaataaatacttaaaatataacagagaaaaaacatttttaactagactggcatattttagtgaatctattgatgaaaatgaacgaaatatgtaattacctttataatttcttgaattattttaaggaaatatatttttcctaacactttaaacttcaaagcgggtgatgcaataataactaacacaaaaagaaacttgcagtgttaagtaaatgatttttctcttcgttttatggcctcccaaaatgaaataattgccaattaatttgaaatgattaattatttttatttaatattgtttcggtttgtattgatggtaaaatgttgatgctctctgacggaaatagcgtcagaatcgagaaacttctactgattcatagatgtcgcttgctagaggaaagtataaaaacgaatttacacaccgcgcccggcgttatttgaactaagagaagtacggagactaacgtttgatactttgcgctttgaaacacgtgtgttaaaaaccctctagtcattttgtgtgaattaacatggcctcctccgagaacgtcatcaccgagttcatgcgcttcaaggtgcgcatggagggcaccgtgaacggccacgagttcgagatcgagggcgagggcgagggccgcccctacgagggccacaacaccgtgaagctgaaggtgaccaagggcggccccctgcccttcgcctgggacatcctgtccccccagttccagtacggctccaaggtgtacgtgaagcaccccgccgacatccccgactacaagaagctgtccttccccgagggcttcaagtgggagcgcgtgatgaacttcgaggacggcggcgtggcgaccgtgacccaggactcctccctgcaggacggctgcttcatctacaaggtgaagttcatcggcgtgaacttcccctccgacggccccgtgatgcagaagaagaccatgggctgggaggcctccaccgagcgcctgtacccccgcgacggcgtgctgaagggcgagacccacaaggccctgaagctgaaggacggcggccactacctggtggagttcaagtccatctacatggccaagaagcccgtgcagctgcccggctactactacgtggacgccaagctggacatcacctcccacaacgaggactacaccatcgtggagcagtacgagcgcaccgagggccgccaccacctgttcctgtaacctaggtaaacgcgttttttaatataaaataacccttgtttcttacttcgtcctggatacatctatgttttttttttcgttaataaatgagagcatttaagttattgtttttaattacttttttttagaaaacagatttcggattttttgtatgcattttatttgaatgtactaatataatcaattaatcaatgaattcatttatttaagggataacaataatccatgaattcacatgcacatttaaaacaaaactaaattacaataggttcatataaaaacaacaagtatgccttctcaactaagaatactataggccgggctagcgcaccatcggtgaccatcaatcaatacagtgataatgaaattccacgcgacattgatgatggaaaagctaggtaattatgtaagctttaactaatattaatataggtcttatataatccggcagaggcaaatgcaccgagcgacttccgcaatagaccacgacgacttcgactaaaatatcttcattatttttttattactttttaaaaaatatgaaaatacggtccattgaatggtcaattatcaccgtcacagatcatcacatcagcagtaccaaagacacatagaataactgacgttatactattttccaacctcgttcgctcgatctgcgccattgagggtggatcatttcacgatcatacggcaaaaatgatcacccaaaatgcactgtaaatcatcgttagtggtttcaagaagtagtagtgaactcttctccagtggtgggtggtgtgattttcctcaatgacaaattcttcagaacactgcccatggaacatacagtaagaaatacaaagggaatcaaagtcccaccgtagccccagaggctcttacttatccttctgtatgaagtcaaacagaactatctcgaaattggatatagaagttccctacgtcaaatagaaagtggaagtcttgatattaaggcggagtgaaagcctcacacccaaaatcccttgaccctctgagggcttgattgaccgatgagtgatcgatatctgaacgtccatgaccaaaacagttactaataaactgagacctatcaagttaggccaagttctctaggaacaggatatcgataaaccactctatcatctcggaaagcagagtactcatagttatcgtataggccttaactcatagtcagttacgtcattttatttgggaagagaatggacgtgagtattctgtcacaaagacgaaatcctattgccatgtgtctttgaatctaatttgggtatcggaaaatctgggagttgtacggcgtatacatcgtttaaaagcagactatataatacgaatcgcaactatgaagccaatcatcacagtgcatctagtgataatagacatcacgacgtcaatggcaccgactatcttaagactagaagttaaactgtctgttgcattgaaatctattacaccgaaatcgttttgctgcttcaaaactgtaacagacaaagctcacagtatcctttctttaaactatgtttttattgcacaaaacttttcaatcatggttcaagtgttttcaataattatatattcaataattattataattttagttccgtaatctcacgtgcatgggactacgtcgatgacaccgacaaaagcatcgccatcctcaacgttcaagaccgcggtcccgagaaaacaatttgttgtgtataatttaaaccaaaacccgaatttaatttttcgca

SEQ ID NO: 17 - protein, 254 aa, synthetic construct
MKPIFLVLLVATSAYAVSKGEELFTGVVPILVELDGDVNGHKFSVSGEGEGDATYGKLTLKFICTTGKLPVPWPTLVTTLTYGVQCFSRYPDHMKQHDFFKSAMPEGYVQERTIFFKDDGNYKTRAEVKFEGDTLVNRIELKGIDFKEDGNILGHKLEYNYNSHNVYIMADKQKNGIKVNFKIRHNIEDGSVQLADHYQQNTPIGDGPVLLPDNHYLSTQSALSKDPNEKRDHMVLLEFVTAAGITLGMDELYK

SEQ ID NO: 18 - DNA, 9060 bp, synthetic construct
  source 1..9060: mol_type = other DNA
tatattgtaaagcacaacatatatattaatgaattttttatttatttttcaggatccatgcgtttcgttctgtgctgcactttgattgcgttggctgtgagtatcattgcttcgttatcaacaatgacgtatttactaagaacactcttagatatgccttcaaattaaagctttcaaagctctgaagttcaccaaatacgactgttttagcgtaagctatttctatcccccaacagccatttagcgactacccgaaaatcactcgatttaacttgggagtttctgcaaactaaaagttcacaggccgtccccgattaaacttttaaacgcttcgcgaaaatatcagagttattcaaaagttgccacaaaaacctttgtccactaatatctatagaaggactggcggttagcagcaaatcatctagattttgggtggttggttcagaattttccattttactcttgggagtcgtttcggtctgcattccctacgcattattagaatccatcgaatgtaatttgtataattacgagttaaatactgtgtacaaaccaatatgtgaatttttattcaactagtttattgtttttaacttataggtaccagttttgaaacgaacttcagagttatctagaaaacacataattatgagtcgcttcactaatctatattaaattatgctttaatacttttaatagcttacttggggaaattgtgatttttcatgtaataacagtccacttggtcataagcagcttttatgggcttgcgctggacatgaatgccgcagaaccaacgatcgttggagcagacggggtcttgagtggagaccgcgtgccggctaacgtagtgtgggacgcctcccgaccaagtggagggctggcttgcgatttgggagaggcctatgtctagcagggaacgattaggagctgatgattatggtcataattgacagtcacttcgtttatagcaatcaaatatcctgggcattttgagggtattttgctaaacgaagacatttattcgaacgtaatttaatttaatttaatttattgcttagatgggtgggcgagctcacagcccacctggtgttaagtggttactggagcccatagacatctacgacgtaaatgcgccacccaccttgagatataagttctaaggtctcagtgtagttacaacggctgccccgcccttcaaaccgaaacgcattaactgcttcacggcagaaataggcagggtggtggtacctacccgtgcggacccacaataggtcctaccaccagtccaatggtatcccaaaaatttatcataacaatcctgatttttaagaatgaggcagtcgttcttagactcttcgtttccaggaagacgacattaatattcggtttaattggctatagtgactatgttatcctagttggtaattaattcactagcataactatatgattatcgttaatccgattcgtctttttctttctctgtttgattgcttaccaatcgctctgggagcaatttggtttgactctgttggtttagtctttttttttaatcatcatcaccttgatgtcaaaataatgttcttgtgaacaatttcgactaacttaacgaggggtgaaaggcaatttggtataagcttaatagtatttatctttaattaaaggtccattttatttggtactagcgacccgccctcgcttcgctacggaaactgtaatttattattgatttctccactattcaatggatgttattatacatataaaccttcctcttcaatcgctctatctattaaaaaaaaaccgcatcaaaatccgttgcgtagttttaaagatttaagcatacgtagggacagacagatatagggacagagaaagcgactttgttttatactatgtagtgattagtatcaacagttcgatgtttttaatttaacttgaattaagtttaccccattcaaatagctgaagtttttttttttttcatattaaaaactttaaatggcttccatgtaaagttgcaaaaatgtcacttaaaatagacacccctcgaagtattgagaagcacaagtaatatattaatgaattttttctttctttttcaggcgctgtcagttaaagctgtgagcaagggcgaggagctgttcaccggggtggtgcccatcctggtcgagctggacggcgacgtaaacggccacaagttcagcgtgtccggcgagggcgagggcgatgccacctacggcaagctgaccctgaagttcatctgcaccaccggcaagctgcccgtgccctggcccaccctcgtgaccaccctgacctacggcgtgcagtgcttcagccgctaccccgaccacatgaagcagcacgacttcttcaagtccgccatgcccgaaggctacgtccaggagcgcaccatcttcttcaaggacgacggcaactacaagacccgcgccgaggtgaagttcgagggcgacaccctggtgaaccgcatcgagctgaagggcatcgacttcaaggaggacggcaacatcctggggcacaagctggagtacaactacaacagccacaacgtctatatcatggccgacaagcagaagaacggcatcaaggtgaacttcaagatccgccacaacatcgaggacggcagcgtgcagctcgccgaccactaccagcagaacacccccatcggcgacggccccgtgctgctgcccgacaaccactacctgagcacccagtccgccctgagcaaagaccccaacgagaagcgcgatcacatggtcctgctggagttcgtgaccgccgccgggatcactctcggcatggacgagctgtacaagtaacctagggctaggaggaaatacaacaaacacgactggagtattccttgtagtgtttaagattttaaatcttacttaatgacttcgaacgatttaacgataactttctctttgtttaactttaatcagcatacataaaaagccccggttttgtaccgggaagaaaaaaaatgtaattgtgttgcctagataataaacgtattatcaaagtgtgtggttttcctttaccaaagacccctttaagatgggcctaatgggcttaagtcggctagtgcatggctcagttcgctttaaatatcgatagtctttaaaaaaaaattatgatgtgaaatctgaaaaggtttgcgcactatgcgctcatgcaatttcaactttaatcaatagccctaaagcagtgctgccaacaaataaaaaaatatttattgtaagtgagataactaaatttgtcagaattcatcgcttctttgctattttttattatggtttgtgtttaattatattttaaacgtgttgatgaaatagtaagataattagcattaaatttacaccactttcgtgaaggttttctggctaatcgtttcagtttgtgtggcataaaactatgggctataactattgctggtgagactttaacagcttcataaggacgggtggattaactcaaaaacacagcttggagggaaagagtttgctaatagccgccagagtgcctccaaaaggggtttaatagtactaggacagttactttacgagtgcatctactccgtgtcgagaagcttagagctcagtatcacatacaaatcgtcgacgagttagctgaaccatgcttttattgctcttggcgttaaaattagtagtgataatgagaacgtatcaggtggatcttgcattatttgaaagatgagactaaagatctgtaggttgtgcgagagaatgtcgcgaggcaaaaatagtttcctctacctgtagataacgagaacacaaattttatacagggtgtataggagaagacgaggaacaattattttaatgatttctgacatctaaatgaacaataagattttacttttgatgaacaaaacaagtaactcacatcttaaactgaacgttactacgttctggtttgctattgtaattttaatcaatgttttctccaatctgcattatgatacaataaaagctcattattcgcgtttccttcactcgcgttttcactattcgcagattaaaatgtgtcccaattcctattttcgcaattaaagatctctttattcgcggatctaatcgatacatagacattgataaaaagaaatccaatattaagtattcaactgaatatcctttataatcgcgctataatcacggtttatctataaagccttgttcggactaggcgagtattttagtcgagtaccgagtaatttagtagctaaatgtgtccgagcaccaaaagtttagtcgagtaggttagtaaataatttagtaaagccaatccattttgttctattttatcgggcgagtagcgcctcccaccacgcgtcctagctcactggctcactgactaaacaagtccgaacctgttgattagtcgagttcattagtggcgcttctcaaatggaactttcggacattcttaaactatcgaagtattctttgggatctcttccaatgctaattctttcagaagacatttatctcttcaatcgatccattttcgtacctataacttatttttcataatcacagaaatttgctcgtccaccttttctaaaatagccattacgattagcttaatcagtttattcactctattgcgttgcagtctgttcatcctgcaaaacaccactcacttgtgtactctactggaccgtaatgcgaacgatttctgtgcagtagcgagtagtttagccactaaattactcggtactcgactaaaatactcgcctagtccgaacaaggctttagcgacatatttacgtaacgtatacaccccgataaagagatttactgtccaaaaaaaacgtcaaaaaatggaacaaattatgtgctttttatttattggtattactaatttcgttaagaatttcatcggaagcagccagcgccgaatgcggtgaatagtaaaactataagaaggaagcggttggaatgatctgggtaaaatgttatttcttacgaattacgatgattctttgattaaatttggaaaagttttgtggtcaaattatttaacattcatcttgtatcatttattgactctaatttcaactaagttatttctgtaatgttaaaatttcgatgcttttctagaatattcaggaatgttccagatattcttgtgtgtagatcgtattgccaccttgtgccaaatagcggcactaaaataattcggcagagctatacaacatttggtaattttatttattttgctattttccccagttttttaaattactgtgtttttaactagcaattacatttaattggatgcaatttacactgccttaataatttttttttagttgtaatttggtttcttacgtttatgctgtatatttttagtgatctgcaaaatgcgaaacactgaacagcttaggaaaatttaaaatgtgagatgtttcttttacttaaataaatacttaaaatataacagagaaaaaacatttttaactagactggcatattttagtgaatctattgatgaaaatgaacgaaatatgtaattacctttataatttcttgaattattttaaggaaatatatttttcctaacactttaaacttcaaagcgggtgatgcaataataactaacacaaaaagaaacttgcagtgttaagtaaatgatttttctcttcgttttatggcctcccaaaatgaaataattgccaattaatttgaaatgattaattatttttatttaatattgtttcggtttgtattgatggtaaaatgttgatgctctctgacggaaatagcgtcagaatcgagaaacttctactgattcatagatgtcgcttgctagaggaaagtataaaaacgaatttacacaccgcgcccggcgttatttgaactaagagaagtacggagactaacgtttgatactttgcgctttgaaacacgtgtgttaaaaaccctctagtcattttgtgtgaattaacatggcctcctccgagaacgtcatcaccgagttcatgcgcttcaaggtgcgcatggagggcaccgtgaacggccacgagttcgagatcgagggcgagggcgagggccgcccctacgagggccacaacaccgtgaagctgaaggtgaccaagggcggccccctgcccttcgcctgggacatcctgtccccccagttccagtacggctccaaggtgtacgtgaagcaccccgccgacatccccgactacaagaagctgtccttccccgagggcttcaagtgggagcgcgtgatgaacttcgaggacggcggcgtggcgaccgtgacccaggactcctccctgcaggacggctgcttcatctacaaggtgaagttcatcggcgtgaacttcccctccgacggccccgtgatgcagaagaagaccatgggctgggaggcctccaccgagcgcctgtacccccgcgacggcgtgctgaagggcgagacccacaaggccctgaagctgaaggacggcggccactacctggtggagttcaagtccatctacatggccaagaagcccgtgcagctgcccggctactactacgtggacgccaagctggacatcacctcccacaacgaggactacaccatcgtggagcagtacgagcgcaccgagggccgccaccacctgttcctgtaacctaggtaaacgcgttttttaatataaaataacccttgtttcttacttcgtcctggatacatctatgttttttttttcgttaataaatgagagcatttaagttattgtttttaattacttttttttagaaaacagatttcggattttttgtatgcattttatttgaatgtactaatataatcaattaatcaatgaattcatttatttaagggataacaataatccatgaattcacatgcacatttaaaacaaaactaaattacaataggttcatataaaaacaacaagtatgccttctcaactaagaatactataggccgggctagcttcggtcaccaccgtgagtattccttatgacacattattcccgcaaaactcttacagaaacttcttagaatgcatcctttttacataactctaacctaaacagtgctaatacacaaaagataaacagtattttttttcacgcaggacttggcaattatatcgcaatgatttgaatatatatggttctatatatgggatattactatatttatgtattacgatttgattttggatattttacgtgctgcctgaatttaattgactatgcgaagaatatttcttggataggaaagttaaattctcgcgaattagtagaacgtccaaatttaaaaataatgtatggttatttatatatctagagattaatgatccttatcgtccttaataatagaggtgaatatatcagataaaggaggagactgcgttatctcatcgaaagaccaacaaatttttgtcataaaacatttcttgaaaataaaatttgaaaagttattaagatgtcgaatttcgaaatccgttttcattaatcataatgcatttttttattgaacataacagcaaaatggatttaataagctttcgaactaaacaaaaggttagttctacaaaaaacaaaagtcttcatgtggaaatctaaatcgacataccgccgcttcggaatacagtatcgcaactaagaaaactcatatcgaggggtttttttttggtggatgagctcacagcccacctggtgttaagtggttactggagcccatagacatccacaacgtaaatgcgccacccaccttgagatataagttctaaggtctcagatatagttacaacggctgccccacccttctaaccgaaacgcattactgcttcacggcagaaataggcagggcggtggtacccacccgcgcggactcacaagacgtcctaccaccagtaaaatggggtggaatgctatctggtttaagcgtcatttatctttgtaattaaaggtctgttttattagcatcaacagttcgatatttttaattgaacttccattacgtttaccacactcaaatagctaaagaagttttttttgtaattatattctttccaaatgtttaaactttaaatggctctcttgtatctttgcaaaaatgtcgcttaaacatttcaatcctcgatatgataaggctatttgtacacacacattgtcttcataacattataatttaactatataaaaacattttgtataaaacaacaataccttacaaaatataacgttcgtggatacacttcatgtaggtgcgacaaacacaggcaattttaatttttttttattgcttaagtgtgtggacgagctaacagcccacctggttttcagtggttactggagcccatagacatgtacaacgcgccacccaccttgagaaatattttttttaaggtctcagtatagttacaacagttatattgcggatttgatttttattacacgttacgttattacttcaccgtggaagtcaatcgaaaacatttgttaagtacgtatttcattagaaaaattggtacccgcctgcgggattcgaacaccgttgcatcgctcgatacgaatgaaccggacggacgtcttatcctttaggccacgacgaataaaattagagaataaaaaaaattaaaatttaataaaaggattggtgaaatgtcttcggaaagagtttagttacgcgttaagaagtaatacaaagaaattcaatcatacgaaattcgttccagtttttatggcattagaacacctttttcaatgtcgtctgaatgttaatctatatatataaaaatgaattgctgttcgttagtctcgctaaaactcgagaacggctggaccgatttgcctaattttggtcttgaattatttgtggaagtccagagaaggttaaaaaggtagataaatatgaaaatgcgcggaattaaataaaaataacaattttgttttttctttaatgtgtcccccaaaagtttaggtcccgcggtatattgtaaagcacaacatatatattaatgaattttttatttatttttca

SEQ ID NO: 19 - protein, 257 aa, synthetic construct
MRFVLCCTLIALAALSVKAVSKGEELFTGVVPILVELDGDVNGHKFSVSGEGEGDATYGKLTLKFICTTGKLPVPWPTLVTTLTYGVQCFSRYPDHMKQHDFFKSAMPEGYVQERTIFFKDDGNYKTRAEVKFEGDTLVNRIELKGIDFKEDGNILGHKLEYNYNSHNVYIMADKQKNGIKVNFKIRHNIEDGSVQLADHYQQNTPIGDGPVLLPDNHYLSTQSALSKDPNEKRDHMVLLEFVTAAGITLGMDELYK

SEQ ID NO: 20 - DNA, 432 bp, Homo sapiens
  source 1..432: mol_type = unassigned DNA
atgtggctgcagaacctgcttctcctgggcactgtggtctgcagcttctccgcacctactcgcccacccaacactgccacccggccctggcagcatgtggatgccatcaaggaggccctgagccttctgaaccacagcagtgacactgatgctgtgatgaatgacacagaagtcgtctctgaaaagtttgactcccaggaaccaacgtgcctgcagactcgcctgaagctgtacaagaacggcctgcagggcagcctcactagtctcatgggctccttgaccatgatggccacccactacgagaaacactgcccacccaccccggaaacttcctgtggaacccagtttatcagcttcaaaaatttcaaagaggacctgaaggagttcctttttatcattccctttgactgctgggaaccagcccagaagtga

SEQ ID NO: 21 - protein, 143 aa, Homo sapiens
MWLQNLLLLGTVVCSFSAPTRPPNTATRPWQHVDAIKEALSLLNHSSDTDAVMNDTEVVSEKFDSQEPTCLQTRLKLYKNGLQGSLTSLMGSLTMMATHYEKHCPPTPETSCGTQFISFKNFKEDLKEFLFIIPFDCWEPAQK

SEQ ID NO: 22 - protein, 147 aa, synthetic construct
MRVKTFVILCCALQYVAYTNAAPTRPPNTATRPWQHVDAIKEALSLLNHSSDTDAVMNDTEVVSEKFDSQEPTCLQTRLKLYKNGLQGSLTSLMGSLTMMATHYEKHCPPTPETSCGTQFISFKNFKEDLKEFLFIIPFDCWEPAQK

SEQ ID NO: 23 - DNA, 1413 bp, unidentified
  source 1..1413: mol_type = unassigned DNA
atgggttggagcctcatcttgctcttccttgtcgctgttgctacgcgtgtcctgtcccaggtacaactgcagcagcctggggctgagctggtgaagcctggggcctcagtgaagatgtcctgcaaggcttctggctacacatttaccagttacaatatgcactgggtaaaacagacacctggtcggggcctggaatggattggagctatttatcccggaaatggtgatacttcctacaatcagaagttcaaaggcaaggccacattgactgcagacaaatcctccagcacagcctacatgcagctcagcagcctgacatctgaggactctgcggtctattactgtgcaagatcgacttactacggcggtgactggtacttcaatgtctggggcgcagggaccacggtcaccgtctctgcagctagcaccaagggcccatcggtcttccccctggcaccctcctccaagagcacctctgggggcacagcggccctgggctgcctggtcaaggactacttccccgaaccggtgacggtgtcgtggaactcaggcgccctgaccagcggcgtgcacaccttcccggctgtcctacagtcctcaggactctactccctcagcagcgtggtgaccgtgccctccagcagcttgggcacccagacctacatctgcaacgtgaatcacaagcccagcaacaccaaggtggacaagaaagcagagcccaaatcttgtgacaaaactcacacatgcccaccgtgcccagcacctgaactcctggggggaccgtcagtcttcctcttccccccaaaacccaaggacaccctcatgatctcccggacccctgaggtcacatgcgtggtggtggacgtgagccacgaagaccctgaggtcaagttcaactggtacgtggacggcgtggaggtgcataatgccaagacaaagccgcgggaggagcagtacaacagcacgtaccgtgtggtcagcgtcctcaccgtcctgcaccaggactggctgaatggcaaggagtacaagtgcaaggtctccaacaaagccctcccagcccccatcgagaaaaccatctccaaagccaaagggcagccccgagaaccacaggtgtacaccctgcccccatcccgggacgagctgaccaagaaccaggtcagcctgacctgcctggtcaaaggcttctatcccagcgacatcgccgtggagtgggagagcaatgggcagccggagaacaactacaagaccacgcctcccgtgctggactccgacggctccttcttcctctacagcaagctcaccgtggacaagagcaggtggcagcaggggaacgtcttctcatgctccgtgatgcatgaggctctgcacaaccactacacgcagaagagcctctccctgtctccgggtaaatga

SEQ ID NO: 24 - protein, 470 aa, unidentified
MGWSLILLFLVAVATRVLSQVQLQQPGAELVKPGASVKMSCKASGYTFTSYNMHWVKQTPGRGLEWIGAIYPGNGDTSYNQKFKGKATLTADKSSSTAYMQLSSLTSEDSAVYYCARSTYYGGDWYFNVWGAGTTVTVSAASTKGPSVFPLAPSSKSTSGGTAALGCLVKDYFPEPVTVSWNSGALTSGVHTFPAVLQSSGLYSLSSVVTVPSSSLGTQTYICNVNHKPSNTKVDKKAEPKSCDKTHTCPPCPAPELLGGPSVFLFPPKPKDTLMISRTPEVTCVVVDVSHEDPEVKFNWYVDGVEVHNAKTKPREEQYNSTYRVVSVLTVLHQDWLNGKEYKCKVSNKALPAPIEKTISKAKGQPREPQVYTLPPSRDELTKNQVSLTCLVKGFYPSDIAVEWESNGQPENNYKTTPPVLDSDGSFFLYSKLTVDKSRWQQGNVFSCSVMHEALHNHYTQKSLSLSPGK

SEQ ID NO: 25 - protein, 472 aa, synthetic construct
MRVKTFVILCCALQYVAYTNAQVQLQQPGAELVKPGASVKMSCKASGYTFTSYNMHWVKQTPGRGLEWIGAIYPGNGDTSYNQKFKGKATLTADKSSSTAYMQLSSLTSEDSAVYYCARSTYYGGDWYFNVWGAGTTVTVSAASTKGPSVFPLAPSSKSTSGGTAALGCLVKDYFPEPVTVSWNSGALTSGVHTFPAVLQSSGLYSLSSVVTVPSSSLGTQTYICNVNHKPSNTKVDKKAEPKSCDKTHTCPPCPAPELLGGPSVFLFPPKPKDTLMISRTPEVTCVVVDVSHEDPEVKFNWYVDGVEVHNAKTKPREEQYNSTYRVVSVLTVLHQDWLNGKEYKCKVSNKALPAPIEKTISKAKGQPREPQVYTLPPSRDELTKNQVSLTCLVKGFYPSDIAVEWESNGQPENNYKTTPPVLDSDGSFFLYSKLTVDKSRWQQGNVFSCSVMHEALHNHYTQKSLSLSPGK

SEQ ID NO: 26 - DNA, 708 bp, unidentified
  source 1..708: mol_type = unassigned DNA
atggattttcaggtgcagattatcagcttcctgctaatcagtgcttcagtcataatgtccagaggacaaattgttctctcccagtctccagcaatcctgtctgcatctccaggggagaaggtcacaatgacttgcagggccagctcaagtgtaagttacatccactggttccagcagaagccaggatcctcccccaaaccctggatttatgccacatccaacctggcttctggagtccctgttcgcttcagtggcagtgggtctgggacttcttactctctcacaatcagcagagtggaggctgaagatgctgccacttattactgccagcagtggactagtaacccacccacgttcggaggggggaccaagctggaaatcaaacgtacggtggctgcaccatctgtcttcatcttcccgccatctgatgagcagttgaaatctggaactgcctctgttgtgtgcctgctgaataacttctatcccagagaggccaaagtacagtggaaggtggataacgccctccaatcgggtaactcccaggagagtgtcacagagcaggacagcaaggacagcacctacagcctcagcagcaccctgacgctgagcaaagcagactacgagaaacacaaagtctacgcctgcgaagtcacccatcagggcctgagctcgcccgtcacaaagagcttcaacaggggagagtgttag

SEQ ID NO: 27 - protein, 235 aa, unidentified
MDFQVQIISFLLISASVIMSRGQIVLSQSPAILSASPGEKVTMTCRASSSVSYIHWFQQKPGSSPKPWIYATSNLASGVPVRFSGSGSGTSYSLTISRVEAEDAATYYCQQWTSNPPTFGGGTKLEIKRTVAAPSVFIFPPSDEQLKSGTASVVCLLNNFYPREAKVQWKVDNALQSGNSQESVTEQDSKDSTYSLSSTLTLSKADYEKHKVYACEVTHQGLSSPVTKSFNRGEC

SEQ ID NO: 28 - protein, 229 aa, synthetic construct
MKPIFLVLLVATSAYAQIVLSQSPAILSASPGEKVTMTCRASSSVSYIHWFQQKPGSSPKPWIYATSNLASGVPVRFSGSGSGTSYSLTISRVEAEDAATYYCQQWTSNPPTFGGGTKLEIKRTVAAPSVFIFPPSDEQLKSGTASVVCLLNNFYPREAKVQWKVDNALQSGNSQESVTEQDSKDSTYSLSSTLTLSKADYEKHKVYACEVTHQGLSSPVTKSFNRGEC

SEQ ID NO: 29 - protein, 470 aa, synthetic construct
MKPIFLVLLVATSAYAVSKGEELFTGVVPILVELDGDVNGHKFSVSGEGEGDATYGKLTLKFICTTGKLPVPWPTLVTTLTYGVQCFSRYPDHMKQHDFFKSAMPEGYVQERTIFFKDDGNYKTRAEVKFEGDTLVNRIELKGIDFKEDGNILGHKLEYNYNSHNVYIMADKQKNGIKVNFKIRHNIEDGSVQLADHYQQNTPIGDGPVLLPDNHYLSTQSALSKDPNEKRDHMVLLEFVTAAGITLGMDELYKAPSVTINQYSDNEIPRDIDDGKASSVISRAWDYVDDTDKSIAILNVQEILKDMASQGDYASQASAVAQTAGIIAHLSAGIPGDACAAANVINSYTDGVRSGNFAGFRQSLGPFFGHVGQNLNLINQLVINPGQLRYSVGPALGCAGGGRIYDFEAAWDAILASSDSSFLNEEYCIVKRLYNSRNSQSNNIAAYITAHLLPPVAQVFHQSAGSITDS

SEQ ID NO: 30 - protein, 454 aa, synthetic construct
VSKGEELFTGVVPILVELDGDVNGHKFSVSGEGEGDATYGKLTLKFICTTGKLPVPWPTLVTTLTYGVQCFSRYPDHMKQHDFFKSAMPEGYVQERTIFFKDDGNYKTRAEVKFEGDTLVNRIELKGIDFKEDGNILGHKLEYNYNSHNVYIMADKQKNGIKVNFKIRHNIEDGSVQLADHYQQNTPIGDGPVLLPDNHYLSTQSALSKDPNEKRDHMVLLEFVTAAGITLGMDELYKAPSVTINQYSDNEIPRDIDDGKASSVISRAWDYVDDTDKSIAILNVQEILKDMASQGDYASQASAVAQTAGIIAHLSAGIPGDACAAANVINSYTDGVRSGNFAGFRQSLGPFFGHVGQNLNLINQLVINPGQLRYSVGPALGCAGGGRIYDFEAAWDAILASSDSSFLNEEYCIVKRLYNSRNSQSNNIAAYITAHLLPPVAQVFHQSAGSITDS

SEQ ID NO: 31 - protein, 3533 aa, synthetic construct
MRFVLCCTLIALAALSVKAVSKGEELFTGVVPILVELDGDVNGHKFSVSGEGEGDATYGKLTLKFICTTGKLPVPWPTLVTTLTYGVQCFSRYPDHMKQHDFFKSAMPEGYVQERTIFFKDDGNYKTRAEVKFEGDTLVNRIELKGIDFKEDGNILGHKLEYNYNSHNVYIMADKQKNGIKVNFKIRHNIEDGSVQLADHYQQNTPIGDGPVLLPDNHYLSTQSALSKDPNEKRDHMVLLEFVTAAGITLGMDELYKFGHHPGNRDTVEVKNRKYNAASSESSYLNKDNDSISAGAHRAKSVEQSQDKSKYTSGPEGVSYSGRSQNYKDSKQAYADYHSDPNGGSASAGQSRDSSLRERNVHYVSDGEAVAASSDARDENRSAQQNAQANWNADGSYGVSADRSGSASSRRRQANYYSDKDITAASKDDSRADSSRRSNAYYNRDSDGSESAGLSDRSASSSKNDNVFVYRTKDSIGGQAKSSRSSHSQESDAYYNSSPDGSYNAGTRDSSISNKKKASSTIYADKDQIRAANDRSSSKQLKQSSAQISSGPKGTSVSSKDRQYSNDKRSKSDAYVGRDGTVAYSNKDSEKTSRQSNTNYADQNSVRSDSAASDQTSNSYDKGYSDKNTVAHSSGSRGSQNQKSSSYRADKDGFSSSTNTEKSRFSSSNSVVETSDGTSASRESSAEDTKSSNSNVQSDETGEEEELFDVVSYQKIEDGKPVIIMKVIPVEKSASQSSSSRSSQESASYSSSSSSSTEESSSSSSRAASSTDASSNTDSNSNSAGSSTSGGSSTYGYSSNSRDGSVSTTGSSSNTDSNSNSVGSRKSGGSSSHEDSSKSRDENVSTTGSSSNTDSNSNSAGSSTSGGSSTYGYSSNSRDGSVSSTGSSSNTDSNSNSAGSSTSGGSSTYGYSSNSRDGSVSSTGSSSNTDSNSNSVGSRKSGGSSSHEDSSKSRDETVSTTDSSSNTDSNSNSVETRKSGGSSSHEDSSKSRDENVSTTGSSSNTDSNSNSAGSSTSGGSSTYGYSSNSRDGSVSSTGSSSNTDSNSNSAGSSTSGGSSTYGYSSNSHDGSVSSTGSSSNTDSNSNSVGSRKSGGSSSHEDSSKSRDENVSTTGSSSNTDSNSNSAGSSTSGGSSTYGYSSNSRDGSVSSTGSSSYTDSNSNSAGSSTSGGSSTYGYSSNSHDGSVSSTGSSSNTDSNSNSVGSRKSGGSSSHEDSSKSRDENVSTTGSSSNTDSNSNSAGSSTSGGSSTYGYSSNSRDGSVSSTGSSSNTDSNSNSAGSSTSGGSSTYGYSSNSHDGSVSSTGSSSNTDSNSNSVESKKSGGSSSHEDSSKSRDGSVSSTGSSSNTDSNSNSAGSSTSGGSSTYGYSSNSRDGSVSSTGSSSNTDSNSNSAGSSTSGGSSTYGYSSNSHDGSVSSTGSSSNTDSISNSVGSRKSGGSSSHEDSSKSRDENVSTTGSSSNTDSNSNSAGSSTSGGSSTYGYSSNSRDGSVSSTGSSSYTDSNSNSAGSSTSGGSSTYGYSSNSHDGSVSSTGSSSNTDSNSNSVGSRKSGGSSSHEDSSKSRDENVSTTGSSSNTDSNSNSAGSSTSGGSSTYGYSSNSRDGSVSSTGSSSYTDSNSNSAGSSTSGGSSTYGYSSNSRDGSVSSTGSSSNTDSNSNSVGSRKSGGSSSHEDSSKSRDENVSTTGSSSNTDSNSNSAGSSTSGGSSTYGYSSNSRDGSVSSTGSSSNTDSNSNSAGSSTSGGSSTYGYSSNSRDGSVSSTGSSSYTDSNSNSAGSSTSGGSSTYGYSSNSRDESVSSTGSSSNTDSNSNSVGSRKSGGSSSHEDSSKSRDENVSTTGSSSNTDSNSNSAGSSTSGGSSTYGYSSNSRDGSVSSTGSSSNTDSNSNSAGSSTSGGSSTYGYSSNSHDGSVSSTGSSSNTDSNSNSVGSRKSGGSSSHEDSSKSRDGSVSSTGSSSNTDSNSNSAGSSTSGGSSTYGYSSNSRDGSVSSTGSSSYTDSNSNSAGSSTSGGSSTYGYSSNSHDGSVSSTGSSSNTDSNSNSVGSRKSDGSSSHEDSSKSRDENVSTTDSSSNTDSNSNSAGSSTSGGSSTYGYSSNSRDGSVSSTGSSSNTDSNSNSAGSSTSGGSSTYGYSSNSRDGSVSSTGSSSNTDSNSNSAGSSTSGGSSNYGYSSNSRDGGVSSTGSSSYTDSNSNSAGSSTSGGSSTYGYSSNSHDGSVSSTGSSSNTDSNSNSVGSRKSGGSSSHEDSSKSRDENVSTTGSSSNTDSNSNSAGSSTSGGSSTYGYSSNSRDGSVSSTGSSSNTDSNSNSAGSSTSGGSSTYGYSSNSRDGSVSSTGSSSYTDSNSNSAGSSTSGGSSTYGYSSNSRDESVSSTGSSSNTDSNSNSVGSRKSGGSSSHEDSSKSRDENVSTTGSSSNTDSNSNSAGSRTSGGSSTYGYSYNSRDGSVSSTGSSSNTDSNSNSAGSSTSGGSSTYGYSSNSRDESVSSTGSSSNTDSNSNSVGSRKSDGSSSHEDSSKSRDESVSTTGSSSNTDSNSSSAGSSTSGGSSTYGYSSNSGDGSVSSTGSSSNTESNSNSEGSRTSGGSSTYGYSSNSRDGSVSSTGSSSNTDSNSNSAGSSTSGGSSTYGYSSNSRDESVSSTGSSSNTDSNSNSVGSRKSDGSSSHEDSSKSRDENVSTTGSSSNTDSNSSSAGSSTSGGSSTYGYSSNSGDGSVSSTGSSSNTDSNSNSAGSSTSGGSSTYGYSSNSRDGSVSSTGSSSNTDSNSNSAGSSTSGGSSTYGYSSNSRDGSVSSTGSSSNTDSNSNSAGSSTSGSSNTHGASHGLASSGGSIASATSTPDILTIALSEDSSEVDIDLGNLGWWWNSDNKAQRAAGGATKSEASSSTQATTVSGADDSADSYTWWWNPRRSSSSSSSASSSSSGSNVGGSSQSSGSSTSGSNARGHLGTVSSTGSTSNTDSSSKSAGSRTSGGSSTYGYSSSHRGGSVSSTGSSSNTDSSTKNAGSSTSGGSSTYGYSSSHRGGSVSSTGSSSNTDSSTKNAGSSTSGGSSTYGYSSSHRGGSVSSTGSSSNTDSSTKSAGSSTSGGSSTYGYSSRHRGGRVSSTGSSSTTDASSNSVGSSTSGGSSTYGYSSNSRDGSVSSTGSSSNTDSNSNSAGSSTSGGSSTYGYSSNSRDGSVSSTGSSSNTDSNSNSAGSSTSGGSSTYGYSSNSRDGSVSSTGSSSNTDASTDLAGSSTSGGSSTYGYSSDCGDGSVSSTGSSSNTDASTDLAGSSTSGGSSTYGYSSDSRDGSVSSTGSSSNTDASTDLAGSSTSGGSSTYGYSSNSRDGSVSSTGSSSNTDASTDLTGSSTSGGSSTYGYSSSNRDGSVLATGSSSNTDASTTEESTTSAGSSTEGYSSSSHDGSVTSTDGSSTSGGASSSSASTAKSDAASSEDGFWWWNRRKSGSGHKSATVQSSTTDKTSTDSASSTDSTSSTSGASTTTSGSSSTSGGSSTSDASSTSSSVSRSHRSGVNRLLHKPGQGKICLCFENIFDIPYHLRKNIGV

SEQ ID NO: 32 - protein, 3514 aa, synthetic construct
VSKGEELFTGVVPILVELDGDVNGHKFSVSGEGEGDATYGKLTLKFICTTGKLPVPWPTLVTTLTYGVQCFSRYPDHMKQHDFFKSAMPEGYVQERTIFFKDDGNYKTRAEVKFEGDTLVNRIELKGIDFKEDGNILGHKLEYNYNSHNVYIMADKQKNGIKVNFKIRHNIEDGSVQLADHYQQNTPIGDGPVLLPDNHYLSTQSALSKDPNEKRDHMVLLEFVTAAGITLGMDELYKFGHHPGNRDTVEVKNRKYNAASSESSYLNKDNDSISAGAHRAKSVEQSQDKSKYTSGPEGVSYSGRSQNYKDSKQAYADYHSDPNGGSASAGQSRDSSLRERNVHYVSDGEAVAASSDARDENRSAQQNAQANWNADGSYGVSADRSGSASSRRRQANYYSDKDITAASKDDSRADSSRRSNAYYNRDSDGSESAGLSDRSASSSKNDNVFVYRTKDSIGGQAKSSRSSHSQESDAYYNSSPDGSYNAGTRDSSISNKKKASSTIYADKDQIRAANDRSSSKQLKQSSAQISSGPKGTSVSSKDRQYSNDKRSKSDAYVGRDGTVAYSNKDSEKTSRQSNTNYADQNSVRSDSAASDQTSNSYDKGYSDKNTVAHSSGSRGSQNQKSSSYRADKDGFSSSTNTEKSRFSSSNSVVETSDGTSASRESSAEDTKSSNSNVQSDETGEEEELFDVVSYQKIEDGKPVIIMKVIPVEKSASQSSSSRSSQESASYSSSSSSSTEESSSSSSRAASSTDASSNTDSNSNSAGSSTSGGSSTYGYSSNSRDGSVSTTGSSSNTDSNSNSVGSRKSGGSSSHEDSSKSRDENVSTTGSSSNTDSNSNSAGSSTSGGSSTYGYSSNSRDGSVSSTGSSSNTDSNSNSAGSSTSGGSSTYGYSSNSRDGSVSSTGSSSNTDSNSNSVGSRKSGGSSSHEDSSKSRDETVSTTDSSSNTDSNSNSVETRKSGGSSSHEDSSKSRDENVSTTGSSSNTDSNSNSAGSSTSGGSSTYGYSSNSRDGSVSSTGSSSNTDSNSNSAGSSTSGGSSTYGYSSNSHDGSVSSTGSSSNTDSNSNSVGSRKSGGSSSHEDSSKSRDENVSTTGSSSNTDSNSNSAGSSTSGGSSTYGYSSNSRDGSVSSTGSSSYTDSNSNSAGSSTSGGSSTYGYSSNSHDGSVSSTGSSSNTDSNSNSVGSRKSGGSSSHEDSSKSRDENVSTTGSSSNTDSNSNSAGSSTSGGSSTYGYSSNSRDGSVSSTGSSSNTDSNSNSAGSSTSGGSSTYGYSSNSHDGSVSSTGSSSNTDSNSNSVESKKSGGSSSHEDSSKSRDGSVSSTGSSSNTDSNSNSAGSSTSGGSSTYGYSSNSRDGSVSSTGSSSNTDSNSNSAGSSTSGGSSTYGYSSNSHDGSVSSTGSSSNTDSISNSVGSRKSGGSSSHEDSSKSRDENVSTTGSSSNTDSNSNSAGSSTSGGSSTYGYSSNSRDGSVSSTGSSSYTDSNSNSAGSSTSGGSSTYGYSSNSHDGSVSSTGSSSNTDSNSNSVGSRKSGGSSSHEDSSKSRDENVSTTGSSSNTDSNSNSAGSSTSGGSSTYGYSSNSRDGSVSSTGSSSYTDSNSNSAGSSTSGGSSTYGYSSNSRDGSVSSTGSSSNTDSNSNSVGSRKSGGSSSHEDSSKSRDENVSTTGSSSNTDSNSNSAGSSTSGGSSTYGYSSNSRDGSVSSTGSSSNTDSNSNSAGSSTSGGSSTYGYSSNSRDGSVSSTGSSSYTDSNSNSAGSSTSGGSSTYGYSSNSRDESVSSTGSSSNTDSNSNSVGSRKSGGSSSHEDSSKSRDENVSTTGSSSNTDSNSNSAGSSTSGGSSTYGYSSNSRDGSVSSTGSSSNTDSNSNSAGSSTSGGSSTYGYSSNSHDGSVSSTGSSSNTDSNSNSVGSRKSGGSSSHEDSSKSRDGSVSSTGSSSNTDSNSNSAGSSTSGGSSTYGYSSNSRDGSVSSTGSSSYTDSNSNSAGSSTSGGSSTYGYSSNSHDGSVSSTGSSSNTDSNSNSVGSRKSDGSSSHEDSSKSRDENVSTTDSSSNTDSNSNSAGSSTSGGSSTYGYSSNSRDGSVSSTGSSSNTDSNSNSAGSSTSGGSSTYGYSSNSRDGSVSSTGSSSNTDSNSNSAGSSTSGGSSNYGYSSNSRDGGVSSTGSSSYTDSNSNSAGSSTSGGSSTYGYSSNSHDGSVSSTGSSSNTDSNSNSVGSRKSGGSSSHEDSSKSRDENVSTTGSSSNTDSNSNSAGSSTSGGSSTYGYSSNSRDGSVSSTGSSSNTDSNSNSAGSSTSGGSSTYGYSSNSRDGSVSSTGSSSYTDSNSNSAGSSTSGGSSTYGYSSNSRDESVSSTGSSSNTDSNSNSVGSRKSGGSSSHEDSSKSRDENVSTTGSSSNTDSNSNSAGSRTSGGSSTYGYSYNSRDGSVSSTGSSSNTDSNSNSAGSSTSGGSSTYGYSSNSRDESVSSTGSSSNTDSNSNSVGSRKSDGSSSHEDSSKSRDESVSTTGSSSNTDSNSSSAGSSTSGGSSTYGYSSNSGDGSVSSTGSSSNTESNSNSEGSRTSGGSSTYGYSSNSRDGSVSSTGSSSNTDSNSNSAGSSTSGGSSTYGYSSNSRDESVSSTGSSSNTDSNSNSVGSRKSDGSSSHEDSSKSRDENVSTTGSSSNTDSNSSSAGSSTSGGSSTYGYSSNSGDGSVSSTGSSSNTDSNSNSAGSSTSGGSSTYGYSSNSRDGSVSSTGSSSNTDSNSNSAGSSTSGGSSTYGYSSNSRDGSVSSTGSSSNTDSNSNSAGSSTSGSSNTHGASHGLASSGGSIASATSTPDILTIALSEDSSEVDIDLGNLGWWWNSDNKAQRAAGGATKSEASSSTQATTVSGADDSADSYTWWWNPRRSSSSSSSASSSSSGSNVGGSSQSSGSSTSGSNARGHLGTVSSTGSTSNTDSSSKSAGSRTSGGSSTYGYSSSHRGGSVSSTGSSSNTDSSTKNAGSSTSGGSSTYGYSSSHRGGSVSSTGSSSNTDSSTKNAGSSTSGGSSTYGYSSSHRGGSVSSTGSSSNTDSSTKSAGSSTSGGSSTYGYSSRHRGGRVSSTGSSSTTDASSNSVGSSTSGGSSTYGYSSNSRDGSVSSTGSSSNTDSNSNSAGSSTSGGSSTYGYSSNSRDGSVSSTGSSSNTDSNSNSAGSSTSGGSSTYGYSSNSRDGSVSSTGSSSNTDASTDLAGSSTSGGSSTYGYSSDCGDGSVSSTGSSSNTDASTDLAGSSTSGGSSTYGYSSDSRDGSVSSTGSSSNTDASTDLAGSSTSGGSSTYGYSSNSRDGSVSSTGSSSNTDASTDLTGSSTSGGSSTYGYSSSNRDGSVLATGSSSNTDASTTEESTTSAGSSTEGYSSSSHDGSVTSTDGSSTSGGASSSSASTAKSDAASSEDGFWWWNRRKSGSGHKSATVQSSTTDKTSTDSASSTDSTSSTSGASTTTSGSSSTSGGSSTSDASSTSSSVSRSHRSGVNRLLHKPGQGKICLCFENIFDIPYHLRKNIGV

SEQ ID NO: 33 - DNA, 60 bp, Bombyx mori
  source 1..60: mol_type = genomic DNA
aacttcgattgaatgtgcgaaatttatagctcaatattttagcacttatcgtattgattt

SEQ ID NO: 34 - DNA, 61 bp, synthetic construct
  source 1..61: mol_type = other DNA
atctacgattgaaagagcgtaatttatagctcaatattttatgctcataacgtattgattt

SEQ ID NO: 35 - DNA, 58 bp, Bombyx mori
  source 1..58: mol_type = genomic DNA
cccgagaaaacaatttgttgtgtataatttaaaccaaaacccgaatttaatttttcgc

SEQ ID NO: 36 - DNA, 58 bp, synthetic construct
  source 1..58: mol_type = other DNA
cccgagaaaagaattcgttctgtataatttaaaccaaaattcgaatttaatttttcgc

SEQ ID NO: 37 - DNA, 50 bp, Bombyx mori
  source 1..50: mol_type = genomic DNA
tatattgtaaagcacaacatatatattaatgaattttttatttatttttc

SEQ ID NO: 38 - DNA, 50 bp, synthetic construct
  source 1..50: mol_type = other DNA
agtattgagaagcacaagtaatatattaatgaattttttctttctttttc